European Patent Specification EP 3 630 795 B1, published July 26, 2023. Title: Engineered aldolase polypeptides and uses thereof. Applicant: Enzymaster (Ningbo) Bio-Engineering Co., Ltd. The sequence listing filed with the application follows.

SEQUENCE LISTING (216 sequences)

SEQ ID NO: 1 - DNA, 1071 bp, Artificial sequence
  Engineered sequence
atgaacggtgaaacctcgcgtccgccggcgctgggttttagctctgataatattgctggtgcaagcccggaagtcgcacaggcactggtgaaacatagttccggccaagcgggtccgtatggcaccgatgaactgacggcccaggtgaaacgtaaattttgcgaaatcttcgaacgcgacgtcgaagtgttcctggttccgaccggtacggcagcaaacgcactgtgtctgtccgcaatgaccccgccgtggggtaatatttactgccatccggcgtcccacatcaacaatgatgaatgtggtgcgccggaatttttctcaaacggcgccaaactgatgaccgttgatggtccggcagctaaactggacattgtccgtctgcgcgaacgtacgcgcgaaaaagtgggtgatgttcataccacgcagccggcatgcgtctctattacccaagctacggaagtgggcagtatctataccctggatgaaattgaagccatcggtgacgtgtgcaaatcatcgagcctgggtctgcacatggatggctctcgttttgctaatgcgctggtgtccctgggctgttcaccggcagaaatgacctggaaagccggtgttgacgcactgagttttggtgcgacgaaaaacggcgttctggcggccgaagcaattgtcctgttcaatacctcgctggctacggaaatgagctatcgtcgcaaacgtgccggccacctgtctagtaaaatgcgctttctgagcgctcagatcgatgcgtacctgaccgatgacctgtggctgcgtaacgcccgcaaagcaaatgcagctgcgcagcgtctggcccaaggtctggaaggcctgggcggtgttgaagtcctgggcggtaccgaagcaaacattctgttctgtcgcctggattctgccatgatcgacgcactgctgaaagctggctttggtttctaccatgatcgttggggtccgaacgtggttcgctttgttaccagcttcgctaccacggcggaagatgtggaccacctgctgaatcaggttcgcctggccgcagaccgtacgcaagaacgc

SEQ ID NO: 2 - protein, 357 aa, Pseudomonas putida [sequence omitted]

SEQ ID NO: 3 - DNA, 1128 bp, Artificial sequence
  Engineered sequence
atgaacggtgaaacctcgcgtccgccggcgctgggttttagctctgataatattgctggtgcaagcccggaagtcgcacaggcactcgttaagcacagttcgggccaggcgggtccctatggcaccgacgagttgacggcacaggtcaagcatagctccggccaagctggaccttatggtacagatgaactgactgctcaagttaaacgtaaattttgcgaaatcttcgaacgcgacgtcgaagtgttcctggttccgaccggtacggcagcaaacgcactgtgtctgtccgcaatgaccccgccgtggggtaatatttactgccatccggcgtcccacatcaacaatgatgaatgtggtgcgccggaatttttctcaaacggcgccaaactgatgaccgttgatggtccggcagctaaactggacattgtccgtctgcgcgaacgtacgcgcgaaaaagtgggtgatgttcataccacgcagccggcatgcgtctctattacccaagctacggaagtgggcagtatctataccctggatgaaattgaagccatcggtgacgtgtgcaaatcatcgagcctgggtctgcacatggatggctctcgttttgctaatgcgctggtgtccctgggctgttcaccggcagaaatgacctggaaagccggtgttgacgcactgagttttggtgcgacgaaaaacggcgttctggcggccgaagcaattgtcctgttcaatacctcgctggctacggaaatgagctatcgtcgcaaacgtgccggccacctgtctagtaaaatgcgctttctgagcgctcagatcgatgcgtacctgaccgatgacctgtggctgcgtaacgcccgcaaagcaaatgcagctgcgcagcgtctggcccaaggtctggaaggcctgggcggtgttgaagtcctgggcggtaccgaagcaaacattctgttctgtcgcctggattctgccatgatcgacgcactgctgaaagctggctttggtttctatcatgatcgttggggtccgaacgtggttcgctttgttaccagcttcgctaccacggcggaagatgtggaccacctgctgaatcaggttcgcctggccgcagaccgtacgcaagaacgc

SEQ ID NO: 4 - protein, 376 aa, Artificial sequence
  Engineered sequence
MNGETSRPPALGFSSDNIAGASPEVAQALVKHSSGQAGPYGTDELTAQVKHSSGQAGPYGTDELTAQVKRKFCEIFERDVEVFLVPTGTAANALCLSAMTPPWGNIYCHPASHINNDECGAPEFFSNGAKLMTVDGPAAKLDIVRLRERTREKVGDVHTTQPACVSITQATEVGSIYTLDEIEAIGDVCKSSSLGLHMDGSRFANALVSLGCSPAEMTWKAGVDALSFGATKNGVLAAEAIVLFNTSLATEMSYRRKRAGHLSSKMRFLSAQIDAYLTDDLWLRNARKANAAAQRLAQGLEGLGGVEVLGGTEANILFCRLDSAMIDALLKAGFGFYHDRWGPNVVRFVTSFATTAEDVDHLLNQVRLAADRTQER

SEQ ID NO: 5 - DNA, 1128 bp, Artificial sequence
  Engineered sequence
atgaacggtgaaacctcgcgtccgccggcgctgggttttagctctgataatattgctggtgcaagcccggaagtcgcacaggcactcgttaagcacagttcgggccagccgggtccctatggcaccgacgagttgacggcacaggtcaagcatagctccggccaagctggaccttatggtacagatgaactgactgctcaagttaaacgtaaattttgcgaaatcttcgaacgcgacgtcgaagtgttcctggttccgaccggtacggcagcaaacgcactgtgtctgtccgcaatgaccccgccgtggggtaatatttactgccatccggcgtcccacatcaacaatgatgaatgtggtgcgccggaatttttctcaaacggcgccaaactgatgaccgttgatggtccggcagctaaactggacattgtccgtctgcgcgaacgtacgcgcgaaaaagtgggtgatgttcataccacgcagccggcatgcgtctctattacccaagctacggaagtgggcagtatctataccctggatgaaattgaagccatcggtgacgtgtgcaaatcatcgagcctgggtctgcacatggatggctctcgttttgctaatgcgctggtgtccctgggctgttcaccggcagaaatgacctggaaagccggtgttgacgcactgagttttggtgcgacgaaaaacggcgttctggcggccgaagcaattgtcctgttcaatacctcgctggctacggaaatgagctatcgtcgcaaacgtgccggccacctgtctagtaaaatgcgctttctgagcgctcagatcgatgcgtacctgaccgatgacctgtggctgcgtaacgcccgcaaagcaaatgcagctgcgcagcgtctggcccaaggtctggaaggcctgggcggtgttgaagtcctgggcggtaccgaagcaaacattctgttctgtcgcctggattctgccatgatcgacgcactgctgaaagctggctttggtttctatcatgatcgttggggtccgaacgtggttcgctttgttaccagcttcgctaccacggcggaagatgtggaccacctgctgaatcaggttcgcctggccgcagaccgtacgcaagaacgc

SEQ ID NO: 6 - protein, 376 aa, Artificial sequence
  Engineered sequence
MNGETSRPPALGFSSDNIAGASPEVAQALVKHSSGQPGPYGTDELTAQVKHSSGQAGPYGTDELTAQVKRKFCEIFERDVEVFLVPTGTAANALCLSAMTPPWGNIYCHPASHINNDECGAPEFFSNGAKLMTVDGPAAKLDIVRLRERTREKVGDVHTTQPACVSITQATEVGSIYTLDEIEAIGDVCKSSSLGLHMDGSRFANALVSLGCSPAEMTWKAGVDALSFGATKNGVLAAEAIVLFNTSLATEMSYRRKRAGHLSSKMRFLSAQIDAYLTDDLWLRNARKANAAAQRLAQGLEGLGGVEVLGGTEANILFCRLDSAMIDALLKAGFGFYHDRWGPNVVRFVTSFATTAEDVDHLLNQVRLAADRTQER

SEQ ID NO: 7 - DNA, 1128 bp, Artificial sequence
  Engineered sequence
atgaacggtgaaacctcgcgtccgccggcgctgggttttagctctgataatattgctggtgcaagcccggaagtcgcacaggcactcgttaagcacagttcgggccaggcgtttccctatggcaccgacgagttgacggcacaggtcaagcatagctccggccaagctggaccttatggtacagatgaactgactgctcaagttaaacgtaaattttgcgaaatcttcgaacgcgacgtcgaagtgttcctggttccgaccggtacggcagcaaacgcactgtgtctgtccgcaatgaccccgccgtggggtaatatttactgccatccggcgtcccacatcaacaatgatgaatgtggtgcgccggaatttttctcaaacggcgccaaactgatgaccgttgatggtccggcagctaaactggacattgtccgtctgcgcgaacgtacgcgcgaaaaagtgggtgatgttcataccacgcagccggcatgcgtctctattacccaagctacggaagtgggcagtatctataccctggatgaaattgaagccatcggtgacgtgtgcaaatcatcgagcctgggtctgcacatggatggctctcgttttgctaatgcgctggtgtccctgggctgttcaccggcagaaatgacctggaaagccggtgttgacgcactgagttttggtgcgacgaaaaacggcgttctggcggccgaagcaattgtcctgttcaatacctcgctggctacggaaatgagctatcgtcgcaaacgtgccggccacctgtctagtaaaatgcgctttctgagcgctcagatcgatgcgtacctgaccgatgacctgtggctgcgtaacgcccgcaaagcaaatgcagctgcgcagcgtctggcccaaggtctggaaggcctgggcggtgttgaagtcctgggcggtaccgaagcaaacattctgttctgtcgcctggattctgccatgatcgacgcactgctgaaagctggctttggtttctatcatgatcgttggggtccgaacgtggttcgctttgttaccagcttcgctaccacggcggaagatgtggaccacctgctgaatcaggttcgcctggccgcagaccgtacgcaagaacgc

SEQ ID NO: 8 - protein, 376 aa, Artificial sequence
  Engineered sequence
MNGETSRPPALGFSSDNIAGASPEVAQALVKHSSGQAFPYGTDELTAQVKHSSGQAGPYGTDELTAQVKRKFCEIFERDVEVFLVPTGTAANALCLSAMTPPWGNIYCHPASHINNDECGAPEFFSNGAKLMTVDGPAAKLDIVRLRERTREKVGDVHTTQPACVSITQATEVGSIYTLDEIEAIGDVCKSSSLGLHMDGSRFANALVSLGCSPAEMTWKAGVDALSFGATKNGVLAAEAIVLFNTSLATEMSYRRKRAGHLSSKMRFLSAQIDAYLTDDLWLRNARKANAAAQRLAQGLEGLGGVEVLGGTEANILFCRLDSAMIDALLKAGFGFYHDRWGPNVVRFVTSFATTAEDVDHLLNQVRLAADRTQER

SEQ ID NO: 9 - DNA, 1128 bp, Artificial sequence
  Engineered sequence
atgaacggtgaaacctcgcgtccgccggcgctgggttttagctctgataatattgctggtgcaagcccggaagtcgcacaggcactcgttaagcacagttcgggccaggcgtatccctatggcaccgacgagttgacggcacaggtcaagcatagctccggccaagctggaccttatggtacagatgaactgactgctcaagttaaacgtaaattttgcgaaatcttcgaacgcgacgtcgaagtgttcctggttccgaccggtacggcagcaaacgcactgtgtctgtccgcaatgaccccgccgtggggtaatatttactgccatccggcgtcccacatcaacaatgatgaatgtggtgcgccggaatttttctcaaacggcgccaaactgatgaccgttgatggtccggcagctaaactggacattgtccgtctgcgcgaacgtacgcgcgaaaaagtgggtgatgttcataccacgcagccggcatgcgtctctattacccaagctacggaagtgggcagtatctataccctggatgaaattgaagccatcggtgacgtgtgcaaatcatcgagcctgggtctgcacatggatggctctcgttttgctaatgcgctggtgtccctgggctgttcaccggcagaaatgacctggaaagccggtgttgacgcactgagttttggtgcgacgaaaaacggcgttctggcggccgaagcaattgtcctgttcaatacctcgctggctacggaaatgagctatcgtcgcaaacgtgccggccacctgtctagtaaaatgcgctttctgagcgctcagatcgatgcgtacctgaccgatgacctgtggctgcgtaacgcccgcaaagcaaatgcagctgcgcagcgtctggcccaaggtctggaaggcctgggcggtgttgaagtcctgggcggtaccgaagcaaacattctgttctgtcgcctggattctgccatgatcgacgcactgctgaaagctggctttggtttctatcatgatcgttggggtccgaacgtggttcgctttgttaccagcttcgctaccacggcggaagatgtggaccacctgctgaatcaggttcgcctggccgcagaccgtacgcaagaacgc

SEQ ID NO: 10 - protein, 376 aa, Artificial sequence
  Engineered sequence
MNGETSRPPALGFSSDNIAGASPEVAQALVKHSSGQAYPYGTDELTAQVKHSSGQAGPYGTDELTAQVKRKFCEIFERDVEVFLVPTGTAANALCLSAMTPPWGNIYCHPASHINNDECGAPEFFSNGAKLMTVDGPAAKLDIVRLRERTREKVGDVHTTQPACVSITQATEVGSIYTLDEIEAIGDVCKSSSLGLHMDGSRFANALVSLGCSPAEMTWKAGVDALSFGATKNGVLAAEAIVLFNTSLATEMSYRRKRAGHLSSKMRFLSAQIDAYLTDDLWLRNARKANAAAQRLAQGLEGLGGVEVLGGTEANILFCRLDSAMIDALLKAGFGFYHDRWGPNVVRFVTSFATTAEDVDHLLNQVRLAADRTQER

SEQ ID NO: 11 - DNA, 1128 bp, Artificial sequence
  Engineered sequence
atgaacggtgaaacctcgcgtccgccggcgctgggttttagctctgataatattgctggtgcaagcccggaagtcgcacaggcactcgttaagcacagttcgggccaggcggatccctatggcaccgacgagttgacggcacaggtcaagcatagctccggccaagctggaccttatggtacagatgaactgactgctcaagttaaacgtaaattttgcgaaatcttcgaacgcgacgtcgaagtgttcctggttccgaccggtacggcagcaaacgcactgtgtctgtccgcaatgaccccgccgtggggtaatatttactgccatccggcgtcccacatcaacaatgatgaatgtggtgcgccggaatttttctcaaacggcgccaaactgatgaccgttgatggtccggcagctaaactggacattgtccgtctgcgcgaacgtacgcgcgaaaaagtgggtgatgttcataccacgcagccggcatgcgtctctattacccaagctacggaagtgggcagtatctataccctggatgaaattgaagccatcggtgacgtgtgcaaatcatcgagcctgggtctgcacatggatggctctcgttttgctaatgcgctggtgtccctgggctgttcaccggcagaaatgacctggaaagccggtgttgacgcactgagttttggtgcgacgaaaaacggcgttctggcggccgaagcaattgtcctgttcaatacctcgctggctacggaaatgagctatcgtcgcaaacgtgccggccacctgtctagtaaaatgcgctttctgagcgctcagatcgatgcgtacctgaccgatgacctgtggctgcgtaacgcccgcaaagcaaatgcagctgcgcagcgtctggcccaaggtctggaaggcctgggcggtgttgaagtcctgggcggtaccgaagcaaacattctgttctgtcgcctggattctgccatgatcgacgcactgctgaaagctggctttggtttctatcatgatcgttggggtccgaacgtggttcgctttgttaccagcttcgctaccacggcggaagatgtggaccacctgctgaatcaggttcgcctggccgcagaccgtacgcaagaacgc

SEQ ID NO: 12 - protein, 376 aa, Artificial sequence
  Engineered sequence
MNGETSRPPALGFSSDNIAGASPEVAQALVKHSSGQADPYGTDELTAQVKHSSGQAGPYGTDELTAQVKRKFCEIFERDVEVFLVPTGTAANALCLSAMTPPWGNIYCHPASHINNDECGAPEFFSNGAKLMTVDGPAAKLDIVRLRERTREKVGDVHTTQPACVSITQATEVGSIYTLDEIEAIGDVCKSSSLGLHMDGSRFANALVSLGCSPAEMTWKAGVDALSFGATKNGVLAAEAIVLFNTSLATEMSYRRKRAGHLSSKMRFLSAQIDAYLTDDLWLRNARKANAAAQRLAQGLEGLGGVEVLGGTEANILFCRLDSAMIDALLKAGFGFYHDRWGPNVVRFVTSFATTAEDVDHLLNQVRLAADRTQER

SEQ ID NO: 13 - DNA, 1128 bp, Artificial sequence
  Engineered sequence
atgaacggtgaaacctcgcgtccgccggcgctgggttttagctctgataatattgctggtgcaagcccggaagtcgcacaggcactcgttaagcacagttcgggccaggcgggtccctatggcccggacgagttgacggcacaggtcaagcatagctccggccaagctggaccttatggtacagatgaactgactgctcaagttaaacgtaaattttgcgaaatcttcgaacgcgacgtcgaagtgttcctggttccgaccggtacggcagcaaacgcactgtgtctgtccgcaatgaccccgccgtggggtaatatttactgccatccggcgtcccacatcaacaatgatgaatgtggtgcgccggaatttttctcaaacggcgccaaactgatgaccgttgatggtccggcagctaaactggacattgtccgtctgcgcgaacgtacgcgcgaaaaagtgggtgatgttcataccacgcagccggcatgcgtctctattacccaagctacggaagtgggcagtatctataccctggatgaaattgaagccatcggtgacgtgtgcaaatcatcgagcctgggtctgcacatggatggctctcgttttgctaatgcgctggtgtccctgggctgttcaccggcagaaatgacctggaaagccggtgttgacgcactgagttttggtgcgacgaaaaacggcgttctggcggccgaagcaattgtcctgttcaatacctcgctggctacggaaatgagctatcgtcgcaaacgtgccggccacctgtctagtaaaatgcgctttctgagcgctcagatcgatgcgtacctgaccgatgacctgtggctgcgtaacgcccgcaaagcaaatgcagctgcgcagcgtctggcccaaggtctggaaggcctgggcggtgttgaagtcctgggcggtaccgaagcaaacattctgttctgtcgcctggattctgccatgatcgacgcactgctgaaagctggctttggtttctatcatgatcgttggggtccgaacgtggttcgctttgttaccagcttcgctaccacggcggaagatgtggaccacctgctgaatcaggttcgcctggccgcagaccgtacgcaagaacgc

SEQ ID NO: 14 - protein, 376 aa, Artificial sequence
  Engineered sequence
MNGETSRPPALGFSSDNIAGASPEVAQALVKHSSGQAGPYGPDELTAQVKHSSGQAGPYGTDELTAQVKRKFCEIFERDVEVFLVPTGTAANALCLSAMTPPWGNIYCHPASHINNDECGAPEFFSNGAKLMTVDGPAAKLDIVRLRERTREKVGDVHTTQPACVSITQATEVGSIYTLDEIEAIGDVCKSSSLGLHMDGSRFANALVSLGCSPAEMTWKAGVDALSFGATKNGVLAAEAIVLFNTSLATEMSYRRKRAGHLSSKMRFLSAQIDAYLTDDLWLRNARKANAAAQRLAQGLEGLGGVEVLGGTEANILFCRLDSAMIDALLKAGFGFYHDRWGPNVVRFVTSFATTAEDVDHLLNQVRLAADRTQER

SEQ ID NO: 15 - DNA, 1128 bp, Artificial sequence
  Engineered sequence
atgaacggtgaaacctcgcgtccgccggcgctgggttttagctctgataatattgctggtgcaagcccggaagtcgcacaggcactcgttaagcacagttcgggccaggcgggtccctatggcaccgtggagttgacggcacaggtcaagcatagctccggccaagctggaccttatggtacagatgaactgactgctcaagttaaacgtaaattttgcgaaatcttcgaacgcgacgtcgaagtgttcctggttccgaccggtacggcagcaaacgcactgtgtctgtccgcaatgaccccgccgtggggtaatatttactgccatccggcgtcccacatcaacaatgatgaatgtggtgcgccggaatttttctcaaacggcgccaaactgatgaccgttgatggtccggcagctaaactggacattgtccgtctgcgcgaacgtacgcgcgaaaaagtgggtgatgttcataccacgcagccggcatgcgtctctattacccaagctacggaagtgggcagtatctataccctggatgaaattgaagccatcggtgacgtgtgcaaatcatcgagcctgggtctgcacatggatggctctcgttttgctaatgcgctggtgtccctgggctgttcaccggcagaaatgacctggaaagccggtgttgacgcactgagttttggtgcgacgaaaaacggcgttctggcggccgaagcaattgtcctgttcaatacctcgctggctacggaaatgagctatcgtcgcaaacgtgccggccacctgtctagtaaaatgcgctttctgagcgctcagatcgatgcgtacctgaccgatgacctgtggctgcgtaacgcccgcaaagcaaatgcagctgcgcagcgtctggcccaaggtctggaaggcctgggcggtgttgaagtcctgggcggtaccgaagcaaacattctgttctgtcgcctggattctgccatgatcgacgcactgctgaaagctggctttggtttctatcatgatcgttggggtccgaacgtggttcgctttgttaccagcttcgctaccacggcggaagatgtggaccacctgctgaatcaggttcgcctggccgcagaccgtacgcaagaacgc

SEQ ID NO: 16 - protein, 376 aa, Artificial sequence
  Engineered sequence
MNGETSRPPALGFSSDNIAGASPEVAQALVKHSSGQAGPYGTVELTAQVKHSSGQAGPYGTDELTAQVKRKFCEIFERDVEVFLVPTGTAANALCLSAMTPPWGNIYCHPASHINNDECGAPEFFSNGAKLMTVDGPAAKLDIVRLRERTREKVGDVHTTQPACVSITQATEVGSIYTLDEIEAIGDVCKSSSLGLHMDGSRFANALVSLGCSPAEMTWKAGVDALSFGATKNGVLAAEAIVLFNTSLATEMSYRRKRAGHLSSKMRFLSAQIDAYLTDDLWLRNARKANAAAQRLAQGLEGLGGVEVLGGTEANILFCRLDSAMIDALLKAGFGFYHDRWGPNVVRFVTSFATTAEDVDHLLNQVRLAADRTQER

SEQ ID NO: 17 - DNA, 1128 bp, Artificial sequence
  Engineered sequence
atgaacggtgaaacctcgcgtccgccggcgctgggttttagctctgataatattgctggtgcaagcccggaagtcgcacaggcactcgttaagcacagttcgggccaggcgggtccctatggcaccgacgagttgacggcacaggtcaagcatagctccggccaagctggaccttatggtacagatgaactgactgctcaagttaaacgtaaattttgcgaaatcttcgaacgcgacgtcgaagtgttcctggttccgaccggtacggcagcaaacgcactgtgtctgtccgcaatgaccccgccgtggggtaatatttactgccatccggcgtcccacatcaacaatgatgaatgtggtgcgccggaatttttctcaaacggcgccaaactgatgaccgttgatggtccggcagctaaactggacattgtccgtctgcgcgaacgtacgcgcgaaaaagtgggtgatgttcataccacgcagccggcatgcgtctctattacccaagctacggaagtgggcagtatctataccctggatgaaattgaagccatcggtgacgtgtgcaaatcatcgagcctgggtctgcacatggatggctctcgttttgctaatgcgctggtgtccctgggctgttcaccggcagaaatgacctggaaagccggtgttgacgcactgagttttggtgcgacgaaaaacggcgttctggcggccgaagcaattgtcctgttcaatacctcgctggctacggaaatgagctatcgtcgcaaacgtgccggccacctgtctagtaaaatgcgctttctgagcgctcagatcgatgcgtacctgaccgatgacctgtggctgcgtaacgcccgcaaagcaaatgcagctgcgcagcgtctggcccaaggtctggaaggcctgggcggtgttgaagtcctgtgcggtaccgaagcaaacattctgttctgtcgcctggattctgccatgatcgacgcactgctgaaagctggctttggtttctatcatgatcgttggggtccgaacgtggttcgctttgttaccagcttcgctaccacggcggaagatgtggaccacctgctgaatcaggttcgcctggccgcagaccgtacgcaagaacgc

SEQ ID NO: 18 - protein, 376 aa, Artificial sequence
  Engineered sequence
MNGETSRPPALGFSSDNIAGASPEVAQALVKHSSGQAGPYGTDELTAQVKHSSGQAGPYGTDELTAQVKRKFCEIFERDVEVFLVPTGTAANALCLSAMTPPWGNIYCHPASHINNDECGAPEFFSNGAKLMTVDGPAAKLDIVRLRERTREKVGDVHTTQPACVSITQATEVGSIYTLDEIEAIGDVCKSSSLGLHMDGSRFANALVSLGCSPAEMTWKAGVDALSFGATKNGVLAAEAIVLFNTSLATEMSYRRKRAGHLSSKMRFLSAQIDAYLTDDLWLRNARKANAAAQRLAQGLEGLGGVEVLCGTEANILFCRLDSAMIDALLKAGFGFYHDRWGPNVVRFVTSFATTAEDVDHLLNQVRLAADRTQER

SEQ ID NO: 19 - DNA, 1128 bp, Artificial sequence
  Engineered sequence
atgaacggtgaaacctcgcgtccgccggcgctgggttttagctctgataatattgctggtgcaagcccggaagtcgcacaggcactcgttaagcacagttcgggccaggcgggtccctatggcaccgacgagttgacggcacaggtcaagcatagctccggccaagctggaccttatggtacagatgaactgactgctcaagttaaacgtaaattttgcgaaatcttcgaacgcgacgtcgaagtgttcctggttccgaccggtacggcagcaaacgcactgtgtctgtccgcaatgaccccgccgtggggtaatatttactgccatccggcgtcccacatcaacaatgatgaatgtggtgcgccggaatttttctcaaacggcgccaaactgatgaccgttgatggtccggcagctaaactggacattgtccgtctgcgcgaacgtacgcgcgaaaaagtgggtgatgttcataccacgcagccggcatgcgtctctattacccaagctacggaagtgggcagtatctataccctggatgaaattgaagccatcggtgacgtgtgcaaatcatcgagcctgggtctgcacatggatggctctcgttttgctaatgcgctggtgtccctgggctgttcaccggcagaaatgacctggaaagccggtgttgacgcactgagttttggtgcgacgaaaaacggcgttctggcggccgaagcaattgtcctgttcaatacctcgctggctacggaaatgagctatcgtcgcaaacgtgccggccacctgtctagtaaaatgcgctttctgagcgctcagatcgatgcgtacctgaccgatgacctgtggctgcgtaacgcccgcaaagcaaatgcagctgcgcagcgtctggcccaaggtctggaaggcctgggcggtgttgaagtcctgggcggtaccgaagcaaacattctgttctgtcgcctggattctgccatgatcgaagcactgctgaaagctggctttggtttctatcatgatcgttggggtccgaacgtggttcgctttgttaccagcttcgctaccacggcggaagatgtggaccacctgctgaatcaggttcgcctggccgcagaccgtacgcaagaacgc

SEQ ID NO: 20 - protein, 376 aa, Artificial sequence
  Engineered sequence
MNGETSRPPALGFSSDNIAGASPEVAQALVKHSSGQAGPYGTDELTAQVKHSSGQAGPYGTDELTAQVKRKFCEIFERDVEVFLVPTGTAANALCLSAMTPPWGNIYCHPASHINNDECGAPEFFSNGAKLMTVDGPAAKLDIVRLRERTREKVGDVHTTQPACVSITQATEVGSIYTLDEIEAIGDVCKSSSLGLHMDGSRFANALVSLGCSPAEMTWKAGVDALSFGATKNGVLAAEAIVLFNTSLATEMSYRRKRAGHLSSKMRFLSAQIDAYLTDDLWLRNARKANAAAQRLAQGLEGLGGVEVLGGTEANILFCRLDSAMIEALLKAGFGFYHDRWGPNVVRFVTSFATTAEDVDHLLNQVRLAADRTQER

SEQ ID NO: 21 - DNA, 1128 bp, Artificial sequence
  Engineered sequence
atgaacggtgaaacctcgcgtccgccggcgctgggttttagctctgataatattgctggtgcaagcccggaagtcgcacaggcactcgttaagcacagttcgggccaggcgggtccctatggcaccgacgagttgacggcacaggtcaagcatagctccggccaagctggaccttatggtaacgatgaactgactgctcaagttaaacgtaaattttgcgaaatcttcgaacgcgacgtcgaagtgttcctggttccgaccggtacggcagcaaacgcactgtgtctgtccgcaatgaccccgccgtggggtaatatttactgccatccggcgtcccacatcaacaatgatgaatgtggtgcgccggaatttttctcaaacggcgccaaactgatgaccgttgatggtccggcagctaaactggacattgtccgtctgcgcgaacgtacgcgcgaaaaagtgggtgatgttcataccacgcagccggcatgcgtctctattacccaagctacggaagtgggcagtatctataccctggatgaaattgaagccatcggtgacgtgtgcaaatcatcgagcctgggtctgcacatggatggctctcgttttgctaatgcgctggtgtccctgggctgttcaccggcagaaatgacctggaaagccggtgttgacgcactgagttttggtgcgacgaaaaacggcgttctggcggccgaagcaattgtcctgttcaatacctcgctggctacggaaatgagctatcgtcgcaaacgtgccggccacctgtctagtaaaatgcgctttctgagcgctcagatcgatgcgtacctgaccgatgacctgtggctgcgtaacgcccgcaaagcaaatgcagctgcgcagcgtctggcccaaggtctggaaggcctgggcggtgttgaagtcctgggcggtaccgaagcaaacattctgttctgtcgcctggattctgccatgatcgacgcactgctgaaagctggctttggtttctatcatgatcgttggggtccgaacgtggttcgctttgttaccagcttcgctaccacggcggaagatgtggaccacctgctgaatcaggttcgcctggccgcagaccgtacgcaagaacgc

SEQ ID NO: 22 - protein, 376 aa, Artificial sequence
  Engineered sequence
MNGETSRPPALGFSSDNIAGASPEVAQALVKHSSGQAGPYGTDELTAQVKHSSGQAGPYGNDELTAQVKRKFCEIFERDVEVFLVPTGTAANALCLSAMTPPWGNIYCHPASHINNDECGAPEFFSNGAKLMTVDGPAAKLDIVRLRERTREKVGDVHTTQPACVSITQATEVGSIYTLDEIEAIGDVCKSSSLGLHMDGSRFANALVSLGCSPAEMTWKAGVDALSFGATKNGVLAAEAIVLFNTSLATEMSYRRKRAGHLSSKMRFLSAQIDAYLTDDLWLRNARKANAAAQRLAQGLEGLGGVEVLGGTEANILFCRLDSAMIDALLKAGFGFYHDRWGPNVVRFVTSFATTAEDVDHLLNQVRLAADRTQER

SEQ ID NO: 23 - DNA, 1128 bp, Artificial sequence
  Engineered sequence
atgaacggtgaaacctcgcgtccgccggcgctgggttttagctctgataatattgctggtgcaagcccggaagtcgcacaggcactcgttaagcacagttcgggccaggcgggtccctatggcaccgacgagttgacggcacaggtcaagcatagctccggccaagctggaccttatggtaaagatgaactgactgctcaagttaaacgtaaattttgcgaaatcttcgaacgcgacgtcgaagtgttcctggttccgaccggtacggcagcaaacgcactgtgtctgtccgcaatgaccccgccgtggggtaatatttactgccatccggcgtcccacatcaacaatgatgaatgtggtgcgccggaatttttctcaaacggcgccaaactgatgaccgttgatggtccggcagctaaactggacattgtccgtctgcgcgaacgtacgcgcgaaaaagtgggtgatgttcataccacgcagccggcatgcgtctctattacccaagctacggaagtgggcagtatctataccctggatgaaattgaagccatcggtgacgtgtgcaaatcatcgagcctgggtctgcacatggatggctctcgttttgctaatgcgctggtgtccctgggctgttcaccggcagaaatgacctggaaagccggtgttgacgcactgagttttggtgcgacgaaaaacggcgttctggcggccgaagcaattgtcctgttcaatacctcgctggctacggaaatgagctatcgtcgcaaacgtgccggccacctgtctagtaaaatgcgctttctgagcgctcagatcgatgcgtacctgaccgatgacctgtggctgcgtaacgcccgcaaagcaaatgcagctgcgcagcgtctggcccaaggtctggaaggcctgggcggtgttgaagtcctgggcggtaccgaagcaaacattctgttctgtcgcctggattctgccatgatcgacgcactgctgaaagctggctttggtttctatcatgatcgttggggtccgaacgtggttcgctttgttaccagcttcgctaccacggcggaagatgtggaccacctgctgaatcaggttcgcctggccgcagaccgtacgcaagaacgc

SEQ ID NO: 24 - protein, 376 aa, Artificial sequence
  Engineered sequence
MNGETSRPPALGFSSDNIAGASPEVAQALVKHSSGQAGPYGTDELTAQVKHSSGQAGPYGKDELTAQVKRKFCEIFERDVEVFLVPTGTAANALCLSAMTPPWGNIYCHPASHINNDECGAPEFFSNGAKLMTVDGPAAKLDIVRLRERTREKVGDVHTTQPACVSITQATEVGSIYTLDEIEAIGDVCKSSSLGLHMDGSRFANALVSLGCSPAEMTWKAGVDALSFGATKNGVLAAEAIVLFNTSLATEMSYRRKRAGHLSSKMRFLSAQIDAYLTDDLWLRNARKANAAAQRLAQGLEGLGGVEVLGGTEANILFCRLDSAMIDALLKAGFGFYHDRWGPNVVRFVTSFATTAEDVDHLLNQVRLAADRTQER

SEQ ID NO: 25 - DNA, 1128 bp, Artificial sequence
  Engineered sequence
atgaacggtgaaacctcgcgtccgccggcgctgggttttagctctgataatattgctggtgcaagcccggaagtcgcacaggcactcgttaagcacagttcgggccaggcgggtccctatggcaccgacgagttgacggcacaggtcaagcatagctccggccaagctggaccttatggtcatgatgaactgactgctcaagttaaacgtaaattttgcgaaatcttcgaacgcgacgtcgaagtgttcctggttccgaccggtacggcagcaaacgcactgtgtctgtccgcaatgaccccgccgtggggtaatatttactgccatccggcgtcccacatcaacaatgatgaatgtggtgcgccggaatttttctcaaacggcgccaaactgatgaccgttgatggtccggcagctaaactggacattgtccgtctgcgcgaacgtacgcgcgaaaaagtgggtgatgttcataccacgcagccggcatgcgtctctattacccaagctacggaagtgggcagtatctataccctggatgaaattgaagccatcggtgacgtgtgcaaatcatcgagcctgggtctgcacatggatggctctcgttttgctaatgcgctggtgtccctgggctgttcaccggcagaaatgacctggaaagccggtgttgacgcactgagttttggtgcgacgaaaaacggcgttctggcggccgaagcaattgtcctgttcaatacctcgctggctacggaaatgagctatcgtcgcaaacgtgccggccacctgtctagtaaaatgcgctttctgagcgctcagatcgatgcgtacctgaccgatgacctgtggctgcgtaacgcccgcaaagcaaatgcagctgcgcagcgtctggcccaaggtctggaaggcctgggcggtgttgaagtcctgggcggtaccgaagcaaacattctgttctgtcgcctggattctgccatgatcgacgcactgctgaaagctggctttggtttctatcatgatcgttggggtccgaacgtggttcgctttgttaccagcttcgctaccacggcggaagatgtggaccacctgctgaatcaggttcgcctggccgcagaccgtacgcaagaacgc

SEQ ID NO: 26 - protein, 376 aa, Artificial sequence
  Engineered sequence
MNGETSRPPALGFSSDNIAGASPEVAQALVKHSSGQAGPYGTDELTAQVKHSSGQAGPYGHDELTAQVKRKFCEIFERDVEVFLVPTGTAANALCLSAMTPPWGNIYCHPASHINNDECGAPEFFSNGAKLMTVDGPAAKLDIVRLRERTREKVGDVHTTQPACVSITQATEVGSIYTLDEIEAIGDVCKSSSLGLHMDGSRFANALVSLGCSPAEMTWKAGVDALSFGATKNGVLAAEAIVLFNTSLATEMSYRRKRAGHLSSKMRFLSAQIDAYLTDDLWLRNARKANAAAQRLAQGLEGLGGVEVLGGTEANILFCRLDSAMIDALLKAGFGFYHDRWGPNVVRFVTSFATTAEDVDHLLNQVRLAADRTQER

SEQ ID NO: 27 - DNA, 1128 bp, Artificial sequence
  Engineered sequence
atgaacggtgaaacctcgcgtccgccggcgctgggttttagctctgataattatgctggtgcaagcccggaagtcgcacaggcactcgttaagcacagttcgggccaggcgggtccctatggcaccgacgagttgacggcacaggtcaagcatagctccggccaagctggaccttatggtacagatgaactgactgctcaagttaaacgtaaattttgcgaaatcttcgaacgcgacgtcgaagtgttcctggttccgaccggtacggcagcaaacgcactgtgtctgtccgcaatgaccccgccgtggggtaatatttactgccatccggcgtcccacatcaacaatgatgaatgtggtgcgccggaatttttctcaaacggcgccaaactgatgaccgttgatggtccggcagctaaactggacattgtccgtctgcgcgaacgtacgcgcgaaaaagtgggtgatgttcataccacgcagccggcatgcgtctctattacccaagctacggaagtgggcagtatctataccctggatgaaattgaagccatcggtgacgtgtgcaaatcatcgagcctgggtctgcacatggatggctctcgttttgctaatgcgctggtgtccctgggctgttcaccggcagaaatgacctggaaagccggtgttgacgcactgagttttggtgcgacgaaaaacggcgttctggcggccgaagcaattgtcctgttcaatacctcgctggctacggaaatgagctatcgtcgcaaacgtgccggccacctgtctagtaaaatgcgctttctgagcgctcagatcgatgcgtacctgaccgatgacctgtggctgcgtaacgcccgcaaagcaaatgcagctgcgcagcgtctggcccaaggtctggaaggcctgggcggtgttgaagtcctgggcggtaccgaagcaaacattctgttctgtcgcctggattctgccatgatcgacgcactgctgaaagctggctttggtttctatcatgatcgttggggtccgaacgtggttcgctttgttaccagcttcgctaccacggcggaagatgtggaccacctgctgaatcaggttcgcctggccgcagaccgtacgcaagaacgc

SEQ ID NO: 28 - protein, 376 aa, Artificial sequence
  Engineered sequence
MNGETSRPPALGFSSDNYAGASPEVAQALVKHSSGQAGPYGTDELTAQVKHSSGQAGPYGTDELTAQVKRKFCEIFERDVEVFLVPTGTAANALCLSAMTPPWGNIYCHPASHINNDECGAPEFFSNGAKLMTVDGPAAKLDIVRLRERTREKVGDVHTTQPACVSITQATEVGSIYTLDEIEAIGDVCKSSSLGLHMDGSRFANALVSLGCSPAEMTWKAGVDALSFGATKNGVLAAEAIVLFNTSLATEMSYRRKRAGHLSSKMRFLSAQIDAYLTDDLWLRNARKANAAAQRLAQGLEGLGGVEVLGGTEANILFCRLDSAMIDALLKAGFGFYHDRWGPNVVRFVTSFATTAEDVDHLLNQVRLAADRTQER

SEQ ID NO: 29 - DNA, 1128 bp, Artificial sequence
  Engineered sequence
atgaacggtgaaacctcgcgtccgccggcgctgggttttagctctgataattgggctggtgcaagcccggaagtcgcacaggcactcgttaagcacagttcgggccaggcgggtccctatggcaccgacgagttgacggcacaggtcaagcatagctccggccaagctggaccttatggtacagatgaactgactgctcaagttaaacgtaaattttgcgaaatcttcgaacgcgacgtcgaagtgttcctggttccgaccggtacggcagcaaacgcactgtgtctgtccgcaatgaccccgccgtggggtaatatttactgccatccggcgtcccacatcaacaatgatgaatgtggtgcgccggaatttttctcaaacggcgccaaactgatgaccgttgatggtccggcagctaaactggacattgtccgtctgcgcgaacgtacgcgcgaaaaagtgggtgatgttcataccacgcagccggcatgcgtctctattacccaagctacggaagtgggcagtatctataccctggatgaaattgaagccatcggtgacgtgtgcaaatcatcgagcctgggtctgcacatggatggctctcgttttgctaatgcgctggtgtccctgggctgttcaccggcagaaatgacctggaaagccggtgttgacgcactgagttttggtgcgacgaaaaacggcgttctggcggccgaagcaattgtcctgttcaatacctcgctggctacggaaatgagctatcgtcgcaaacgtgccggccacctgtctagtaaaatgcgctttctgagcgctcagatcgatgcgtacctgaccgatgacctgtggctgcgtaacgcccgcaaagcaaatgcagctgcgcagcgtctggcccaaggtctggaaggcctgggcggtgttgaagtcctgggcggtaccgaagcaaacattctgttctgtcgcctggattctgccatgatcgacgcactgctgaaagctggctttggtttctatcatgatcgttggggtccgaacgtggttcgctttgttaccagcttcgctaccacggcggaagatgtggaccacctgctgaatcaggttcgcctggccgcagaccgtacgcaagaacgc

SEQ ID NO: 30 - protein, 376 aa, Artificial sequence
  Engineered sequence
MNGETSRPPALGFSSDNWAGASPEVAQALVKHSSGQAGPYGTDELTAQVKHSSGQAGPYGTDELTAQVKRKFCEIFERDVEVFLVPTGTAANALCLSAMTPPWGNIYCHPASHINNDECGAPEFFSNGAKLMTVDGPAAKLDIVRLRERTREKVGDVHTTQPACVSITQATEVGSIYTLDEIEAIGDVCKSSSLGLHMDGSRFANALVSLGCSPAEMTWKAGVDALSFGATKNGVLAAEAIVLFNTSLATEMSYRRKRAGHLSSKMRFLSAQIDAYLTDDLWLRNARKANAAAQRLAQGLEGLGGVEVLGGTEANILFCRLDSAMIDALLKAGFGFYHDRWGPNVVRFVTSFATTAEDVDHLLNQVRLAADRTQER

SEQ ID NO: 31 - DNA, 1128 bp, Artificial sequence
  Engineered sequence
atgaacggtgaaacctcgcgtccgccggcgctgggttttagctctgataatattgctggtgcaagcccggaagtcgcacaggcactcgttaagcacagttcgggccaggcgggtccctatggcaccgacgagttgacggcacaggtcaagcatagctccggccaagctggaccttatggtacagatgaactgactgctcaagttaaacgtaaattttgcgaaatcttcgaacgcgacgtcgaagtgttcctggttccgaccggtacggcagcaaacgcactgtgtctgtccgcaatgaccccgccgtggggtaatatttactgccatccggcgtcccacatcaacaatgatgaatgtggtgcgccggaatttttctcaaacggcgccaaactgatgaccgttgatggtccggcagctaaactggacattgtccgtctgcgcgaacgtacgcgcgaaaaagtgggtgatgttcataccacgcagccggcatgcgtctctattacccaagctacggaagtgggcagtatctataccctggatgaaattgaagccatcggtgacgtgtgcaaatcatcgagcctgggtctgcacatggatggctctcgttttgctaatgcgctggtgtccctgggctgttcaccggcagaaatgacctggaaagccggtgttgacgcactgagttttggtgcgacgaaaaacggcgttctggcggccgaagcaattgtcctgttcaatacctcgctggctacggaaatgagctatcgtcgcaaacgtgccggccacctggtgagtaaaatgcgctttctgagcgctcagatcgatgcgtacctgaccgatgacctgtggctgcgtaacgcccgcaaagcaaatgcagctgcgcagcgtctggcccaaggtctggaaggcctgggcggtgttgaagtcctgggcggtaccgaagcaaacattctgttctgtcgcctggattctgccatgatcgacgcactgctgaaagctggctttggtttctatcatgatcgttggggtccgaacgtggttcgctttgttaccagcttcgctaccacggcggaagatgtggaccacctgctgaatcaggttcgcctggccgcagaccgtacgcaagaacgc

SEQ ID NO: 32 - protein, 376 aa, Artificial sequence
  Engineered sequence
MNGETSRPPALGFSSDNIAGASPEVAQALVKHSSGQAGPYGTDELTAQVKHSSGQAGPYGTDELTAQVKRKFCEIFERDVEVFLVPTGTAANALCLSAMTPPWGNIYCHPASHINNDECGAPEFFSNGAKLMTVDGPAAKLDIVRLRERTREKVGDVHTTQPACVSITQATEVGSIYTLDEIEAIGDVCKSSSLGLHMDGSRFANALVSLGCSPAEMTWKAGVDALSFGATKNGVLAAEAIVLFNTSLATEMSYRRKRAGHLVSKMRFLSAQIDAYLTDDLWLRNARKANAAAQRLAQGLEGLGGVEVLGGTEANILFCRLDSAMIDALLKAGFGFYHDRWGPNVVRFVTSFATTAEDVDHLLNQVRLAADRTQER

SEQ ID NO: 33 - DNA, 1128 bp, Artificial sequence
  Engineered sequence
atgaacggtgaaacctcgcgtccgccggcgctgggttttagctctgataatattgctggtgcaagcccggaagtcgcacaggcactcgttaagcacagttcgggccaggcgggtccctatggcaccgacgagttgacggcacaggtcaagcatagctccggccaagctggaccttatggtacagatgaactgactgctcaagttaaacgtaaattttgcgaaatcttcgaacgcgacgtcgaagtgttcctggttccgaccggtacggcagcaaacgcactgtgtctgtccgcaatgaccccgccgtggggtaatatttactgccatccggcgtcccacatcaacaatgatgaatgtggtgcgccggaatttttctcaaacggcgccaaactgatgaccgttgatggtccggcagctaaactggacattgtccgtctgcgcgaacgtacgcgcgaaaaagtgggtgatgttcataccacgcagccggcatgcgtctctattacccaagctacggaagtgggcagtatctataccctggatgaaattgaagccatcggtgacgtgtgcaaatcatcgagcctgggtctgcacatggatggctctcgttttgctaatgcgctggtgtccctgggctgttcaccggcagaaatgacctggaaagccggtgttgacgcactgagttttggtgcgacgaaaaacggcgttctggcggccgaagcaattgtcctgttcaatacctcgctggctacggaaatgagctatcgtcgcaaacgtgccggccacctgcatagtaaaatgcgctttctgagcgctcagatcgatgcgtacctgaccgatgacctgtggctgcgtaacgcccgcaaagcaaatgcagctgcgcagcgtctggcccaaggtctggaaggcctgggcggtgttgaagtcctgggcggtaccgaagcaaacattctgttctgtcgcctggattctgccatgatcgacgcactgctgaaagctggctttggtttctatcatgatcgttggggtccgaacgtggttcgctttgttaccagcttcgctaccacggcggaagatgtggaccacctgctgaatcaggttcgcctggccgcagaccgtacgcaagaacgc

SEQ ID NO: 34 - protein, 376 aa, Artificial sequence
  Engineered sequence
MNGETSRPPALGFSSDNIAGASPEVAQALVKHSSGQAGPYGTDELTAQVKHSSGQAGPYGTDELTAQVKRKFCEIFERDVEVFLVPTGTAANALCLSAMTPPWGNIYCHPASHINNDECGAPEFFSNGAKLMTVDGPAAKLDIVRLRERTREKVGDVHTTQPACVSITQATEVGSIYTLDEIEAIGDVCKSSSLGLHMDGSRFANALVSLGCSPAEMTWKAGVDALSFGATKNGVLAAEAIVLFNTSLATEMSYRRKRAGHLHSKMRFLSAQIDAYLTDDLWLRNARKANAAAQRLAQGLEGLGGVEVLGGTEANILFCRLDSAMIDALLKAGFGFYHDRWGPNVVRFVTSFATTAEDVDHLLNQVRLAADRTQER

SEQ ID NO: 35 - DNA, 1128 bp, Artificial sequence
  Engineered sequence
atgaacggtgaaacctcgcgtccgccggcgctgggttttagctctgataatattgctggtgcaagcccggaagtcgcacaggcactcgttaagcacagttcgggccaggcgggtccctatggcaccgacgagttgacggcacaggtcaagcatagctccggccaagctggaccttatggtacagatgaactgactgctcaagttaaacgtaaattttgcgaaatcttcgaacgcgacgtcgaagtgttcctggttccgaccggtacggcagcaaacgcactgtgtctgtccgcaatgaccccgccgtggggtaatatttactgccatccggcgtcccacatcaacaatgatgaatgtggtgcgccggaatttttctcaaacggcgccaaactgatgaccgttgatggtccggcagctaaactggacattgtccgtctgcgcgaacgtacgcgcgaaaaagtgggtgatgttcataccacgcagccggcatgcgtctctattacccaagctacggaagtgggcagtatctataccctggatgaaattgaagccatcggtgacgtgtgcaaatcatcgagcctgggtctgcacatggatggctctcgttttgctaatgcgctggtgtccctgggctgttcaccggcagaaatgacctggaaagccggtgttgacgcactgagttttggtgcgacgaaaaacggcgttctggcggccgaagcaattgtcctgttcaatacctcgctggctacggaaatgagctatcgtcgcaaacgtgccggccacctgaccagtaaaatgcgctttctgagcgctcagatcgatgcgtacctgaccgatgacctgtggctgcgtaacgcccgcaaagcaaatgcagctgcgcagcgtctggcccaaggtctggaaggcctgggcggtgttgaagtcctgggcggtaccgaagcaaacattctgttctgtcgcctggattctgccatgatcgacgcactgctgaaagctggctttggtttctatcatgatcgttggggtccgaacgtggttcgctttgttaccagcttcgctaccacggcggaagatgtggaccacctgctgaatcaggttcgcctggccgcagaccgtacgcaagaacgc

SEQ ID NO: 36 - protein, 376 aa, Artificial sequence
  Engineered sequence
MNGETSRPPALGFSSDNIAGASPEVAQALVKHSSGQAGPYGTDELTAQVKHSSGQAGPYGTDELTAQVKRKFCEIFERDVEVFLVPTGTAANALCLSAMTPPWGNIYCHPASHINNDECGAPEFFSNGAKLMTVDGPAAKLDIVRLRERTREKVGDVHTTQPACVSITQATEVGSIYTLDEIEAIGDVCKSSSLGLHMDGSRFANALVSLGCSPAEMTWKAGVDALSFGATKNGVLAAEAIVLFNTSLATEMSYRRKRAGHLTSKMRFLSAQIDAYLTDDLWLRNARKANAAAQRLAQGLEGLGGVEVLGGTEANILFCRLDSAMIDALLKAGFGFYHDRWGPNVVRFVTSFATTAEDVDHLLNQVRLAADRTQER

SEQ ID NO: 37 - DNA, 1128 bp, Artificial sequence
  Engineered sequence
atgaacggtgaaacctcgcgtccgccggcgctgggttttagctctgataatattgctggtgcaagcccggaagtcgcacaggcactcgttaagcacagttcgggccaggcgggtccctatggcaccgacgagttgacggcacaggtcaagcatagctccggccaagctggaccttatggtacagatgaactgactgctcaagttaaacgtaaattttgcgaaatcttcgaacgcgacgtcgaagtgttcctggttccgaccggtacggcagcaaacgcactgtgtctgtccgcaatgaccccgccgtggggtaatatttactgccatccggcgtcccacatcaacaatgatgaatgtggtgcgccggaatttttctcaaacggcgccaaactgatgaccgttgatggtccggcagctaaactggacattgtccgtctgcgcgaacgtacgcgcgaaaaagtgggtgatgttcataccacgcagccggcatgcgtctctattacccaagctacggaagtgggcagtatctataccctggatgaaattgaagccatcggtgacgtgtgcaaatcatcgagcctgggtctgcacatggatggctctcgttttgctaatgcgctggtgtccctgggctgttcaccggcagaaatgacctggaaagccggtgttgacgcactgagttttggtgcgacgaaaaacggcgttctggcggccgaagcaattgtcctgttcaatacctcgctggctacggaaatgagctatcgtcgcaaacgtgccggccacctgtctagtaaaatgcgctttctgagcgctcagatcgatgcgtacctgaccgatgacctgtggctgcgtaacgcccgcaaagcaaatgcagctgcgcagcgtctggcccaaggtctggaaggcctgggcggtgttgaagtcctgggcggtaccgaagcaaacattctgttctgtcgcctggattctgccatgatcgacgcactgctgaaagctggctttggtttcgtgcatgatcgttggggtccgaacgtggttcgctttgttaccagcttcgctaccacggcggaagatgtggaccacctgctgaatcaggttcgcctggccgcagaccgtacgcaagaacgc

SEQ ID NO: 38 - protein, 376 aa, Artificial sequence
  Engineered sequence
MNGETSRPPALGFSSDNIAGASPEVAQALVKHSSGQAGPYGTDELTAQVKHSSGQAGPYGTDELTAQVKRKFCEIFERDVEVFLVPTGTAANALCLSAMTPPWGNIYCHPASHINNDECGAPEFFSNGAKLMTVDGPAAKLDIVRLRERTREKVGDVHTTQPACVSITQATEVGSIYTLDEIEAIGDVCKSSSLGLHMDGSRFANALVSLGCSPAEMTWKAGVDALSFGATKNGVLAAEAIVLFNTSLATEMSYRRKRAGHLSSKMRFLSAQIDAYLTDDLWLRNARKANAAAQRLAQGLEGLGGVEVLGGTEANILFCRLDSAMIDALLKAGFGFVHDRWGPNVVRFVTSFATTAEDVDHLLNQVRLAADRTQER

SEQ ID NO: 39 - DNA, 1128 bp, Artificial sequence
  Engineered sequence
atgaacggtgaaacctcgcgtccgccggcgctgggttttagctctgataatattgctggtgcaagcccggaagtcgcacaggcactcgttaagcacagttcgggccaggcgggtccctatggcaccgacgagttgacggcacaggtcaagcatagctccggccaagctggaccttatggtacagatgaactgactgctcaagttaaacgtaaattttgcgaaatcttcgaacgcgacgtcgaagtgttcctggttccgaccggtacggcagcaaacgcactgtgtctgtccgcaatgaccccgccgtggggtaatatttactgccatccggcgtcccacatcaacaatgatgaatgtggtgcgccggaatttttctcaaacggcgccaaactgatgaccgttgatggtccggcagctaaactggacattgtccgtctgcgcgaacgtacgcgcgaaaaagtgggtgatgttcataccacgcagccggcatgcgtctctattacccaagctacggaagtgggcagtatctataccctggatgaaattgaagccatcggtgacgtgtgcaaatcatcgagcctgggtctgcacatggatggctctcgttttgctaatgcgctggtgtccctgggctgttcaccggcagaaatgacctggaaagccggtgttgacgcactgagttttggtgcgacgaaaaacggcgttctggcggccgaagcaattgtcctgttcaatacctcgctggctacggaaatgagctatcgtcgcaaacgtgccggccacctgtctagtaaaatgcgctttctgagcgctcagatcgatgcgtacctgaccgatgacctgtggctgcgtaacgcccgcaaagcaaatgcagctgcgcagcgtctggcccaaggtctggaaggcctgggcggtgttgaagtcctgggcggtaccgaagcaaacattctgttctgtcgcctggattctgccatgatcgacgcactgctgaaagctggctttggtttcgggcatgatcgttggggtccgaacgtggttcgctttgttaccagcttcgctaccacggcggaagatgtggaccacctgctgaatcaggttcgcctggccgcagaccgtacgcaagaacgc

SEQ ID NO: 40 - protein, 376 aa, Artificial sequence
  Engineered sequence
MNGETSRPPALGFSSDNIAGASPEVAQALVKHSSGQAGPYGTDELTAQVKHSSGQAGPYGTDELTAQVKRKFCEIFERDVEVFLVPTGTAANALCLSAMTPPWGNIYCHPASHINNDECGAPEFFSNGAKLMTVDGPAAKLDIVRLRERTREKVGDVHTTQPACVSITQATEVGSIYTLDEIEAIGDVCKSSSLGLHMDGSRFANALVSLGCSPAEMTWKAGVDALSFGATKNGVLAAEAIVLFNTSLATEMSYRRKRAGHLSSKMRFLSAQIDAYLTDDLWLRNARKANAAAQRLAQGLEGLGGVEVLGGTEANILFCRLDSAMIDALLKAGFGFGHDRWGPNVVRFVTSFATTAEDVDHLLNQVRLAADRTQER

SEQ ID NO: 41 - DNA, 1128 bp, Artificial sequence
  Engineered sequence
atgaacggtgaaacctcgcgtccgccggcgctgggttttagctctgataatattgctggtgcaagcccggaagtcgcacaggcactcgttaagcacagttcgggccaggcgggtccctatggcaccgacgagttgacggcacaggtcaagcatagctccggccaagctggaccttatggtacagatgaactgactgctcaagttaaacgtaaattttgcgaaatcttcgaacgcgacgtcgaagtgttcctggttccgaccggtacggcagcaaacgcactgtgtctgtccgcaatgaccccgccgtggggtaatatttactgccatccggcgtcccacatcaacaatgatgaatgtggtgcgccggaatttttctcaaacggcgccaaactgatgaccgttgatggtccggcagctaaactggacattgtccgtctgcgcgaacgtacgcgcgaaaaagtgggtgatgttcataccacgcagccggcatgcgtctctattacccaagctacggaagtgggcagtatctataccctggatgaaattgaagccatcggtgacgtgtgcaaatcatcgagcctgggtctgcacatggatggctctcgttttgctaatgcgctggtgtccctgggctgttcaccggcagaaatgacctggaaagccggtgttgacgcactgagttttggtgcgacgaaaaacggcgttctggcggccgaagcaattgtcctgttcaatacctcgctggctacggaaatgagctatcgtcgcaaacgtgccggccacctgtctagtaaaatgcgctttctgagcgctcagatcgatgcgtacctgaccgatgacctgtggctgcgtaacgcccgcaaagcaaatgcagctgcgcagcgtctggcccaaggtctggaaggcctgggcggtgttgaagtcctgggcggtaccgaagcaaacattctgttctgtcgcctggattctgccatgatcgacgcactgctgaaagctggctttggtttcattcatgatcgttggggtccgaacgtggttcgctttgttaccagcttcgctaccacggcggaagatgtggaccacctgctgaatcaggttcgcctggccgcagaccgtacgcaagaacgc

SEQ ID NO: 42 - protein, 376 aa, Artificial sequence
  Engineered sequence
MNGETSRPPALGFSSDNIAGASPEVAQALVKHSSGQAGPYGTDELTAQVKHSSGQAGPYGTDELTAQVKRKFCEIFERDVEVFLVPTGTAANALCLSAMTPPWGNIYCHPASHINNDECGAPEFFSNGAKLMTVDGPAAKLDIVRLRERTREKVGDVHTTQPACVSITQATEVGSIYTLDEIEAIGDVCKSSSLGLHMDGSRFANALVSLGCSPAEMTWKAGVDALSFGATKNGVLAAEAIVLFNTSLATEMSYRRKRAGHLSSKMRFLSAQIDAYLTDDLWLRNARKANAAAQRLAQGLEGLGGVEVLGGTEANILFCRLDSAMIDALLKAGFGFIHDRWGPNVVRFVTSFATTAEDVDHLLNQVRLAADRTQER

SEQ ID NO: 43 - DNA, 1128 bp, Artificial sequence
  Engineered sequence
atgaacggtgaaacctcgcgtccgccggcgctgggttttagctctgataatattgctggtgcaagcccggaagtcgcacaggcactcgttaagcacagttcgggccaggcgggtccctatggcaccgacgagttgacggcacaggtcaagcatagctccggccaagctggaccttatggtacagatgaactgactgctcaagttaaacgtaaattttgcgaaatcttcgaacgcgacgtcgaagtgttcctggttccgaccggtacggcagcaaacgcactgtgtctgtccgcaatgaccccgccgtggggtaatatttactgccatccggcgtcccacatcaacaatgatgaatgtggtgcgccggaatttttctcaaacggcgccaaactgatgaccgttgatggtccggcagctaaactggacattgtccgtctgcgcgaacgtacgcgcgaaaaagtgggtgatgttcataccacgcagccggcatgcgtctctattacccaagctacggaagtgggcagtatctataccctggatgaaattgaagccatcggtgacgtgtgcaaatcatcgagcctgggtctgcacatggatggctctcgttttgctaatgcgctggtgtccctgggctgttcaccggcagaaatgacctggaaagccggtgttgacgcactgagttttggtgcgacgaaaaacggcgttctggcggccgaagcaattgtcctgttcaatacctcgctggctacggaaatgagctatcgtcgcaaacgtgccggccacctgtctagtaaatatcgctttctgagcgctcagatcgatgcgtacctgaccgatgacctgtggctgcgtaacgcccgcaaagcaaatgcagctgcgcagcgtctggcccaaggtctggaaggcctgggcggtgttgaagtcctgggcggtaccgaagcaaacattctgttctgtcgcctggattctgccatgatcgacgcactgctgaaagctggctttggtttctatcatgatcgttggggtccgaacgtggttcgctttgttaccagcttcgctaccacggcggaagatgtggaccacctgctgaatcaggttcgcctggccgcagaccgtacgcaagaacgc

SEQ ID NO: 44 - protein, 376 aa, Artificial sequence
  Engineered sequence
MNGETSRPPALGFSSDNIAGASPEVAQALVKHSSGQAGPYGTDELTAQVKHSSGQAGPYGTDELTAQVKRKFCEIFERDVEVFLVPTGTAANALCLSAMTPPWGNIYCHPASHINNDECGAPEFFSNGAKLMTVDGPAAKLDIVRLRERTREKVGDVHTTQPACVSITQATEVGSIYTLDEIEAIGDVCKSSSLGLHMDGSRFANALVSLGCSPAEMTWKAGVDALSFGATKNGVLAAEAIVLFNTSLATEMSYRRKRAGHLSSKYRFLSAQIDAYLTDDLWLRNARKANAAAQRLAQGLEGLGGVEVLGGTEANILFCRLDSAMIDALLKAGFGFYHDRWGPNVVRFVTSFATTAEDVDHLLNQVRLAADRTQER

SEQ ID NO: 45 - DNA, 1128 bp, Artificial sequence
  Engineered sequence
atgaacggtgaaacctcgcgtccgccggcgctgggttttagctctgataatattgctggtgcaagcccggaagtcgcacaggcactcgttaagcacagttcgggccaggcgggtccctatggcaccgacgagttgacggcacaggtcaagcatagctccggccaagctgatccttatggtacagatgaactgactgctcaagttaaacgtaaattttgcgaaatcttcgaacgcgacgtcgaagtgttcctggttccgaccggtacggcagcaaacgcactgtgtctgtccgcaatgaccccgccgtggggtaatatttactgccatccggcgtcccacatcaacaatgatgaatgtggtgcgccggaatttttctcaaacggcgccaaactgatgaccgttgatggtccggcagctaaactggacattgtccgtctgcgcgaacgtacgcgcgaaaaagtgggtgatgttcataccacgcagccggcatgcgtctctattacccaagctacggaagtgggcagtatctataccctggatgaaattgaagccatcggtgacgtgtgcaaatcatcgagcctgggtctgcacatggatggctctcgttttgctaatgcgctggtgtccctgggctgttcaccggcagaaatgacctggaaagccggtgttgacgcactgagttttggtgcgacgaaaaacggcgttctggcggccgaagcaattgtcctgttcaatacctcgctggctacggaaatgagctatcgtcgcaaacgtgccggccacctgaccagtaaatatcgctttctgagcgctcagatcgatgcgtacctgaccgatgacctgtggctgcgtaacgcccgcaaagcaaatgcagctgcgcagcgtctggcccaaggtctggaaggcctgggcggtgttgaagtcctgggcggtaccgaagcaaacattctgttctgtcgcctggattctgccatgatcgacgcactgctgaaagctggctttggtttcgggcatcgtcgttggggtccgaacgtggttcgctttgttaccagcttcgctaccacggcggaagatgtggaccacctgctgaatcaggttcgcctggccgcagaccgtacgcaagaacgc

SEQ ID NO: 46 - protein, 376 aa, Artificial sequence
  Engineered sequence
MNGETSRPPALGFSSDNIAGASPEVAQALVKHSSGQAGPYGTDELTAQVKHSSGQADPYGTDELTAQVKRKFCEIFERDVEVFLVPTGTAANALCLSAMTPPWGNIYCHPASHINNDECGAPEFFSNGAKLMTVDGPAAKLDIVRLRERTREKVGDVHTTQPACVSITQATEVGSIYTLDEIEAIGDVCKSSSLGLHMDGSRFANALVSLGCSPAEMTWKAGVDALSFGATKNGVLAAEAIVLFNTSLATEMSYRRKRAGHLTSKYRFLSAQIDAYLTDDLWLRNARKANAAAQRLAQGLEGLGGVEVLGGTEANILFCRLDSAMIDALLKAGFGFGHRRWGPNVVRFVTSFATTAEDVDHLLNQVRLAADRTQER

SEQ ID NO: 47 - DNA, 1128 bp, Artificial sequence
  Engineered sequence
atgaacggtgaaacctcgcgtccgccggcgctgggttttagctctgataatattgctggtgcaagcccggaagtcgcacaggcactcgttaagcacagttcgggccaggcgggtccctatggcaccgacgagttgacggcacaggtcaagcatagctccggccaagctgatccttatggtaacgatgaactgactgctcaagttaaacgtaaattttgcgaaatcttcgaacgcgacgtcgaagtgttcctggttccgaccggtacggcagcaaacgcactgtgtctgtccgcaatgaccccgccgtggggtaatatttactgccatccggcgtcccacatcaacaatgatgaatgtggtgcgccggaatttttctcaaacggcgccaaactgatgaccgttgatggtccggcagctaaactggacattgtccgtctgcgcgaacgtacgcgcgaaaaagtgggtgatgttcataccacgcagccggcatgcgtctctattacccaagctacggaagtgggcagtatctataccctggatgaaattgaagccatcggtgacgtgtgcaaatcatcgagcctgggtctgcacatggatggctctcgttttgctaatgcgctggtgtccctgggctgttcaccggcagaaatgacctggaaagccggtgttgacgcactgagttttggtgcgacgaaaaacggcgttctggcggccgaagcaattgtcctgttcaatacctcgctggctacggaaatgagctatcgtcgcaaacgtgccggccacctgaccagtaaatatcgctttctgagcgctcagatcgatgcgtacctgaccgatgacctgtggctgcgtaacgcccgcaaagcaaatgcagctgcgcagcgtctggcccaaggtctggaaggcctgggcggtgttgaagtcctgggcggtaccgaagcaaacattctgttctgtcgcctggattctgccatgatcgacgcactgctgaaagctggctttggtttcgggcatcgtcgttggggtccgaacgtggttcgctttgttaccagcttcgctaccacggcggaagatgtggaccacctgctgaatcaggttcgcctggccgcagaccgtacgcaagaacgc

SEQ ID NO: 48 - protein, 376 aa, Artificial sequence
  Engineered sequence
MNGETSRPPALGFSSDNIAGASPEVAQALVKHSSGQAGPYGTDELTAQVKHSSGQADPYGNDELTAQVKRKFCEIFERDVEVFLVPTGTAANALCLSAMTPPWGNIYCHPASHINNDECGAPEFFSNGAKLMTVDGPAAKLDIVRLRERTREKVGDVHTTQPACVSITQATEVGSIYTLDEIEAIGDVCKSSSLGLHMDGSRFANALVSLGCSPAEMTWKAGVDALSFGATKNGVLAAEAIVLFNTSLATEMSYRRKRAGHLTSKYRFLSAQIDAYLTDDLWLRNARKANAAAQRLAQGLEGLGGVEVLGGTEANILFCRLDSAMIDALLKAGFGFGHRRWGPNVVRFVTSFATTAEDVDHLLNQVRLAADRTQER

SEQ ID NO: 49 - DNA, 1128 bp, Artificial sequence
  Engineered sequence
atgaacggtgaaacctcgcgtccgccggcgctgggttttagctctgataatattgctggtgcaagcccggaagtcgcacaggcactcgttaagcacagttcgggccaggcgggtccctatggcaccgacgagttgacggcacaggtcaagcatagctccggccaagctaaaccttatggtacagatgaactgactgctcaagttaaacgtaaattttgcgaaatcttcgaacgcgacgtcgaagtgttcctggttccgaccggtacggcagcaaacgcactgtgtctgtccgcaatgaccccgccgtggggtaatatttactgccatccggcgtcccacatcaacaatgatgaatgtggtgcgccggaatttttctcaaacggcgccaaactgatgaccgttgatggtccggcagctaaactggacattgtccgtctgcgcgaacgtacgcgcgaaaaagtgggtgatgttcataccacgcagccggcatgcgtctctattacccaagctacggaagtgggcagtatctataccctggatgaaattgaagccatcggtgacgtgtgcaaatcatcgagcctgggtctgcacatggatggctctcgttttgctaatgcgctggtgtccctgggctgttcaccggcagaaatgacctggaaagccggtgttgacgcactgagttttggtgcgacgaaaaacggcgttctggcggccgaagcaattgtcctgttcaatacctcgctggctacggaaatgagctatcgtcgcaaacgtgccggccacctgctgagtaaaatgcgctttctgagcgctcagatcgatgcgtacctgaccgatgacctgtggctgcgtaacgcccgcaaagcaaatgcagctgcgcagcgtctggcccaaggtctggaaggcctgggcggtgttgaagtcctgggcggtaccgaagcaaacattctgttctgtcgcctggattctgccatgatcgacgcactgctgaaagctggctttggtttcgggcataaacgttggggtccgaacgtggttcgctttgttaccagcttcgctaccacggcggaagatgtggaccacctgctgaatcaggttcgcctggccgcagaccgtacgcaagaacgc

SEQ ID NO: 50 - protein, 376 aa, Artificial sequence
  Engineered sequence
MNGETSRPPALGFSSDNIAGASPEVAQALVKHSSGQAGPYGTDELTAQVKHSSGQAKPYGTDELTAQVKRKFCEIFERDVEVFLVPTGTAANALCLSAMTPPWGNIYCHPASHINNDECGAPEFFSNGAKLMTVDGPAAKLDIVRLRERTREKVGDVHTTQPACVSITQATEVGSIYTLDEIEAIGDVCKSSSLGLHMDGSRFANALVSLGCSPAEMTWKAGVDALSFGATKNGVLAAEAIVLFNTSLATEMSYRRKRAGHLLSKMRFLSAQIDAYLTDDLWLRNARKANAAAQRLAQGLEGLGGVEVLGGTEANILFCRLDSAMIDALLKAGFGFGHKRWGPNVVRFVTSFATTAEDVDHLLNQVRLAADRTQER

SEQ ID NO: 51 - DNA, 1128 bp, Artificial sequence
  Engineered sequence
atgaacggtgaaacctcgcgtccgccggcgctgggttttagctctgataatattgctggtgcaagcccggaagtcgcacaggcactcgttaagcacagttcgggccaggcgggtccctatggcaccgacgagttgacggcacaggtcaagcatagctccggccaagctaaaccttatggtaacgatgaactgactgctcaagttaaacgtaaattttgcgaaatcttcgaacgcgacgtcgaagtgttcctggttccgaccggtacggcagcaaacgcactgtgtctgtccgcaatgaccccgccgtggggtaatatttactgccatccggcgtcccacatcaacaatgatgaatgtggtgcgccggaatttttctcaaacggcgccaaactgatgaccgttgatggtccggcagctaaactggacattgtccgtctgcgcgaacgtacgcgcgaaaaagtgggtgatgttcataccacgcagccggcatgcgtctctattacccaagctacggaagtgggcagtatctataccctggatgaaattgaagccatcggtgacgtgtgcaaatcatcgagcctgggtctgcacatggatggctctcgttttgctaatgcgctggtgtccctgggctgttcaccggcagaaatgacctggaaagccggtgttgacgcactgagttttggtgcgacgaaaaacggcgttctggcggccgaagcaattgtcctgttcaatacctcgctggctacggaaatgagctatcgtcgcaaacgtgccggccacctgaccagtaaaatgcgctttctgagcgctcagatcgatgcgtacctgaccgatgacctgtggctgcgtaacgcccgcaaagcaaatgcagctgcgcagcgtctggcccaaggtctggaaggcctgggcggtgttgaagtcctgggcggtaccgaagcaaacattctgttctgtcgcctggattctgccatgatcgacgcactgctgaaagctggctttggtttcgggcataaacgttggggtccgaacgtggttcgctttgttaccagcttcgctaccacggcggaagatgtggaccacctgctgaatcaggttcgcctggccgcagaccgtacgcaagaacgc

SEQ ID NO: 52 - protein, 376 aa, Artificial sequence
  Engineered sequence
MNGETSRPPALGFSSDNIAGASPEVAQALVKHSSGQAGPYGTDELTAQVKHSSGQAKPYGNDELTAQVKRKFCEIFERDVEVFLVPTGTAANALCLSAMTPPWGNIYCHPASHINNDECGAPEFFSNGAKLMTVDGPAAKLDIVRLRERTREKVGDVHTTQPACVSITQATEVGSIYTLDEIEAIGDVCKSSSLGLHMDGSRFANALVSLGCSPAEMTWKAGVDALSFGATKNGVLAAEAIVLFNTSLATEMSYRRKRAGHLTSKMRFLSAQIDAYLTDDLWLRNARKANAAAQRLAQGLEGLGGVEVLGGTEANILFCRLDSAMIDALLKAGFGFGHKRWGPNVVRFVTSFATTAEDVDHLLNQVRLAADRTQER

SEQ ID NO: 53 - DNA, 1128 bp, Artificial sequence
  Engineered sequence
atgaacggtgaaacctcgcgtccgccggcgctgggttttagctctgataatattgctggtgcaagcccggaagtcgcacaggcactcgttaagcacagttcgggccaggcgggtccctatggcaccgacgagttgacggcacaggtcaagcatagctccggccaagctgatccttatggtacagatgaactgactgctcaagttaaacgtaaattttgcgaaatcttcgaacgcgacgtcgaagtgttcctggttccgaccggtacggcagcaaacgcactgtgtctgtccgcaatgaccccgccgtggggtaatatttactgccatccggcgtcccacatcaacaatgatgaatgtggtgcgccggaatttttctcaaacggcgccaaactgatgaccgttgatggtccggcagctaaactggacattgtccgtctgcgcgaacgtacgcgcgaaaaagtgggtgatgttcataccacgcagccggcatgcgtctctattacccaagctacggaagtgggcagtatctataccctggatgaaattgaagccatcggtgacgtgtgcaaatcatcgagcctgggtctgcacatggatggctctcgttttgctaatgcgctggtgtccctgggctgttcaccggcagaaatgacctggaaagccggtgttgacgcactgagttttggtgcgacgaaaaacggcgttctggcggccgaagcaattgtcctgttcaatacctcgctggctacggaaatgagctatcgtcgcaaacgtgccggccacctgtctagtaaaatgcgctttctgagcgctcagatcgatgcgtacctgaccgatgacctgtggctgcgtaacgcccgcaaagcaaatgcagctgcgcagcgtctggcccaaggtctggaaggcctgggcggtgttgaagtcctgggcggtaccgaagcaaacattctgttctgtcgcctggattctgccatgatcgacgcactgctgaaagctggctttggtttcgggcataaacgttggggtccgaacgtggttcgctttgttaccagcttcgctaccacggcggaagatgtggaccacctgctgaatcaggttcgcctggccgcagaccgtacgcaagaacgc

SEQ ID NO: 54 - protein, 376 aa, Artificial sequence
  Engineered sequence
MNGETSRPPALGFSSDNIAGASPEVAQALVKHSSGQAGPYGTDELTAQVKHSSGQADPYGTDELTAQVKRKFCEIFERDVEVFLVPTGTAANALCLSAMTPPWGNIYCHPASHINNDECGAPEFFSNGAKLMTVDGPAAKLDIVRLRERTREKVGDVHTTQPACVSITQATEVGSIYTLDEIEAIGDVCKSSSLGLHMDGSRFANALVSLGCSPAEMTWKAGVDALSFGATKNGVLAAEAIVLFNTSLATEMSYRRKRAGHLSSKMRFLSAQIDAYLTDDLWLRNARKANAAAQRLAQGLEGLGGVEVLGGTEANILFCRLDSAMIDALLKAGFGFGHKRWGPNVVRFVTSFATTAEDVDHLLNQVRLAADRTQER

SEQ ID NO: 55 - DNA, 1128 bp, Artificial sequence
  Engineered sequence
atgaacggtgaaacctcgcgtccgccggcgctgggttttagctctgataatattgctggtgcaagcccggaagtcgcacaggcactcgttaagcacagttcgggccaggcgggtccctatggcaccgacgagttgacggcacaggtcaagcatagctccggccaagctgatccttatggtacagatgaactgactgctcaagttaaacgtaaattttgcgaaatcttcgaacgcgacgtcgaagtgttcctggttccgaccggtacggcagcaaacgcactgtgtctgtccgcaatgaccccgccgtggggtaatatttactgccatccggcgtcccacatcaacaatgatgaatgtggtgcgccggaatttttctcaaacggcgccaaactgatgaccgttgatggtccggcagctaaactggacattgtccgtctgcgcgaacgtacgcgcgaaaaagtgggtgatgttcataccacgcagccggcatgcgtctctattacccaagctacggaagtgggcagtatctataccctggatgaaattgaagccatcggtgacgtgtgcaaatcatcgagcctgggtctgcacatggatggctctcgttttgctaatgcgctggtgtccctgggctgttcaccggcagaaatgacctggaaagccggtgttgacgcactgagttttggtgcgacgaaaaacggcgttctggcggccgaagcaattgtcctgttcaatacctcgctggctacggaaatgagctatcgtcgcaaacgtgccggccacctgctgagtaaaatgcgctttctgagcgctcagatcgatgcgtacctgaccgatgacctgtggctgcgtaacgcccgcaaagcaaatgcagctgcgcagcgtctggcccaaggtctggaaggcctgggcggtgttgaagtcctgggcggtaccgaagcaaacattctgttctgtcgcctggattctgccatgatcgacgcactgctgaaagctggctttggtttcgggcataaacgttggggtccgaacgtggttcgctttgttaccagcttcgctaccacggcggaagatgtggaccacctgctgaatcaggttcgcctggccgcagaccgtacgcaagaacgc

SEQ ID NO: 56 - protein, 376 aa, Artificial sequence
  Engineered sequence
MNGETSRPPALGFSSDNIAGASPEVAQALVKHSSGQAGPYGTDELTAQVKHSSGQADPYGTDELTAQVKRKFCEIFERDVEVFLVPTGTAANALCLSAMTPPWGNIYCHPASHINNDECGAPEFFSNGAKLMTVDGPAAKLDIVRLRERTREKVGDVHTTQPACVSITQATEVGSIYTLDEIEAIGDVCKSSSLGLHMDGSRFANALVSLGCSPAEMTWKAGVDALSFGATKNGVLAAEAIVLFNTSLATEMSYRRKRAGHLLSKMRFLSAQIDAYLTDDLWLRNARKANAAAQRLAQGLEGLGGVEVLGGTEANILFCRLDSAMIDALLKAGFGFGHKRWGPNVVRFVTSFATTAEDVDHLLNQVRLAADRTQER

SEQ ID NO: 57 - DNA, 1128 bp, Artificial sequence
  Engineered sequence
atgaacggtgaaacctcgcgtccgccggcgctgggttttagctctgataatattgctggtgcaagcccggaagtcgcacaggcactcgttaagcacagttcgggccaggcgggtccctatggcaccgacgagttgacggcacaggtcaagcatagctccggccaagctgatccttatggtacagatgaactgactgctcaagttaaacgtaaattttgcgaaatcttcgaacgcgacgtcgaagtgttcctggttccgaccggtacggcagcaaacgcactgtgtctgtccgcaatgaccccgccgtggggtaatatttactgccatccggcgtcccacatcaacaatgatgaatgtggtgcgccggaatttttctcaaacggcgccaaactgatgaccgttgatggtccggcagctaaactggacattgtccgtctgcgcgaacgtacgcgcgaaaaagtgggtgatgttcataccacgcagccggcatgcgtctctattacccaagctacggaagtgggcagtatctataccctggatgaaattgaagccatcggtgacgtgtgcaaatcatcgagcctgggtctgcacatggatggctctcgttttgctaatgcgctggtgtccctgggctgttcaccggcagaaatgacctggaaagccggtgttgacgcactgagttttggtgcgacgaaaaacggcgttctggcggccgaagcaattgtcctgttcaatacctcgctggctacggaaatgagctatcgtcgcaaacgtgccggccacctgaccagtaaaatgcgctttctgagcgctcagatcgatgcgtacctgaccgatgacctgtggctgcgtaacgcccgcaaagcaaatgcagctgcgcagcgtctggcccaaggtctggaaggcctgggcggtgttgaagtcctgggcggtaccgaagcaaacattctgttctgtcgcctggattctgccatgatcgacgcactgctgaaagctggctttggtttcgggcataaacgttggggtccgaacgtggttcgctttgttaccagcttcgctaccacggcggaagatgtggaccacctgctgaatcaggttcgcctggccgcagaccgtacgcaagaacgc

SEQ ID NO: 58 - protein, 376 aa, Artificial sequence
  Engineered sequence
MNGETSRPPALGFSSDNIAGASPEVAQALVKHSSGQAGPYGTDELTAQVKHSSGQADPYGTDELTAQVKRKFCEIFERDVEVFLVPTGTAANALCLSAMTPPWGNIYCHPASHINNDECGAPEFFSNGAKLMTVDGPAAKLDIVRLRERTREKVGDVHTTQPACVSITQATEVGSIYTLDEIEAIGDVCKSSSLGLHMDGSRFANALVSLGCSPAEMTWKAGVDALSFGATKNGVLAAEAIVLFNTSLATEMSYRRKRAGHLTSKMRFLSAQIDAYLTDDLWLRNARKANAAAQRLAQGLEGLGGVEVLGGTEANILFCRLDSAMIDALLKAGFGFGHKRWGPNVVRFVTSFATTAEDVDHLLNQVRLAADRTQER

SEQ ID NO: 59 - DNA, 1128 bp, Artificial sequence
  Engineered sequence
atgaacggtgaaacctcgcgtccgccggcgctgggttttagctctgataattgggctggtgcaagcccggaagtcgcacaggcactcgttaagcacagttcgggccaggcgggtccctatggcaccgacgagttgacggcacaggtcaagcatagctccggccaagctgatccttatggtacagatgaactgactgctcaagttaaacgtaaattttgcgaaatcttcgaacgcgacgtcgaagtgttcctggttccgaccggtacggcagcaaacgcactgtgtctgtccgcaatgaccccgccgtggggtaatatttactgccatccggcgtcccacatcaacaatgatgaatgtggtgcgccggaatttttctcaaacggcgccaaactgatgaccgttgatggtccggcagctaaactggacattgtccgtctgcgcgaacgtacgcgcgaaaaagtgggtgatgttcataccacgcagccggcatgcgtctctattacccaagctacggaagtgggcagtatctataccctggatgaaattgaagccatcggtgacgtgtgcaaatcatcgagcctgggtctgcacatggatggctctcgttttgctaatgcgctggtgtccctgggctgttcaccggcagaaatgacctggaaagccggtgttgacgcactgagttttggtgcgacgaaaaacggcgttctggcggccgaagcaattgtcctgttcaatacctcgctggctacggaaatgagctatcgtcgcaaacgtgccggccacctggtgagtaaaatgcgctttctgagcgctcagatcgatgcgtacctgaccgatgacctgtggctgcgtaacgcccgcaaagcaaatgcagctgcgcagcgtctggcccaaggtctggaaggcctgggcggtgttgaagtcctgggcggtaccgaagcaaacattctgttctgtcgcctggattctgccatgatcgacgcactgctgaaagctggctttggtttcgggcataaacgttggggtccgaacgtggttcgctttgttaccagcttcgctaccacggcggaagatgtggaccacctgctgaatcaggttcgcctggccgcagaccgtacgcaagaacgc

SEQ ID NO: 60 - protein, 376 aa, Artificial sequence
  Engineered sequence
MNGETSRPPALGFSSDNWAGASPEVAQALVKHSSGQAGPYGTDELTAQVKHSSGQADPYGTDELTAQVKRKFCEIFERDVEVFLVPTGTAANALCLSAMTPPWGNIYCHPASHINNDECGAPEFFSNGAKLMTVDGPAAKLDIVRLRERTREKVGDVHTTQPACVSITQATEVGSIYTLDEIEAIGDVCKSSSLGLHMDGSRFANALVSLGCSPAEMTWKAGVDALSFGATKNGVLAAEAIVLFNTSLATEMSYRRKRAGHLVSKMRFLSAQIDAYLTDDLWLRNARKANAAAQRLAQGLEGLGGVEVLGGTEANILFCRLDSAMIDALLKAGFGFGHKRWGPNVVRFVTSFATTAEDVDHLLNQVRLAADRTQER

SEQ ID NO: 61 - DNA, 1128 bp, Artificial sequence
  Engineered sequence
atgaacggtgaaacctcgcgtccgccggcgctgggttttagctctgataatattgctggtgcaagcccggaagtcgcacaggcactcgttaagcacagttcgggccaggcgggtccctatggcaccgacgagttgacggcacaggtcaagcatagctccggccaagctgacccttatggtaccgatgaactgactgctcaagttaaacgtaaattttgcgaaatcttcgaacgcgacgtcgaagtgttcctggttccgaccggtacggcagcaaacgcactgtgtctgtccgcaatgaccccgccgtggggtaatatttactgccatccggcgtcccacatcaacaatgatgaatgtggtgcgccggaatttttctcaaacggcgccaaactgatgaccgttgatggtccggcagctaaactggacattgtccgtctgcgcgaacgtacgcgcgaaaaagtgggtgatgttcataccacgcagccggcatgcgtctctattacccaagctacggaagtgggcagtatctataccctggatgaaattgaagccatcggtgacgtgtgcaaatcatcgagcctgggtctgcacatggatggctctcgttttgctaatgcgctggtgtccctgggctgttcaccggcagaaatgacctggaaagccggtgttgacgcactgagttttggtgcgacgaaaaacggcgttctggcggccgaagcaattgtcctgttcaatacctcgctggctacggaaatgagctatcgtcgcaaacgtgccggccacctgacgagtaaataccgctttctgagcgctcagatcgatgcgtacctgaccgatgacctgtggctgcgtaacgcccgcaaagcaaatgcagctgcgcagcgtctggcccaaggtctggaaggcctgggcggtgttgaagtcctgggcggtaccgaagcaaacattctgttctgtcgcctggattctgccatgatcgacgcactgctgaaagctggctttggtttcgggcataagcgttggggtccgaacgtggttcgctttgttaccagcttcgctaccacggcggaagatgtggaccacctgctgaatcaggttcgcctggccgcagaccgtacgcaagaacgc

SEQ ID NO: 62 - protein, 376 aa, Artificial sequence
  Engineered sequence
MNGETSRPPALGFSSDNIAGASPEVAQALVKHSSGQAGPYGTDELTAQVKHSSGQADPYGTDELTAQVKRKFCEIFERDVEVFLVPTGTAANALCLSAMTPPWGNIYCHPASHINNDECGAPEFFSNGAKLMTVDGPAAKLDIVRLRERTREKVGDVHTTQPACVSITQATEVGSIYTLDEIEAIGDVCKSSSLGLHMDGSRFANALVSLGCSPAEMTWKAGVDALSFGATKNGVLAAEAIVLFNTSLATEMSYRRKRAGHLTSKYRFLSAQIDAYLTDDLWLRNARKANAAAQRLAQGLEGLGGVEVLGGTEANILFCRLDSAMIDALLKAGFGFGHKRWGPNVVRFVTSFATTAEDVDHLLNQVRLAADRTQER

SEQ ID NO: 63 - DNA, 1128 bp, Artificial sequence
  Engineered sequence
atgaacggtgaaacctcgcgtccgccggcgctgggttttagctctgataatattgctggtgcaagcccggaagtcgcacaggcactcgttaagcacagttcgggccaggcgggtccctatggcaccgacgagttgacggcacaggtcaagcatagctccggccaagctggaccttatggtacagatgaactgactgctcaagttaaacgtaaattttgcgaaatcttcgaacgcgacgtcgaagtgttcctggttccgaccggtacggcagcaaacgcactgtgtctgtccgcaatgaccccgccgtggggtaatatttactgccatccggcgtcccacatcaacaatgatgaatgtggtgcgccggaatttttctcaaacggcgccaaactgatgaccgttgatggtccggcagctaaactggacattgtccgtctgcgcgaacgtacgcgcgaaaaagtgggtgatgttcataccacgcagccggcatgcgtctctattacccaagctacggaagtgggcagtatctataccctggatgaaattgaagccatcggtgacgtgtgcaaatcatcgagcctgggtctgcacatggatggctctcgttttgctaatgcgctggtgtccctgggctgttcaccggcagaaatgacctggaaagccggtgttgacgcactgagttttggtgcgacgaaaaacggcgttctggcggccgaagcaattgtcctgttcaatacctcgctggctacggaaatgagctatcgtcgcaaacgtgccggccacctgtctagtaaaatgcgctttctgagcgctcagatcgatgcgtacctgaccgatgacctgtggctgcgtaacgcccgcaaagcaaatgcagctgcgcagcgtctggcccaaggtctggaaggcctgggcggtgttgaagtcctgggcggtaccgaagcaaacattctgttctgtcgcctggattctgccatgatcgacgcactgctgaaagctggctttggtttcgggtatgatcgttggggtccgaacgtggttcgctttgttaccagcttcgctaccacggcggaagatgtggaccacctgctgaatcaggttcgcctggccgcagaccgtacgcaagaacgc

SEQ ID NO: 64 - protein, 376 aa, Artificial sequence
  Engineered sequence
MNGETSRPPALGFSSDNIAGASPEVAQALVKHSSGQAGPYGTDELTAQVKHSSGQAGPYGTDELTAQVKRKFCEIFERDVEVFLVPTGTAANALCLSAMTPPWGNIYCHPASHINNDECGAPEFFSNGAKLMTVDGPAAKLDIVRLRERTREKVGDVHTTQPACVSITQATEVGSIYTLDEIEAIGDVCKSSSLGLHMDGSRFANALVSLGCSPAEMTWKAGVDALSFGATKNGVLAAEAIVLFNTSLATEMSYRRKRAGHLSSKMRFLSAQIDAYLTDDLWLRNARKANAAAQRLAQGLEGLGGVEVLGGTEANILFCRLDSAMIDALLKAGFGFGYDRWGPNVVRFVTSFATTAEDVDHLLNQVRLAADRTQER

SEQ ID NO: 65 - DNA, 1128 bp, Artificial sequence
  Engineered sequence
atgaacggtgaaacctcgcgtccgccggcgctgggttttagctctgataatattgctggtgcaagcccggaagtcgcacaggcactcgttaagcacagttcgggccaggcgggtccctatggcaccgacgagttgacggcacaggtcaagcatagctccggccaagctggaccttatggtacagatgaactgactgctcaagttaaacgtaaattttgcgaaatcttcgaacgcgacgtcgaagtgttcctggttccgaccggtacggcagcaaacgcactgtgtctgtccgcaatgaccccgccgtggggtaatatttactgccatccggcgtcccacatcaacaatgatgaatgtggtgcgccggaatttttctcaaacggcgccaaactgatgaccgttgatggtccggcagctaaactggacattgtccgtctgcgcgaacgtacgcgcgaaaaagtgggtgatgttcataccacgcagccggcatgcgtctctattacccaagctacggaagtgggcagtatctataccctggatgaaattgaagccatcggtgacgtgtgcaaatcatcgagcctgggtctgcacatggatggctctcgttttgctaatgcgctggtgtccctgggctgttcaccggcagaaatgacctggaaagccggtgttgacgcactgagttttggtgcgacgaaaaacggcgttctggcggccgaagcaattgtcctgttcaatacctcgctggctacggaaatgagctatcgtcgcaaacgtgccggccacctgaccagtaaaatgcgctttctgagcgctcagatcgatgcgtacctgaccgatgacctgtggctgcgtaacgcccgcaaagcaaatgcagctgcgcagcgtctggcccaaggtctggaaggcctgggcggtgttgaagtcctgggcggtaccgaagcaaacattctgttctgtcgcctggattctgccatgatcgacgcactgctgaaagctggctttggtttcgggcatgatcgttggggtccgaacgtggttcgctttgttaccagcttcgctaccacggcggaagatgtggaccacctgctgaatcaggttcgcctggccgcagaccgtacgcaagaacgc

SEQ ID NO: 66 - protein, 376 aa, Artificial sequence
  Engineered sequence
MNGETSRPPALGFSSDNIAGASPEVAQALVKHSSGQAGPYGTDELTAQVKHSSGQAGPYGTDELTAQVKRKFCEIFERDVEVFLVPTGTAANALCLSAMTPPWGNIYCHPASHINNDECGAPEFFSNGAKLMTVDGPAAKLDIVRLRERTREKVGDVHTTQPACVSITQATEVGSIYTLDEIEAIGDVCKSSSLGLHMDGSRFANALVSLGCSPAEMTWKAGVDALSFGATKNGVLAAEAIVLFNTSLATEMSYRRKRAGHLTSKMRFLSAQIDAYLTDDLWLRNARKANAAAQRLAQGLEGLGGVEVLGGTEANILFCRLDSAMIDALLKAGFGFGHDRWGPNVVRFVTSFATTAEDVDHLLNQVRLAADRTQER

SEQ ID NO: 67 - DNA, 1128 bp, Artificial sequence
  Engineered sequence
atgaacggtgaaacctcgcgtccgccggcgctgggttttagctctgataatattgctggtgcaagcccggaagtcgcacaggcactcgttaagcacagttcgggccaggcgggtccctatggcaccgacgagttgacggcacaggtcaagcatagctccggccaagctggaccttatggtacagatgaactgactgctcaagttaaacgtaaattttgcgaaatcttcgaacgcgacgtcgaagtgttcctggttccgaccggtacggcagcaaacgcactgtgtctgtccgcaatgaccccgccgtggggtaatatttactgccatccggcgtcccacatcaacaatgatgaatgtggtgcgccggaatttttctcaaacggcgccaaactgatgaccgttgatggtccggcagctaaactggacattgtccgtctgcgcgaacgtacgcgcgaaaaagtgggtgatgttcataccacgcagccggcatgcgtctctattacccaagctacggaagtgggcagtatctataccctggatgaaattgaagccatcggtgacgtgtgcaaatcatcgagcctgggtctgcacatggatggctctcgttttgctaatgcgctggtgtccctgggctgttcaccggcagaaatgacctggaaagccggtgttgacgcactgagttttggtgcgacgaaaaacggcgttctggcggccgaagcaattgtcctgttcaatacctcgctggctacggaaatgagctatcgtcgcaaacgtgccggccacctgaccagtaaatatcgctttctgagcgctcagatcgatgcgtacctgaccgatgacctgtggctgcgtaacgcccgcaaagcaaatgcagctgcgcagcgtctggcccaaggtctggaaggcctgggcggtgttgaagtcctgggcggtaccgaagcaaacattctgttctgtcgcctggattctgccatgatcgacgcactgctgaaagctggctttggtttcgggcatcgtcgttggggtccgaacgtggttcgctttgttaccagcttcgctaccacggcggaagatgtggaccacctgctgaatcaggttcgcctggccgcagaccgtacgcaagaacgc

SEQ ID NO: 68 - protein, 376 aa, Artificial sequence
  Engineered sequence
MNGETSRPPALGFSSDNIAGASPEVAQALVKHSSGQAGPYGTDELTAQVKHSSGQAGPYGTDELTAQVKRKFCEIFERDVEVFLVPTGTAANALCLSAMTPPWGNIYCHPASHINNDECGAPEFFSNGAKLMTVDGPAAKLDIVRLRERTREKVGDVHTTQPACVSITQATEVGSIYTLDEIEAIGDVCKSSSLGLHMDGSRFANALVSLGCSPAEMTWKAGVDALSFGATKNGVLAAEAIVLFNTSLATEMSYRRKRAGHLTSKYRFLSAQIDAYLTDDLWLRNARKANAAAQRLAQGLEGLGGVEVLGGTEANILFCRLDSAMIDALLKAGFGFGHRRWGPNVVRFVTSFATTAEDVDHLLNQVRLAADRTQER

SEQ ID NO: 69 - DNA, 1128 bp, Artificial sequence
  Engineered sequence
atgaacggtgaaacctcgcgtccgccggcgctgggttttagctctgataatattgctggtgcaagcccggaagtcgcacaggcactcgttaagcacagttcgggccaggcgggtccctatggcaccgacgagttgacggcacaggtcaagcatagctccggccaagctggaccttatggtacagatgaactgactgctcaagttaaacgtaaattttgcgaaatcttcgaacgcgacgtcgaagtgttcctggttccgaccggtacggcagcaaacgcactgtgtctgtccgcaatgaccccgccgtggggtaatatttactgccatccggcgtcccacatcaacaatgatgaatgtggtgcgccggaatttttctcaaacggcgccaaactgatgaccgttgatggtccggcagctaaactggacattgtccgtctgcgcgaacgtacgcgcgaaaaagtgggtgatgttcataccacgcagccggcatgcgtctctattacccaagctacggaagtgggcagtatctataccctggatgaaattgaagccatcggtgacgtgtgcaaatcatcgagcctgggtctgcacatggatggctctcgttttgctaatgcgctggtgtccctgggctgttcaccggcagaaatgacctggaaagccggtgttgacgcactgagttttggtgcgacgaaaaacggcgttctggcggccgaagcaattgtcctgttcaatacctcgctggctacggaaatgagctatcgtcgcaaacgtgccggccacctggtgagtaaatatcgctttctgagcgctcagatcgatgcgtacctgaccgatgacctgtggctgcgtaacgcccgcaaagcaaatgcagctgcgcagcgtctggcccaaggtctggaaggcctgggcggtgttgaagtcctgggcggtaccgaagcaaacattctgttctgtcgcctggattctgccatgatcgacgcactgctgaaagctggctttggtttcgggcatgatcgttggggtccgaacgtggttcgctttgttaccagcttcgctaccacggcggaagatgtggaccacctgctgaatcaggttcgcctggccgcagaccgtacgcaagaacgc

SEQ ID NO: 70 - protein, 376 aa, Artificial sequence
  Engineered sequence
MNGETSRPPALGFSSDNIAGASPEVAQALVKHSSGQAGPYGTDELTAQVKHSSGQAGPYGTDELTAQVKRKFCEIFERDVEVFLVPTGTAANALCLSAMTPPWGNIYCHPASHINNDECGAPEFFSNGAKLMTVDGPAAKLDIVRLRERTREKVGDVHTTQPACVSITQATEVGSIYTLDEIEAIGDVCKSSSLGLHMDGSRFANALVSLGCSPAEMTWKAGVDALSFGATKNGVLAAEAIVLFNTSLATEMSYRRKRAGHLVSKYRFLSAQIDAYLTDDLWLRNARKANAAAQRLAQGLEGLGGVEVLGGTEANILFCRLDSAMIDALLKAGFGFGHDRWGPNVVRFVTSFATTAEDVDHLLNQVRLAADRTQER

SEQ ID NO: 71 - DNA, 1128 bp, Artificial sequence
  Engineered sequence
atgaacggtgaaacctcgcgtccgccggcgctgggttttagctctgataatattgctggtgcaagcccggaagtcgcacaggcactcgttaagcacagttcgggccaggcgggtccctatggcaccgacgagttgacggcacaggtcaagcatagctccggccaagctggaccttatggtacagatgaactgactgctcaagttaaacgtaaattttgcgaaatcttcgaacgcgacgtcgaagtgttcctggttccgaccggtacggcagcaaacgcactgtgtctgtccgcaatgaccccgccgtggggtaatatttactgccatccggcgtcccacatcaacaatgatgaatgtggtgcgccggaatttttctcaaacggcgccaaactgatgaccgttgatggtccggcagctaaactggacattgtccgtctgcgcgaacgtacgcgcgaaaaagtgggtgatgttcataccacgcagccggcatgcgtctctattacccaagctacggaagtgggcagtatctataccctggatgaaattgaagccatcggtgacgtgtgcaaatcatcgagcctgggtctgcacatggatggctctcgttttgctaatgcgctggtgtccctgggctgttcaccggcagaaatgacctggaaagccggtgttgacgcactgagttttggtgcgacgaaaaacggcgttctggcggccgaagcaattgtcctgttcaatacctcgctggctacggaaatgagctatcgtcgcaaacgtgccggccacctggtgagtaaatatcgctttctgagcgctcagatcgatgcgtacctgaccgatgacctgtggctgcgtaacgcccgcaaagcaaatgcagctgcgcagcgtctggcccaaggtctggaaggcctgggcggtgttgaagtcctgggcggtaccgaagcaaacattctgttctgtcgcctggattctgccatgatcgacgcactgctgaaagctggctttggtttcgggcataaacgttggggtccgaacgtggttcgctttgttaccagcttcgctaccacggcggaagatgtggaccacctgctgaatcaggttcgcctggccgcagaccgtacgcaagaacgc

SEQ ID NO: 72 - protein, 376 aa, Artificial sequence
  Engineered sequence
MNGETSRPPALGFSSDNIAGASPEVAQALVKHSSGQAGPYGTDELTAQVKHSSGQAGPYGTDELTAQVKRKFCEIFERDVEVFLVPTGTAANALCLSAMTPPWGNIYCHPASHINNDECGAPEFFSNGAKLMTVDGPAAKLDIVRLRERTREKVGDVHTTQPACVSITQATEVGSIYTLDEIEAIGDVCKSSSLGLHMDGSRFANALVSLGCSPAEMTWKAGVDALSFGATKNGVLAAEAIVLFNTSLATEMSYRRKRAGHLVSKYRFLSAQIDAYLTDDLWLRNARKANAAAQRLAQGLEGLGGVEVLGGTEANILFCRLDSAMIDALLKAGFGFGHKRWGPNVVRFVTSFATTAEDVDHLLNQVRLAADRTQER

SEQ ID NO: 73 - DNA, 1128 bp, Artificial sequence
  Engineered sequence
atgaacggtgaaacctcgcgtccgccggcgctgggttttagctctgataatattgctggtgcaagcccggaagtcgcacaggcactcgttaagcacagttcgggccaggcgggtccctatggcaccgacgagttgacggcacaggtcaagcatagctccggccaagctggaccttatggtacagatgaactgactgctcaagttaaacgtaaattttgcgaaatcttcgaacgcgacgtcgaagtgttcctggttccgaccggtacggcagcaaacgcactgtgtctgtccgcaatgaccccgccgtggggtaatatttactgccatccggcgtcccacatcaacaatgatgaatgtggtgcgccggaatttttctcaaacggcgccaaactgatgaccgttgatggtccggcagctaaactggacattgtccgtctgcgcgaacgtacgcgcgaaaaagtgggtgatgttcataccacgcagccggcatgcgtctctattacccaagctacggaagtgggcagtatctataccctggatgaaattgaagccatcggtgacgtgtgcaaatcatcgagcctgggtctgcacatggatggctctcgttttgctaatgcgctggtgtccctgggctgttcaccggcagaaatgacctggaaagccggtgttgacgcactgagttttggtgcgacgaaaaacggcgttctggcggccgaagcaattgtcctgttcaatacctcgctggctacggaaatgagctatcgtcgcaaacgtgccggccacctgctgagtaaatatcgctttctgagcgctcagatcgatgcgtacctgaccgatgacctgtggctgcgtaacgcccgcaaagcaaatgcagctgcgcagcgtctggcccaaggtctggaaggcctgggcggtgttgaagtcctgggcggtaccgaagcaaacattctgttctgtcgcctggattctgccatgatcgacgcactgctgaaagctggctttggtttcgggcataaacgttggggtccgaacgtggttcgctttgttaccagcttcgctaccacggcggaagatgtggaccacctgctgaatcaggttcgcctggccgcagaccgtacgcaagaacgc

SEQ ID NO: 74 - protein, 376 aa, Artificial sequence
  Engineered sequence
MNGETSRPPALGFSSDNIAGASPEVAQALVKHSSGQAGPYGTDELTAQVKHSSGQAGPYGTDELTAQVKRKFCEIFERDVEVFLVPTGTAANALCLSAMTPPWGNIYCHPASHINNDECGAPEFFSNGAKLMTVDGPAAKLDIVRLRERTREKVGDVHTTQPACVSITQATEVGSIYTLDEIEAIGDVCKSSSLGLHMDGSRFANALVSLGCSPAEMTWKAGVDALSFGATKNGVLAAEAIVLFNTSLATEMSYRRKRAGHLLSKYRFLSAQIDAYLTDDLWLRNARKANAAAQRLAQGLEGLGGVEVLGGTEANILFCRLDSAMIDALLKAGFGFGHKRWGPNVVRFVTSFATTAEDVDHLLNQVRLAADRTQER

SEQ ID NO: 75 - DNA, 1128 bp, Artificial sequence
  Engineered sequence
atgaacggtgaaacctcgcgtccgccggcgctgggttttagctctgataatattgctggtgcaagcccggaagtcgcacaggcactcgttaagcacagttcgggccaggcgggtccctatggcaccgacgagttgacggcacaggtcaagcatagctccggccaagctgacccttatggtaccgatgaactgactgctcaagttaaacgtaaattttgcgaaatcttcgaacgcgacgtcgaagtgttcctggttccgaccggtacggcagcaaacgcactgtgtctgtccgcaatgaccccgccgtggggtaatatttactgccatgcggcgtcccacatcaacaatgatgaatgtggtgcgccggaatttttctcaaacggcgccaaactgatgaccgttgatggtccggcagctaaactggacattgtccgtctgcgcgaacgtacgcgcgaaaaagtgggtgatgttcatagcacgcagccggcatgcgtctctattacccaagctacggaagtgggcagtatctataccctggatgaaattgaagccatcggtgacgtgtgcaaatcatcgagcctgggtctgcacatggatggctctcgttttgctaatgcgctggtgtccctgggctgttcaccggcagaaatgacctggaaagccggtgttgacgcactgagttttggtgcgacgaaaaacggcgttctggcggccgaagcaattgtcctgttcaatacctcgctggctacggaaatgagctatcgtcgcaaacgtgccggccacctgacgagtaaataccgctttctgagcgctcagatcgatgcgtacctgaccgatgacctgtggctgcgtaacgcccgcaaagcaaatgcagctgcgcagcgtctggcccaaggtctggaaggcctgggcggtgttgaagtcctgggcggtaccgaagcaaacattctgttctgtcgcctggattctgccatgatcgacgcactgctgaaagctggctttggtttcgggaccaagcgttggggtccgaacgtggttcgctttgttaccagcttcgctaccacggcggaagatgtggaccacctgctgaatcaggttcgcctggccgcagaccgtacgcaagaacgc

SEQ ID NO: 76 - protein, 376 aa, Artificial sequence
  Engineered sequence
MNGETSRPPALGFSSDNIAGASPEVAQALVKHSSGQAGPYGTDELTAQVKHSSGQADPYGTDELTAQVKRKFCEIFERDVEVFLVPTGTAANALCLSAMTPPWGNIYCHAASHINNDECGAPEFFSNGAKLMTVDGPAAKLDIVRLRERTREKVGDVHSTQPACVSITQATEVGSIYTLDEIEAIGDVCKSSSLGLHMDGSRFANALVSLGCSPAEMTWKAGVDALSFGATKNGVLAAEAIVLFNTSLATEMSYRRKRAGHLTSKYRFLSAQIDAYLTDDLWLRNARKANAAAQRLAQGLEGLGGVEVLGGTEANILFCRLDSAMIDALLKAGFGFGTKRWGPNVVRFVTSFATTAEDVDHLLNQVRLAADRTQER

SEQ ID NO: 77 - DNA, 1128 bp, Artificial sequence
  Engineered sequence
atgaacggtgaaacctcgcgtccgccggcgctgggttttagctctgataatattgctggtgcaagcccggaagtcgcacaggcactcgttaagcacagttcgggccaggcgggtccctatggcaccgacgagttgacggcacaggtcaagcatagctccggccaagctgacccttatggtaccgatgaactgactgctcaagttaaacgtaaattttgcgaaatcttcgaacgcgacgtcgaagtgttcctggttccgaccggtacggcagcaaacgcactgtgtctgtccgcaatgaccccgccgtggggtaatatttactgccatccggcgtcccacatcaacaatgatgaatgtggtgcgccggaatttttctcaaacggcgccaaactgatgaccgttgatggtccggcagctaaactggacattgtccgtctgcgcgaacgtacgcgcgaaaaagtgggtgatgttcataccacgcagccggcatgcgtctctattacccaagctacggaagtgggcagtatctataccctggatgaaattgaagccatcggtgacgtgtgcaaatcatcgagcctgggtctgcacatggatggctctcgttttgctaatgcgctggtgtccctgggctgttcaccggcagaaatgacctggaaagccggtgttgacgcactgagttttggtgcgacgaaaaacggcgttctggcggccgaagcaattgtcctgttcaatacctcgctggctacggaaatgagctatcgtcgcaaacgtgccggccacctgacgagtaaataccgctttctgagcgctcagatcgatgcgtacctgaccgatgacctgtggctgcgtaacgcccgcaaagcaaatgcagctgcgcagcgtctggcccaaggtctggaaggcctgggcggtgttgaagtcctgggcggtaccgaagcaaacattctgttctgtcgcctggattctgccatgatcgacgcactgctgaaagctggctttggtttcgggacgaagcgttggggtccgaacgtggttcgctttgttaccagcttcgctaccacggcggaagatgtggaccacctgctgaatcaggttcgcctggccgcagaccgtacgcaagaacgc

SEQ ID NO: 78 - protein, 376 aa, Artificial sequence
  Engineered sequence
MNGETSRPPALGFSSDNIAGASPEVAQALVKHSSGQAGPYGTDELTAQVKHSSGQADPYGTDELTAQVKRKFCEIFERDVEVFLVPTGTAANALCLSAMTPPWGNIYCHPASHINNDECGAPEFFSNGAKLMTVDGPAAKLDIVRLRERTREKVGDVHTTQPACVSITQATEVGSIYTLDEIEAIGDVCKSSSLGLHMDGSRFANALVSLGCSPAEMTWKAGVDALSFGATKNGVLAAEAIVLFNTSLATEMSYRRKRAGHLTSKYRFLSAQIDAYLTDDLWLRNARKANAAAQRLAQGLEGLGGVEVLGGTEANILFCRLDSAMIDALLKAGFGFGTKRWGPNVVRFVTSFATTAEDVDHLLNQVRLAADRTQER

SEQ ID NO: 79 - DNA, 1128 bp, Artificial sequence
  Engineered sequence
atgaacggtgaaacctcgcgtccgccggcgctgggttttagctctgataatattgctggtgcaagcccggaagtcgcacaggcactcgttaagcacagttcgggccaggcgggtccctatggcaccgacgagttgacggcacaggtcaagcatagctccggccaagctgacccttatggtaccgatgaactgactgctcaagttaaacgtaaattttgcgaaatcttcgaacgcgacgtcgaagtgttcctggttccgaccggtacggcagcaaacgcactgtgtctgtccgcaatgaccccgccgtggggtaatatttactgccatccggcgtcccacatcaacaatgatgaatgtggtgcgccggaatttttctcaaacggcgccaaactgatgaccgttgatggtccggcagctaaactggacattgtccgtctgcgcgaacgtacgcgcgaaaaagtgggtgatgttcataccacgcagccggcatgcgtctctattacccaagctacggaagtgggcagtatctataccctggatgaaattgaagccatcggtgacgtgtgcaaatcatcgagcctgggtctgcacatggatggctctcgttttgctaatgcgctggtgtccctgggctgttcaccggcagaaatgacctggaaagccggtgttgacgcactgagttttggtgcgacgaaaaacggcgttctggcggccgaagcaattgtcctgttcaatacctcgctggctacggaaatgagctatcgtcgcaaacgtgccggccacctgacgagtaaataccgctttctgagcgctcagatcgatgcgtacctgaccgatgacctgtggctgcgtaacgcccgcaaagcaaatgcagctgcgcagcgtctggcccaaggtctggaaggcctgggcggtgttgaagtcctgggcggtaccgaagcaaacattctgttctgtcgcctggattctgccatgatcgacgcactgctgaaagctggctttggtttcgggtataagcgttggggtccgaacgtggttcgctttgttaccagcttcgctaccacggcggaagatgtggaccacctgctgaatcaggttcgcctggccgcagaccgtacgcaagaacgc

SEQ ID NO: 80 - protein, 376 aa, Artificial sequence
  Engineered sequence
MNGETSRPPALGFSSDNIAGASPEVAQALVKHSSGQAGPYGTDELTAQVKHSSGQADPYGTDELTAQVKRKFCEIFERDVEVFLVPTGTAANALCLSAMTPPWGNIYCHPASHINNDECGAPEFFSNGAKLMTVDGPAAKLDIVRLRERTREKVGDVHTTQPACVSITQATEVGSIYTLDEIEAIGDVCKSSSLGLHMDGSRFANALVSLGCSPAEMTWKAGVDALSFGATKNGVLAAEAIVLFNTSLATEMSYRRKRAGHLTSKYRFLSAQIDAYLTDDLWLRNARKANAAAQRLAQGLEGLGGVEVLGGTEANILFCRLDSAMIDALLKAGFGFGYKRWGPNVVRFVTSFATTAEDVDHLLNQVRLAADRTQER

SEQ ID NO: 81 - DNA, 1128 bp, Artificial sequence
  Engineered sequence
atgaacggtgaaacctcgcgtccgccggcgctgggttttagctctgataatattgctggtgcaagcccggaagtcgcacaggcactcgttaagcacagttcgggccaggcgggtccctatggcaccgacgagttgacggcacaggtcaagcatagctccggccaagctgacccttatggtaccgatgaactgactgctcaagttaaacgtaaattttgcgaaatcttcgaacgcgacgtcgaagtgttcctggttccgaccggtacggcagcaaacgcactgtgtctgtccgcaatgaccccgccgtggggtaatatttactgccatgcggcgtcccacatcaacaatgatgaatgtggtgcgccggaatttttctcaaacggcgccaaactgatgaccgttgatggtccggcagctaaactggacattgtccgtctgcgcgaacgtacgcgcgaaaaagtgggtgatgttcatagcacgcagccggcatgcgtctctattacccaagctacggaagtgggcagtatctataccctggatgaaattgaagccatcggtgacgtgtgcaaatcatcgagcctgggtctgcacatggatggctctcgttttgctaatgcgctggtgtccctgggctgttcaccggcagaaatgacctggaaagccggtgttgacgcactgagttttggtgcgacgaaaaacggcgttctggcggccgaagcaattgtcctgttcaatacctcgctggctacggaaatgagctatcgtcgcaaacgtgccggccacctgacgagtaaataccgctttctgagcgctcagatcgatgcgtacctgaccgatgacctgtggctgcgtaacgcccgcaaagcaaatgcagctgcgcagcgtctggcccaaggtctggaaggcctgggcggtgttgaagtcctgggcggtaccgaagcaaacattctgttctgtcgcctggattctgccatgatcgacgcactgctgaaagctggctttggtttcgggcataagcgttggggtccgaacgtggttcgctttgttaccagcttcgctaccacggcggaagatgtggaccacctgctgaatcaggttcgcctggccgcagaccgtacgcaagaacgc

SEQ ID NO: 82 - protein, 376 aa, Artificial sequence
  Engineered sequence
MNGETSRPPALGFSSDNIAGASPEVAQALVKHSSGQAGPYGTDELTAQVKHSSGQADPYGTDELTAQVKRKFCEIFERDVEVFLVPTGTAANALCLSAMTPPWGNIYCHAASHINNDECGAPEFFSNGAKLMTVDGPAAKLDIVRLRERTREKVGDVHSTQPACVSITQATEVGSIYTLDEIEAIGDVCKSSSLGLHMDGSRFANALVSLGCSPAEMTWKAGVDALSFGATKNGVLAAEAIVLFNTSLATEMSYRRKRAGHLTSKYRFLSAQIDAYLTDDLWLRNARKANAAAQRLAQGLEGLGGVEVLGGTEANILFCRLDSAMIDALLKAGFGFGHKRWGPNVVRFVTSFATTAEDVDHLLNQVRLAADRTQER

SEQ ID NO: 83 - DNA, 1128 bp, Artificial sequence
  Engineered sequence
atgaacggtgaaacctcgcgtccgccggcgctgggttttagctctgataatattgctggtgcaagcccggaagtcgcacaggcactcgttaagcacagttcgggccaggcgggtccctatggcaccgacgagttgacggcacaggtcaagcatagctccggccaagctgacccttatggtaccgatgaactgactgctcaagttaaacgtaaattttgcgaaatcttcgaacgcgacgtcgaagtgttcctggttccgaccggtacggcagcaaacgcactgtgtctgtccgcaatgaccccgccgtggggtaatatttactgccatccggcgtcccacatcaacaatgatgaatgtggtgcgccggaatttttctcaaacggcgccaaactgatgaccgttgatggtccggcagctaaactggacattgtccgtctgcgcgaacgtacgcgcgaaaaagtgggtgatgttcataccacgcagccggcatgcgtctctattacccaagctacggaagtgggcagtatctataccctggatgaaattgaagccatcggtgacgtgtgcaaatcatcgagcctgggtctgcacatggatggctctcgttttgctaatgcgctggtgtccctgggctgttcaccggcagaaatgacctggaaagccggtgttgacgcactgagttttggtgcgacgaaaaacggcgttctggcggccgaagcaattgtcctgttcaatacctcgctggctacggaaatgagctatcgtcgcaaacgtgccggccacctgattagtaaataccgctttctgagcgctcagatcgatgcgtacctgaccgatgacctgtggctgcgtaacgcccgcaaagcaaatgcagctgcgcagcgtctggcccaaggtctggaaggcctgggcggtgttgaagtcctgggcggtaccgaagcaaacattctgttctgtcgcctggattctgccatgatcgacgcactgctgaaagctggctttggtttcgggcataagcgttggggtccgaacgtggttcgctttgttaccagcttcgctaccacggcggaagatgtggaccacctgctgaatcaggttcgcctggccgcagaccgtacgcaagaacgc

SEQ ID NO: 84 - protein, 376 aa, Artificial sequence
  Engineered sequence
MNGETSRPPALGFSSDNIAGASPEVAQALVKHSSGQAGPYGTDELTAQVKHSSGQADPYGTDELTAQVKRKFCEIFERDVEVFLVPTGTAANALCLSAMTPPWGNIYCHPASHINNDECGAPEFFSNGAKLMTVDGPAAKLDIVRLRERTREKVGDVHTTQPACVSITQATEVGSIYTLDEIEAIGDVCKSSSLGLHMDGSRFANALVSLGCSPAEMTWKAGVDALSFGATKNGVLAAEAIVLFNTSLATEMSYRRKRAGHLISKYRFLSAQIDAYLTDDLWLRNARKANAAAQRLAQGLEGLGGVEVLGGTEANILFCRLDSAMIDALLKAGFGFGHKRWGPNVVRFVTSFATTAEDVDHLLNQVRLAADRTQER

SEQ ID NO: 85 - DNA, 1128 bp, Artificial sequence
  Engineered sequence
atgaacggtgaaacctcgcgtccgccggcgctgggttttagctctgaaaatattgctggtgcaagcccggaagtcgcacaggcactcgttaagcacagttcgggccaggcgggtccctatggcaccgacgagttgacggcacaggtcaagcatagctccggccaagctgacccttatggtaccgatgaactgactgctcaagttaaacgtaaattttgcgaaatcttcgaacgcgacgtcgaagtgttcctggttccgaccggtacggcagcaaacgcactgtgtctgtccgcaatgaccccgccgtggggtaatatttactgccatccggcgtcccacatcaacaatgatgaatgtggtgcgccggaatttttctcaaacggcgccaaactgatgaccgttgatggtccggcagctaaactggacattgtccgtctgcgcgaacgtacgcgcgaaaaagtgggtgatgttcataccacgcagccggcatgcgtctctattacccaagctacggaagtgggcagtatctataccctggatgaaattgaagccatcggtgacgtgtgcaaatcatcgagcctgggtctgcacatggatggctctcgttttgctaatgcgctggtgtccctgggctgttcaccggcagaaatgacctggaaagccggtgttgacgcactgagttttggtgcgacgaaaaacggcgttctggcggccgaagcaattgtcctgttcaatacctcgctggctacggaaatgagctatcgtcgcaaacgtgccggccacctgacgagtaaataccgctttctgagcgctcagatcgatgcgtacctgaccgatgacctgtggctgcgtaacgcccgcaaagcaaatgcagctgcgcagcgtctggcccaaggtctggaaggcctgggcggtgttgaagtcctgggcggtaccgaagcaaacattctgttctgtcgcctggattctgccatgatcgacgcactgctgaaagctggctttggtttcgggcataagcgttggggtccgaacgtggttcgctttgttaccagcttcgctaccacggcggaagatgtggaccacctgctgaatcaggttcgcctggccgcagaccgtacgcaagaacgc

SEQ ID NO: 86 - protein, 376 aa, Artificial sequence
  Engineered sequence
MNGETSRPPALGFSSENIAGASPEVAQALVKHSSGQAGPYGTDELTAQVKHSSGQADPYGTDELTAQVKRKFCEIFERDVEVFLVPTGTAANALCLSAMTPPWGNIYCHPASHINNDECGAPEFFSNGAKLMTVDGPAAKLDIVRLRERTREKVGDVHTTQPACVSITQATEVGSIYTLDEIEAIGDVCKSSSLGLHMDGSRFANALVSLGCSPAEMTWKAGVDALSFGATKNGVLAAEAIVLFNTSLATEMSYRRKRAGHLTSKYRFLSAQIDAYLTDDLWLRNARKANAAAQRLAQGLEGLGGVEVLGGTEANILFCRLDSAMIDALLKAGFGFGHKRWGPNVVRFVTSFATTAEDVDHLLNQVRLAADRTQER

SEQ ID NO: 87 - DNA, 1128 bp, Artificial sequence
  Engineered sequence
atgaacggtgaaacctcgcgtccgccggcgctgggttttagctctgataatattgctggtgcaagcccggaagtcgcacaggcactcgttaagcacagttcgggccaggcgggtccctatgacaccgacgagttgacggcacaggtcaagcatagctccggccaagctgacccttatggtaccgatgaactgactgctcaagttaaacgtaaattttgcgaaatcttcgaacgcgacgtcgaagtgttcctggttccgaccggtacggcagcaaacgcactgtgtctgtccgcaatgaccccgccgtggggtaatatttactgccatccggcgtcccacatcaacaatgatgaatgtggtgcgccggaatttttctcaaacggcgccagactgatgaccgttgatggtccggcagctaaactggacattgtccgtctgcgagaacgtacgcgcgaaaaagtgggtgatgttcataccacgcagccggcatgcgtctctattacccaagctacggaagtgggcagtatctataccctggatgaaattgaagccatcggtgacgtgtgcaaatcatcgagcctgggtctgcacatggatggctctcgttttgctaatgcgctggtgtccctgggctgttcaccggcagaaatgacctggaaagccggtgttgacgcactgagttttggtgcgacgaaaaacggcgttctggcggccgaagcaattgtcctgttcaatacctcgctggctacggaaatgagctatcgtcgcaaacgtgccggccacctgacgagtaaataccgctttctgagcgctcagatcgatgcgtacctgaccgatgacctgtggctgcgtaacgcccgcaaagcaaatgcagctgcgcagcgtctggcccaaggtctggaaggcctgggcggtgttgaagtcctgggcggtaccgaagcaaacattctgttctgtcgcctggattctgccatgatcgacgcactgctgaaagctggctttggtttcgggacgaagcgttggggtccgaacgtggttcgctttgttaccagcttcgctaccacggcggaagatgtggaccacctgctgaatcaggttcgcctggccgcagaccgtacgcaagaacgc

SEQ ID NO: 88 - protein, 376 aa, Artificial sequence
  Engineered sequence
MNGETSRPPALGFSSDNIAGASPEVAQALVKHSSGQAGPYDTDELTAQVKHSSGQADPYGTDELTAQVKRKFCEIFERDVEVFLVPTGTAANALCLSAMTPPWGNIYCHPASHINNDECGAPEFFSNGARLMTVDGPAAKLDIVRLRERTREKVGDVHTTQPACVSITQATEVGSIYTLDEIEAIGDVCKSSSLGLHMDGSRFANALVSLGCSPAEMTWKAGVDALSFGATKNGVLAAEAIVLFNTSLATEMSYRRKRAGHLTSKYRFLSAQIDAYLTDDLWLRNARKANAAAQRLAQGLEGLGGVEVLGGTEANILFCRLDSAMIDALLKAGFGFGTKRWGPNVVRFVTSFATTAEDVDHLLNQVRLAADRTQER

SEQ ID NO: 89 - DNA, 1128 bp, Artificial sequence
  Engineered sequence
atgaacggtgaaacctcgcgtccgccggcgctgggttttagctctgataatattgctggtgcaagcccggaagtcgcacaggcactcgttaagcacagttcgggccaggcgggtccctatggcaccgacgagttgacggcacaggtcaagcatagctccggccaagctgacccttatggtaccgatgaactgactgctcaagttaaacgtaaattttgcgaaatcttcgaacgcgacgtcgaagtgttcctggttccgaccggtacggcagcaaacgcactgtgtctgtccgcaatgaccccgccgtggggtaatatttactgccatccggcgtcccacatcaacaatgatgaatgtggtgcgccggaatttttctcaaacggcgccaaactgatgaccgttgatggtccggcagctaaactggacattgtccgtctgcgcgaacgtacgcgcgaaaaagtgggtgatgttcataccacgcagccggcatgcgtctctattacccaagctacggaagtgggcagtatctataccctggatgaaattgaagccatcggtgacgtgtgcaaatcatcgagcctgggtctgcacattgatggctctcgttttgctaatgcgctggtgtccctgggctgttcaccggcagaaatgacctggaaagccggtgttgacgcgctgagttttggtgcgacgaaaaacggcgttctggcggccgaagcaattgtcctgttcaatacctcgctggttacggaaatgagctatcgtcgcaaacgtgccggccacctgacgagtaaataccgctttctgagcgctcagatcgatgcgtacctgaccgatgacctgtggctgcgtaacgcccgcaaagcaaatgcagctgcgcagcgtctggcccaaggtctggaaggcctgggcggtgttgaagtcctgggcggtaccgaagcaaacattctgttctgtcgcctggattctgccatgatcgacgcactgctgaaagctggctttggtttcgggacgaagcgttggggtccgaacgtggttcgctttgttaccagcttcgctaccacggcggaagatgtggaccacctgctgaatcaggttcgcctggccgcagaccgtacgcaagaacgc

SEQ ID NO: 90 - protein, 376 aa, Artificial sequence
  Engineered sequence
MNGETSRPPALGFSSDNIAGASPEVAQALVKHSSGQAGPYGTDELTAQVKHSSGQADPYGTDELTAQVKRKFCEIFERDVEVFLVPTGTAANALCLSAMTPPWGNIYCHPASHINNDECGAPEFFSNGAKLMTVDGPAAKLDIVRLRERTREKVGDVHTTQPACVSITQATEVGSIYTLDEIEAIGDVCKSSSLGLHIDGSRFANALVSLGCSPAEMTWKAGVDALSFGATKNGVLAAEAIVLFNTSLVTEMSYRRKRAGHLTSKYRFLSAQIDAYLTDDLWLRNARKANAAAQRLAQGLEGLGGVEVLGGTEANILFCRLDSAMIDALLKAGFGFGTKRWGPNVVRFVTSFATTAEDVDHLLNQVRLAADRTQER

SEQ ID NO: 91 - DNA, 1128 bp, Artificial sequence
  Engineered sequence
atgaacggtgaaacctcgcgtccgccggcgctgggttttagctctgataatattgctggtgcaagcccggaagtcgcacaggcactcgttaagcacagttcgggccaggcgggtccctatggcaccgacgagttgacggcacaggtcaagcatagctccggccaagctgacccttatggtaccgatgaactgactgctcaagttaaacgtaaattttgcgaaatcttcgaacgcgacgtcgaagtgttcctggttccgaccggtacggcagcaaacgcactgtgtctgtccgcaatgaccccgccgtggggtaatatttactgccatccggcgtcccacatcaacaatgatgaatgtggtgcgccggaatttttctcaaacggcgccaaactgatgaccgttgatggtccggcagctaaactggacattgtccgtctgcgcgaacgtacgcgcgaaaaagtgggtgatgttcatacgacgcagccggcatgcgtctctattacccaagctacggaagtgggcagtatctataccctggatgaaattgaagccatcggtgacgtgtgcaaatcatcgagcctgggtctgcacatggatggctctcgttttgctaatgcgctggtgtccctgggctgttcaccggcagaaatgacctggaaagccggtgttgacgcactgagttttggtgcgacgaaaaacggcgttctggcggccgaagcaattgtcctgttcaatacctcgctggctacggaaatgagctatcgtcgcaaacgtgccggccacctgatcagtaaataccgctttctgagcgctcagatcgatgcgtacctgaccgatgacctgtggctgcgtaacgcccgcaaagcaaatgcagctgcgcagcgtctggcccaaggtctggaaggcctgggcggtgttgaagtcctgggcggtaccgaagcaaacattctgttctgtcgcctggattctgccatgatcgacgcactgctgaaagctggctttggtttcgggtccgagcgttggggtccgaacgtggttcgctttgttaccagcttcgctaccacggcggaagatgtggaccacctgctgaatcaggttcgcctggccgcagaccgtacgcaagaacgc

SEQ ID NO: 92 - protein, 376 aa, Artificial sequence
  Engineered sequence
MNGETSRPPALGFSSDNIAGASPEVAQALVKHSSGQAGPYGTDELTAQVKHSSGQADPYGTDELTAQVKRKFCEIFERDVEVFLVPTGTAANALCLSAMTPPWGNIYCHPASHINNDECGAPEFFSNGAKLMTVDGPAAKLDIVRLRERTREKVGDVHTTQPACVSITQATEVGSIYTLDEIEAIGDVCKSSSLGLHMDGSRFANALVSLGCSPAEMTWKAGVDALSFGATKNGVLAAEAIVLFNTSLATEMSYRRKRAGHLISKYRFLSAQIDAYLTDDLWLRNARKANAAAQRLAQGLEGLGGVEVLGGTEANILFCRLDSAMIDALLKAGFGFGSERWGPNVVRFVTSFATTAEDVDHLLNQVRLAADRTQER

SEQ ID NO: 93 - DNA, 1128 bp, Artificial sequence
  Engineered sequence
atgaacggtgaaacctcgcgtccgccggcgctgggttttagctctgataatattgctggtgcaagcccggaagtcgcacaggcactcgttaagcacagttcgggccaggcgggtccctatggcaccgacgagttgacggcacaggtcaagcatagctccggccaagctgacccttatggtaccgatgaactgactgctcaagttaaacgtaaattttgcgaaatcttcgaacgcgacgtcgaagtgttcctggttccgaccggtacggcagcaaacgcactgtgtctgtccgcaatgaccccgccgtggggtaatatttactgccatcccgcgtcccacatcaacaatgatgaatgtggtgcgccggaatttttctcaaacggcgccaaactgatgaccgttgatggtccggcagctaaactggacattgtccgtctgcgcgaacgtacgcgctggaaagtgggtgatgttcattcgacgcagccggcatgcgtctctattacccaagctacggaagtgggcagtatctataccctggatgaaattgaagccatcggtgacgtgtgcaaatcatcgagcctgggtctgcacatggatggctctcgttttgctaatgcgctggtgtccctgggctgttcaccggcagaaatgacctggaaagccggtgttgacgcactgagttttggtgcgacgaaaaacggcgttctggcggccgaagcaattgtcctgttcaatacctcgctggctacggaaatgagctatcgtcgcaaacgtgccggccacctgaccagtaaataccgctttctgagcgctcagatcgatgcgtacctgaccgatgacctgtggctgcgtaacgcccgcaaagcaaatgcagctgcgcagcgtctggcccaaggtctggaaggcctgggcggtgttgaagtcctgggcggtaccgaagcaaacattctgttctgtcgcctggattctgccatgatcgacgcactgctgaaagctggctttggtttcgggtacaagcgttggggtccgaacgtggttcgctttgttaccagcttcgctaccacggcggaagatgtggaccacctgctgaatcaggttcgcctggccgcagaccgtacgcaagaacgc

SEQ ID NO: 94 - protein, 376 aa, Artificial sequence
  Engineered sequence
MNGETSRPPALGFSSDNIAGASPEVAQALVKHSSGQAGPYGTDELTAQVKHSSGQADPYGTDELTAQVKRKFCEIFERDVEVFLVPTGTAANALCLSAMTPPWGNIYCHPASHINNDECGAPEFFSNGAKLMTVDGPAAKLDIVRLRERTRWKVGDVHSTQPACVSITQATEVGSIYTLDEIEAIGDVCKSSSLGLHMDGSRFANALVSLGCSPAEMTWKAGVDALSFGATKNGVLAAEAIVLFNTSLATEMSYRRKRAGHLTSKYRFLSAQIDAYLTDDLWLRNARKANAAAQRLAQGLEGLGGVEVLGGTEANILFCRLDSAMIDALLKAGFGFGYKRWGPNVVRFVTSFATTAEDVDHLLNQVRLAADRTQER

SEQ ID NO: 95 - DNA, 1128 bp, Artificial sequence
  Engineered sequence
atgaacggtgaaacctcgcgtccgccggcgctgggttttagctctgataatattgctggtgcaagcccggaagtcgcacaggcactcgttaagcacagttcgggccaggcgggtccctatggcaccgacgagttgacggcacaggtcaagcatagctccggccaagctgacccttatggtaccgatgaactgactgctcaagttaaacgtaaattttgcgaaatcttcgaacgcgacgtcgaagtgttcctggttccgaccggtacggcagcaaacgcactgtgtctgtccgcaatgaccccgccgtggggtaatatttactgccatcacgcgtcccacatcaacaatgatgaatgtggtgcgccggaatttttctcaaacggcgccaaactgatgaccgttgatggtccggcagctaaactggacattgtccgtctgcgcgaacgtacgcgcgaaaaagtgggtgatgttcatacgacgcagccggcatgcgtctctattacccaagctacggaagtgggcagtatctataccctggatgaaattgaagccatcggtgacgtgtgcaaatcatcgagcctgggtctgcacatggatggctctcgttttgctaatgcgctggtgtccctgggctgttcaccggcagaaatgacctggaaagccggtgttgacgcactgagttttggtgcgacgaaaaacggcgttctggcggccgaagcaattgtcctgttcaatacctcgctggctacggaaatgagctatcgtcgcaaacgtgccggccacctgatcagtaaataccgctttctgagcgctcagatcgatgcgtacctgaccgatgacctgtggctgcgtaacgcccgcaaagcaaatgcagctgcgcagcgtctggcccaaggtctggaaggcctgggcggtgttgaagtcctgggcggtaccgaagcaaacattctgttctgtcgcctggattctgccatgatcgacgcactgctgaaagctggctttggtttcgggtacaagcgttggggtccgaacgtggttcgctttgttaccagcttcgctaccacggcggaagatgtggaccacctgctgaatcaggttcgcctggccgcagaccgtacgcaagaacgc

SEQ ID NO: 96 - protein, 376 aa, Artificial sequence
  Engineered sequence
MNGETSRPPALGFSSDNIAGASPEVAQALVKHSSGQAGPYGTDELTAQVKHSSGQADPYGTDELTAQVKRKFCEIFERDVEVFLVPTGTAANALCLSAMTPPWGNIYCHHASHINNDECGAPEFFSNGAKLMTVDGPAAKLDIVRLRERTREKVGDVHTTQPACVSITQATEVGSIYTLDEIEAIGDVCKSSSLGLHMDGSRFANALVSLGCSPAEMTWKAGVDALSFGATKNGVLAAEAIVLFNTSLATEMSYRRKRAGHLISKYRFLSAQIDAYLTDDLWLRNARKANAAAQRLAQGLEGLGGVEVLGGTEANILFCRLDSAMIDALLKAGFGFGYKRWGPNVVRFVTSFATTAEDVDHLLNQVRLAADRTQER

SEQ ID NO: 97 - DNA, 1128 bp, Artificial sequence
  Engineered sequence
atgaacggtgaaacctcgcgtccgccggcgctgggttttagctctgataatattgctggtgcaagcccggaagtcgcacaggcactcgttaagcacagttcgggccaggcgggtccctatggcaccgacgagttgacggcacaggtcaagcatagctccggccaagctgacccttatggtaccgatgaactgactgctcaagttaaacgtaaattttgcgaaatcttcgaacgcgacgtcgaagtgttcctggttccgaccggtacggcagcaaacgcactgtgtctgtccgcaatgaccccgccgtggggtaatatttactgccatcgcgcgtcccacatcaacaatgatgaatgtggtgcgccggaatttttctcaaacggcgccaaactgatgaccgttgatggtccggcagctaaactggacattgtccgtctgcgcgaacgtacgcgcgaaaaagtgggtgatgttcattcgacgcagccggcatgcgtctctattacccaagctacggaagtgggcagtatctataccctggatgaaattgaagccatcggtgacgtgtgcaaatcatcgagcctgggtctgcacatggatggctctcgttttgctaatgcgctggtgtccctgggctgttcaccggcagaaatgacctggaaagccggtgttgacgcactgagttttggtgcgacgaaaaacggcgttctggcggccgaagcaattgtcctgttcaatacctcgctggctacggaaatgagctatcgtcgcaaacgtgccggccacctgatcagtaaataccgctttctgagcgctcagatcgatgcgtacctgaccgatgacctgtggctgcgtaacgcccgcaaagcaaatgcagctgcgcagcgtctggcccaaggtctggaaggcctgggcggtgttgaagtcctgggcggtaccgaagcaaacattctgttctgtcgcctggattctgccatgatcgacgcactgctgaaagctggctttggtttcgggtacgagcgttggggtccgaacgtggttcgctttgttaccagcttcgctaccacggcggaagatgtggaccacctgctgaatcaggttcgcctggccgcagaccgtacgcaagaacgc

SEQ ID NO: 98 - protein, 376 aa, Artificial sequence
  Engineered sequence
MNGETSRPPALGFSSDNIAGASPEVAQALVKHSSGQAGPYGTDELTAQVKHSSGQADPYGTDELTAQVKRKFCEIFERDVEVFLVPTGTAANALCLSAMTPPWGNIYCHRASHINNDECGAPEFFSNGAKLMTVDGPAAKLDIVRLRERTREKVGDVHSTQPACVSITQATEVGSIYTLDEIEAIGDVCKSSSLGLHMDGSRFANALVSLGCSPAEMTWKAGVDALSFGATKNGVLAAEAIVLFNTSLATEMSYRRKRAGHLISKYRFLSAQIDAYLTDDLWLRNARKANAAAQRLAQGLEGLGGVEVLGGTEANILFCRLDSAMIDALLKAGFGFGYERWGPNVVRFVTSFATTAEDVDHLLNQVRLAADRTQER

SEQ ID NO: 99 - DNA, 1128 bp, Artificial sequence
  Engineered sequence
atgaacggtgaaacctcgcgtccgccggcgctgggttttagctctgataatattgctggtgcaagcccggaagtcgcacaggcactcgttaagcacagttcgggccaggcgggtccctatggcaccgacgagttgacggcacaggtcaagcatagctccggccaagctgacccttatggtaccgatgaactgactgctcaagttaaacgtaaattttgcgaaatcttcgaacgcgacgtcgaagtgttcctggttccgaccggtacggcagcaaacgcactgtgtctgtccgcaatgaccccgccgtggggtaatatttactgccatcgcgcgtcccacatcaacaatgatgaatgtggtgcgccggaatttttctcaaacggcgccaaactgatgaccgttgatggtccggcagctaaactggacattgtccgtctgcgcgaacgtacgcgcgaaaaagtgggtgatgttcatacgacgcagccggcatgcgtctctattacccaagctacggaagtgggcagtatctataccctggatgaaattgaagccatcggtgacgtgtgcaaatcatcgagcctgggtctgcacatggatggctctcgttttgctaatgcgctggtgtccctgggctgttcaccggcagaaatgacctggaaagccggtgttgacgcactgagttttggtgcgacgaaaaacggcgttctggcggccgaagcaattgtcctgttcaatacctcgctggctacggaaatgagctatcgtcgcaaacgtgccggccacctgatcagtaaataccgctttctgagcgctcagatcgatgcgtacctgaccgatgacctgtggctgcgtaacgcccgcaaagcaaatgcagctgcgcagcgtctggcccaaggtctggaaggcctgggcggtgttgaagtcctgggcggtaccgaagcaaacattctgttctgtcgcctggattctgccatgatcgacgcactgctgaaagctggctttggtttcgggtacaagcgttggggtccgaacgtggttcgctttgttaccagcttcgctaccacggcggaagatgtggaccacctgctgaatcaggttcgcctggccgcagaccgtacgcaagaacgc

SEQ ID NO: 100 - protein, 376 aa, Artificial sequence
  Engineered sequence
MNGETSRPPALGFSSDNIAGASPEVAQALVKHSSGQAGPYGTDELTAQVKHSSGQADPYGTDELTAQVKRKFCEIFERDVEVFLVPTGTAANALCLSAMTPPWGNIYCHRASHINNDECGAPEFFSNGAKLMTVDGPAAKLDIVRLRERTREKVGDVHTTQPACVSITQATEVGSIYTLDEIEAIGDVCKSSSLGLHMDGSRFANALVSLGCSPAEMTWKAGVDALSFGATKNGVLAAEAIVLFNTSLATEMSYRRKRAGHLISKYRFLSAQIDAYLTDDLWLRNARKANAAAQRLAQGLEGLGGVEVLGGTEANILFCRLDSAMIDALLKAGFGFGYKRWGPNVVRFVTSFATTAEDVDHLLNQVRLAADRTQER

SEQ ID NO: 101 - DNA, 1128 bp, Artificial sequence
  Engineered sequence
atgaacggtgaaacctcgcgtccgccggcgctgggttttagctctgataatattgctggtgcaagcccggaagtcgcacaggcactcgttaagcacagttcgggccaggcgggtccctatggcaccgacgagttgacggcacaggtcaagcatagctccggccaagctgacccttatggtaccgatgaactgactgctcaagttaaacgtaaattttgcgaaatcttcgaacgcgacgtcgaagtgttcctggttccgaccggtacggcagcaaacgcactgtgtctgtccgcaatgaccccgccgtggggtaatatttactgccatcacgcgtcccacatcaacaatgatgaatgtggtgcgccggaatttttctcaaacggcgccaaactgatgaccgttgatggtccggcagctaaactggacattgtccgtctgcgcgaacgtacgcgcgaaaaagtgggtgatgttcatacgacgcagccggcatgcgtctctattacccaagctacggaagtgggcagtatctataccctggatgaaattgaagccatcggtgacgtgtgcaaatcatcgagcctgggtctgcacatggatggctctcgttttgctaatgcgctggtgtccctgggctgttcaccggcagaaatgacctggaaagccggtgttgacgcactgagttttggtgcgacgaaaaacggcgttctggcggccgaagcaattgtcctgttcaatacctcgctggctacggaaatgagctatcgtcgcaaacgtgccggccacctgatcagtaaataccgctttctgagcgctcagatcgatgcgtacctgaccgatgacctgtggctgcgtaacgcccgcaaagcaaatgcagctgcgcagcgtctggcccaaggtctggaaggcctgggcggtgttgaagtcctgggcggtaccgaagcaaacattctgttctgtcgcctggattctgccatgatcgacgcactgctgaaagctggctttggtttcgggaacaagcgttggggtccgaacgtggttcgctttgttaccagcttcgctaccacggcggaagatgtggaccacctgctgaatcaggttcgcctggccgcagaccgtacgcaagaacgc

SEQ ID NO: 102 - protein, 376 aa, Artificial sequence
  Engineered sequence
MNGETSRPPALGFSSDNIAGASPEVAQALVKHSSGQAGPYGTDELTAQVKHSSGQADPYGTDELTAQVKRKFCEIFERDVEVFLVPTGTAANALCLSAMTPPWGNIYCHHASHINNDECGAPEFFSNGAKLMTVDGPAAKLDIVRLRERTREKVGDVHTTQPACVSITQATEVGSIYTLDEIEAIGDVCKSSSLGLHMDGSRFANALVSLGCSPAEMTWKAGVDALSFGATKNGVLAAEAIVLFNTSLATEMSYRRKRAGHLISKYRFLSAQIDAYLTDDLWLRNARKANAAAQRLAQGLEGLGGVEVLGGTEANILFCRLDSAMIDALLKAGFGFGNKRWGPNVVRFVTSFATTAEDVDHLLNQVRLAADRTQER

SEQ ID NO: 103 - DNA, 1128 bp, Artificial sequence
  Engineered sequence
atgaacggtgaaacctcgcgtccgccggcgctgggttttagctctgataatattgctggtgcaagcccggaagtcgcacaggcactcgttaagcacagttcgggccaggcgggtccctatggcaccgacgagttgacggcacaggtcaagcatagctccggccaagctgacccttatggtaccgatgaactgactgctcaagttaaacgtaaattttgcgaaatcttcgaacgcgacgtcgaagtgttcctggttccgaccggtacggcagcaaacgcactgtgtctgtccgcaatgaccccgccgtggggtaataattactgccatccggcgtcccacatcaacaatgatgaatgtggtgcgccggaatttttctcaaacggcgccaaactgatgaccgttgatggtccggcagctaaactggacattgtccgtctgcgcgaacgtacgaaggaaaaagtgggtgatgttcataccacgcagccggcatgcgtctctattacccaagctacggaagtgggcagtatctataccctggatgaaattgaagccatcggtgacgtgtgcaaatcatcgagcctgggtctgcacatggatggctctcgttttgctaatgcgctggtgtccctgggctgttcaccggcagaaatgacctggaaagccggtgttgacgcactgagttttggtgcgacgaaaaacggcgttctggcggccgaagcaattgtcctgttcaatacctcgctggctacggaaatgagctatcgtcgcaaacgtgccggccacctgacgagtaaataccgctttctgagcgctcagatcgatgcgtacctgaccgatgacctgtggctgcgtaacgcccgcaaagcaaatgcagctgcgcagcgtctggcccaaggtctggaaggcctgggcggtgttgaagtcctgggcggtaccgaagcaaacattctgttctgtcgcctggattctgccatgatcgacgcactgctgaaagctggctttggtttcgggacgaagcgttggggtccgaacgtggttcgctttgttaccagcttcgctaccacggcggaagatgtggaccacctgctgaatcaggttcgcctggccgcagaccgtacgcaagaacgc

SEQ ID NO: 104 - protein, 376 aa, Artificial sequence
  Engineered sequence
MNGETSRPPALGFSSDNIAGASPEVAQALVKHSSGQAGPYGTDELTAQVKHSSGQADPYGTDELTAQVKRKFCEIFERDVEVFLVPTGTAANALCLSAMTPPWGNNYCHPASHINNDECGAPEFFSNGAKLMTVDGPAAKLDIVRLRERTKEKVGDVHTTQPACVSITQATEVGSIYTLDEIEAIGDVCKSSSLGLHMDGSRFANALVSLGCSPAEMTWKAGVDALSFGATKNGVLAAEAIVLFNTSLATEMSYRRKRAGHLTSKYRFLSAQIDAYLTDDLWLRNARKANAAAQRLAQGLEGLGGVEVLGGTEANILFCRLDSAMIDALLKAGFGFGTKRWGPNVVRFVTSFATTAEDVDHLLNQVRLAADRTQER

SEQ ID NO: 105 - DNA, 1128 bp, Artificial sequence
  Engineered sequence
atgaacggtgaaacctcgcgtccgccggcgctgggttttagctctgataatattgctggtgcaagcccggaagtcgcacaggcactcgttaagcacagttcgggccaggcgggtccctatggcaccgacgagttgacggcacaggtcaagcatagctccggccaagctgacccttatggtaccgatgaactgactgctcaagttaaacgtaaattttgcgaaatcttcgaacgcgacgtcgaagtgttcctggttccgaccggtacggcagcaaacgcactgtgtctgtccgcaatgaccccgccgtggggtaatatttactgccatccggcgtcccacatcaacaatgatgaatgtggtgcgccggaatttttctcaaacggcgccaaactgatgaccgttgatggtccggcagctaaactggacattgtccgtctgcgcgaacgtacgagtgaaaaagtgggtgatgttcataccacgcagccggcatgcgtctctattacccaagctacggaagtgggcagtatctataccctggatgaaattgaagccatcggtgacgtgtgcaaatcatcgagcctgggtctgcacatggatggctctcgttttgctaatgcgctggtgtccctgggctgttcaccggcagaaatgacctggaaagccggtgttgacgcactgagttttggtgcgacgaaaaacggcgttctggcggccgaagcaattgtcctgttcaatacctcgctggctacggaaatgagctatcgtcgcaaacgtgccggccacctgacgagtaaataccgctttctgagcgctcagatcgatgcgtacctgaccgatgacctgtggctgcgtaacgcccgcaaagcaaatgcagctgcgcagcgtctggcccaaggtctggaaggcctgggcggtgttgaagtcctgggcggtaccgaagcaaacattctgttctgtcgcctggattctgccatgatcgacgcactgctgaaagctggctttggtttcgggacgaagcgttggggtccgaacgtggttcgctttgttaccagcttcgctaccacggcggaagatgtggaccacctgctgaatcaggttcgcctggccgcagaccgtacgcaagaacgc

SEQ ID NO: 106 - protein, 376 aa, Artificial sequence
  Engineered sequence
MNGETSRPPALGFSSDNIAGASPEVAQALVKHSSGQAGPYGTDELTAQVKHSSGQADPYGTDELTAQVKRKFCEIFERDVEVFLVPTGTAANALCLSAMTPPWGNIYCHPASHINNDECGAPEFFSNGAKLMTVDGPAAKLDIVRLRERTSEKVGDVHTTQPACVSITQATEVGSIYTLDEIEAIGDVCKSSSLGLHMDGSRFANALVSLGCSPAEMTWKAGVDALSFGATKNGVLAAEAIVLFNTSLATEMSYRRKRAGHLTSKYRFLSAQIDAYLTDDLWLRNARKANAAAQRLAQGLEGLGGVEVLGGTEANILFCRLDSAMIDALLKAGFGFGTKRWGPNVVRFVTSFATTAEDVDHLLNQVRLAADRTQER

SEQ ID NO: 107 - DNA, 1128 bp, Artificial sequence
  Engineered sequence
atgaacggtgaaacctcgcgtccgccggcgctgggttttagctctgataatattgctggtgcaagcccggaagtcgcacaggcactcgttaagcacagttcgggccaggcgggtccctatggcaccgacgagttgacggcacaggtcaagcatagctccggccaagctgacccttatggtaccgatgaactgactgctcaagttaaacgtaaattttgcgaaatcttcgaacgcgacgtcgaagtgttcctggttccgaccggtacggcagcaaacgcactgtgtctgtccgcaatgaccccgccgtggggtaatatttactgccatccggcgtcccacatcaacaatgatgaatgtggtgcgccggaatttttctcaaacggcgccaaactgatgaccgttgatggtccggcagctaaactggacattgtccgtctgcgcgaacgtacgcgcgaaaaagtgggtgatgttcataccacgcagccggcatgcgtctctattacccaagctacggaagtgggcagtatctataccctggatgaaattgaagccatcggtgacgtgtgcaaatcatcgagcctgggtctgcacatggatggctctcgttttgctaatgcgctggtgtccctgggctgttcaccggcagaaatgacctggaaagccggtgttgacgcactgagttttggtgcgacgaaaaacggcgttctggcggccgaagcaattgtcctgttcaatacctcgctggctacggaaatgagctatcgtcgcaaacgtgccggccacctgacgagtaaataccgctttctgagcgctcagatcgatgcgtacctgaccgatgacctgtggctgcgtaacgcccgcaaagcaaatgcagctgcgcagcgtctggcccaaggtctggaaggcctgggcggtgttgaagtcctgggcggtaccgaagcaaacattctgttctgtcgcctggattctgccatgatcgacgcactgctgaaagctggctttacgttcgggacgaagcgttggggtccgaacgtggttcgctttgttaccagcttcgctaccacggcggaagatgtggaccacctgctgaatcaggttcgcctggccgcagaccgtacgcaagaacgc

SEQ ID NO: 108 - protein, 376 aa, Artificial sequence
  Engineered sequence
MNGETSRPPALGFSSDNIAGASPEVAQALVKHSSGQAGPYGTDELTAQVKHSSGQADPYGTDELTAQVKRKFCEIFERDVEVFLVPTGTAANALCLSAMTPPWGNIYCHPASHINNDECGAPEFFSNGAKLMTVDGPAAKLDIVRLRERTREKVGDVHTTQPACVSITQATEVGSIYTLDEIEAIGDVCKSSSLGLHMDGSRFANALVSLGCSPAEMTWKAGVDALSFGATKNGVLAAEAIVLFNTSLATEMSYRRKRAGHLTSKYRFLSAQIDAYLTDDLWLRNARKANAAAQRLAQGLEGLGGVEVLGGTEANILFCRLDSAMIDALLKAGFTFGTKRWGPNVVRFVTSFATTAEDVDHLLNQVRLAADRTQER

SEQ ID NO: 109 - DNA, 1128 bp, Artificial sequence
  Engineered sequence
atgaacggtgaaacctcgcgtccgccggcgctgggttttagctctgataatattgctggtgcaagcccggaagtcgcacaggcactcgttaagcacagttcgggccaggcgggtccctatggcaccgacgagttgacggcacaggtcaagcatagctccggccaagctgacccttatggtaccgatgaactgactgctcaagttaaacgtaaattttgcgaaatcttcgaacgcgacgtcgaagtgttcctggttccgaccggtacggcagcaaacgcactgtgtctgtccgcaatgaccccgccgtggggtaatatttactgccatccggcgtcccacatcaacaatgatgaatgtggtgcgccggaatttttctcaaacggcgccaaactgatgaccgttgatggtccggcagctaaactggacattgtccgtctgcgcgaacgtacgcgcgaaaaagtgggtgatgttcataccacgcagccggcatgcgtctctattacccaagctacggaagtgggcagtatctataccctggatgaaattgaagccatcggtgacgtgtgcaaatcatcgagcctgggtctgcacatggatggctctcgttttgctaatgcgctggtgtccctgggctgttcaccggcagaaatgacctggaaagccggtgttgacgcactgagttttggtgcgacgaaaaacggcgttctggcggccgaagcaattgtcctgttcaatacctcgctggctacggaaatgagctatcgtcgcaaacgtgccggccacctgacgagtaaataccgctttctgagcgctcagatcgatgcgtacctgaccgatgacctgtggctgcgtaacgcccgcaaagcaaatgcagctgcgcagcgtctggcccaaggtctggaaggcctgggcggtgttgaagtcctgggcggtaccgaagcaaacattctgttctgtcgcctggattctgccatgatcgacgcactgctgaaagctggctttaagttcgggacgaagcgttggggtccgaacgtggttcgctttgttaccagcttcgctaccacggcggaagatgtggaccacctgctgaatcaggttcgcctggccgcagaccgtacgcaagaacgc

SEQ ID NO: 110 - protein, 376 aa, Artificial sequence
  Engineered sequence
MNGETSRPPALGFSSDNIAGASPEVAQALVKHSSGQAGPYGTDELTAQVKHSSGQADPYGTDELTAQVKRKFCEIFERDVEVFLVPTGTAANALCLSAMTPPWGNIYCHPASHINNDECGAPEFFSNGAKLMTVDGPAAKLDIVRLRERTREKVGDVHTTQPACVSITQATEVGSIYTLDEIEAIGDVCKSSSLGLHMDGSRFANALVSLGCSPAEMTWKAGVDALSFGATKNGVLAAEAIVLFNTSLATEMSYRRKRAGHLTSKYRFLSAQIDAYLTDDLWLRNARKANAAAQRLAQGLEGLGGVEVLGGTEANILFCRLDSAMIDALLKAGFKFGTKRWGPNVVRFVTSFATTAEDVDHLLNQVRLAADRTQER

SEQ ID NO: 111 - DNA, 1128 bp, Artificial sequence
  Engineered sequence
atgaacggtgaaacctcgcgtccgccggcgctgggttttagctctgataatattgctggtgcaagcccggaagtcgcacaggcactcgttaagcacagttcgggccaggcgggtccctatggcaccgacgagttgacggcacaggtcaagcatagctccggccaagctgacccttatggtaccgatgaactgactgctcaagttaaacgtaaattttgcgaaatcttcgaacgcgacgtcgaagtgttcctggttccgaccggtacggcagcaaacgcactgtgtctgtccgcaatgaccccgccgtggggtaatatttactgccatcacgcgtcccacatcaacaatgatgaatgtggtgcgccggaatttttctcaaacggcgccaaactgatgaccgttgatggtccggcagctaaactggacattgtccgtctgcgcgaacgtacgcgcgaaaaagtgggtgatgttcatacgacgcagccggcatgcgtctctattacccaagctacggaagtgggcagtatctataccctggatgaaattgaagccatcggtgacgtgtgcaaatcatcgagcctgggtctgcacatggatggctctcgctttgctaatgcgctggtgtccctgggctgttcaccggcagaaatgacctggaaagccggtgttgacgcactgagttttggtgcgacgaaaaacggcgttctggcggccgaagcaattgtcctgttcaatacctcgctggctacggaaatgagctatcgtcgcaaacgtgccggccacctgatcagtaaataccgctttctgagcgctcagatcgatgcgtacctgaccgatgacctgtggctgcgtaacgcccgcaaagcaaatgcagctgcgcagcgtctggcccaaggtctggaaggcctgggcggtgttgaagtcctgggcggtaccgaagcaaacattctgttctgtcgcctggattctgccatgatcgacgcactgctgaaagctggctttggtttcgggtacgggcgttggggtccgaacgtggttcgctttgttaccagcttcgctaccacggcggaagatgtggaccacctgctgaatcaggttcgcctggccgcagaccgtacgcaagaacgc

SEQ ID NO: 112 - protein, 376 aa, Artificial sequence
  Engineered sequence
MNGETSRPPALGFSSDNIAGASPEVAQALVKHSSGQAGPYGTDELTAQVKHSSGQADPYGTDELTAQVKRKFCEIFERDVEVFLVPTGTAANALCLSAMTPPWGNIYCHHASHINNDECGAPEFFSNGAKLMTVDGPAAKLDIVRLRERTREKVGDVHTTQPACVSITQATEVGSIYTLDEIEAIGDVCKSSSLGLHMDGSRFANALVSLGCSPAEMTWKAGVDALSFGATKNGVLAAEAIVLFNTSLATEMSYRRKRAGHLISKYRFLSAQIDAYLTDDLWLRNARKANAAAQRLAQGLEGLGGVEVLGGTEANILFCRLDSAMIDALLKAGFGFGYGRWGPNVVRFVTSFATTAEDVDHLLNQVRLAADRTQER

SEQ ID NO: 113 - DNA, 1128 bp, Artificial sequence
  Engineered sequence
atgaacggtgaaacctcgcgtccgccggcgctgggttttagctctgaaaatattgctggtgcaagcccggaagtcgcacaggcactcgttaagcacagttcgggccaggcgggtccctatggcaccgacgagttgacggcacaggtcaagcatagctccggccaagctgacccttatggtaccgatgaactgactgctcaagttaaacgtaaattttgcgaaatcttcgaacgcgacgtcgaagtgttcctggttccgaccggtacggcagcaaacgcactgtgtctgtccgcaatgaccccgccgtggggtaatatttactgccatcacgcgtcccacatcaacaatgatgaatgtggtgcgccggaatttttctcaaacggcgccaaactgatgaccgttgatggtccggcagctaaactggacattgtccgtctgcgcgaacgtacgcgcgaaaaagtgggtgatgttcatacgacgcagccggcatgcgtctctattacccaagctacggaagtgggcagtatctataccctggatgaaattgaagccatcggtgacgtgtgcaaatcatcgagcctgggtctgcacatggatggctctcgttttgctaatgcgctggtgtccctgggctgttcaccggcagaaatgacctggaaagccggtgttgacgcactgagttttggtgcgacgaaaaacggcgttctggcggccgaagcaattgtcctgttcaatacctcgctggctacggaaatgagctatcgtcgcaaacgtgccggccacctgatcagtaaataccgctttctgagcgctcagatcgatgcgtacctgaccgatgacctgtggctgcgtaacgcccgcaaagcaaatgcagctgcgcagcgtctggcccaaggtctggaaggcctgggcggtgttgaagtcctgggcggtaccgaagcaaacattctgttctgtcgcctggattctgccatgatcgacgcactgctgaaagctggctttggtttcgggtacaagcgttggggtccgaacgtgtgtcgctttgttaccagcttcgctaccacggcggaagatgtggaccacctgctgaatcaggttcgcctggccgcagaccgtacgcaagaacgc

SEQ ID NO: 114 - protein, 376 aa, Artificial sequence
  Engineered sequence
MNGETSRPPALGFSSENIAGASPEVAQALVKHSSGQAGPYGTDELTAQVKHSSGQADPYGTDELTAQVKRKFCEIFERDVEVFLVPTGTAANALCLSAMTPPWGNIYCHHASHINNDECGAPEFFSNGAKLMTVDGPAAKLDIVRLRERTREKVGDVHTTQPACVSITQATEVGSIYTLDEIEAIGDVCKSSSLGLHMDGSRFANALVSLGCSPAEMTWKAGVDALSFGATKNGVLAAEAIVLFNTSLATEMSYRRKRAGHLISKYRFLSAQIDAYLTDDLWLRNARKANAAAQRLAQGLEGLGGVEVLGGTEANILFCRLDSAMIDALLKAGFGFGYKRWGPNVCRFVTSFATTAEDVDHLLNQVRLAADRTQER

SEQ ID NO: 115 - DNA, 1128 bp, Artificial sequence
  Engineered sequence
atgaacggtgaaacctcgcgtccgccggcgctgggttttagctctgaaaatattgctggtgcaagcccggaagtcgcacaggcactcgttaagcacagttcgggccaggcgggtccctatggcaccgacgagttgacggcacaggtcaagcatagctccggccaagctgacccttatggtaccgatgaactgactgctcaagttaaacgtaaattttgcgaaatcttcgaacgcgacgtcgaagtgttcctggttccgaccggtacggcagcaaacgcactgtgtctgtccgcaatgaccccgccgtggggtaatatttactgccatcacgcgtcccacatcaacaatgatgaatgtggtgcgccggaatttttctcaaacggcgccaaactgatgaccgttgatggtccggcagctaaactggacattgtccgtctgcgcgaacgtacgaaggaaaaagtgggtgatgttcattcgacgcagccggcatgcgtctctattacccaagctacggaagtgggcagtatctataccctggatgaaattgaagccatcggtgacgtgtgcaaatcatcgagcctgggtctgcacatggatggctctcgttttgctaatgcgctggtgtccctgggctgttcaccggcagaaatgacctggaaagccggtgttgacgcactgagttttggtgcgacgaaaaacggcgttctggcggccgaagcaattgtcctgttcaatacctcgctggctacggaaatgagctatcgtcgcaaacgtgccggccacctgatcagtaaataccgctttctgagcgctcagatcgatgcgtacctgaccgatgacctgtggctgcgtaacgcccgcaaagcaaatgcagctgcgcagcgtctggcccaaggtctggaaggcctgggcggtgttgaagtcctgggcggtaccgaagcaaacattctgttctgtcgcctggattctgccatgatcgacgcactgctgaaagctggctttcgcttcgggtacaagcgttggggtccgaacgtggttcgctttgttaccagcttcgctaccacggcggaagatgtggaccacctgctgaatcaggttcgcctggccgcagaccgtacgcaagaacgc

SEQ ID NO: 116 - protein, 376 aa, Artificial sequence
  Engineered sequence
MNGETSRPPALGFSSENIAGASPEVAQALVKHSSGQAGPYGTDELTAQVKHSSGQADPYGTDELTAQVKRKFCEIFERDVEVFLVPTGTAANALCLSAMTPPWGNIYCHHASHINNDECGAPEFFSNGAKLMTVDGPAAKLDIVRLRERTKEKVGDVHSTQPACVSITQATEVGSIYTLDEIEAIGDVCKSSSLGLHMDGSRFANALVSLGCSPAEMTWKAGVDALSFGATKNGVLAAEAIVLFNTSLATEMSYRRKRAGHLISKYRFLSAQIDAYLTDDLWLRNARKANAAAQRLAQGLEGLGGVEVLGGTEANILFCRLDSAMIDALLKAGFRFGYKRWGPNVVRFVTSFATTAEDVDHLLNQVRLAADRTQER

SEQ ID NO: 117 - DNA, 1128 bp, Artificial sequence
  Engineered sequence
atgaacggtgaaacctcgcgtccgccggcgctgggttttagctctgaaaatattgctggtgcaagcccggaagtcgcacaggcactcgttaagcacagttcgggccaggcgggtccctatggcaccgacgagttgacggcacaggtcaagcatagctccggccaagctgacccttatggtaccgatgaactgactgctcaagttaaacgtaaattttgcgaaatcttcgaacgcgacgtcgaagtgttcctggttccgaccggtacggcagcaaacgcactgtgtctgtccgcaatgaccccgccgtggggtaatatttactgccatcacgcgtcccacatcaacaatgatgaatgtggtgcgccggaatttttctcaaacggcgccaaactgatgaccgttgatggtccggcagctaaactggacattgtccgtctgcgcgaacgtacgcgcgaaaaagtgggtgatgttcatacgacgcagccggcatgcgtctctattacccaagctacggaagtgggcagtatctataccctggatgaaattgaagccatcggtgacgtgtgcaaatcatcgagcctgggtctgcacatggatggctctcgttttgctaatgcgctggtgtccctgggctgttcaccggcagaaatgacctggaaagccggtgttgacgcactgagttttggtgcgacgaaaaacggcgttctggcggccgaagcaattgtcctgttcaatacctcgctggctacggaaatgagctatcgtcgcaaacgtgccggccacctgatcagtaaataccgctttctgagcgctcagatcgatgcgtacctgaccgatgacctgtggctgcgtaacgcccgcaaagcaaatgcagctgcgcagcgtctggcccaaggtctggaaggcctgggcggtgttgaagtcctgggcggtaccgaagcaaacattctgttctgtcgcctggattctgccatgatcgacgcactgctgaaagctggctttggtttcgggtacaagcgttggggtccgaacgtggttcgctttgttaccagcttcgctaccacggcggaagatgtggaccacctgctgaatcaggttcgcctggccgcagaccgtacgcaagaacgc

SEQ ID NO: 118 - protein, 376 aa, Artificial sequence
  Engineered sequence
MNGETSRPPALGFSSENIAGASPEVAQALVKHSSGQAGPYGTDELTAQVKHSSGQADPYGTDELTAQVKRKFCEIFERDVEVFLVPTGTAANALCLSAMTPPWGNIYCHHASHINNDECGAPEFFSNGAKLMTVDGPAAKLDIVRLRERTREKVGDVHTTQPACVSITQATEVGSIYTLDEIEAIGDVCKSSSLGLHMDGSRFANALVSLGCSPAEMTWKAGVDALSFGATKNGVLAAEAIVLFNTSLATEMSYRRKRAGHLISKYRFLSAQIDAYLTDDLWLRNARKANAAAQRLAQGLEGLGGVEVLGGTEANILFCRLDSAMIDALLKAGFGFGYKRWGPNVVRFVTSFATTAEDVDHLLNQVRLAADRTQER

SEQ ID NO: 119 - DNA, 1128 bp, Artificial sequence
  Engineered sequence
atgaacggtgaaacctcgcgtccgccggcgctgggttttagctctgaaaatattgctggtgcaagcccggaagtcgcacaggcactcgttaagcacagttcgggccaggcgggtccctatggcaccgacgagttgacggcacaggtcaagcatagctccggccaagctgacccttatggtaccgatgaactgactgctcaagttaaacgtaaattttgcgaaatcttcgaacgcgacgtcgaagtgttcctggttccgaccggtacggcagcaaacgcactgtgtctgtccgcaatgaccccgccgtggggtaatatttactgccatcacgcgtcccacatcaacaatgatgaatgtggtgcgccggaatttttctcaaacggcgccaaactgatgaccgttgatggtccggcagctaaactggacattgtccgtctgcgcgaacgtacgtccgaaaaagtgggtgatgttcatacgacgcagccggcatgcgtctctattacccaagctacggaagtgggcagtatctataccctggatgaaattgaagccatcggtgacgtgtgcaaatcatcgagcctgggtctgcacatggatggctctcgttttgctaatgcgctggtgtccctgggctgttcaccggcagaaatgacctggaaagccggtgttgacgcactgagttttggtgcgacgaaaaacggcgttctggcggccgaagcaattgtcctgttcaatacctcgctggctacggaaatgagctatcgtcgcaaacgtgccggccacctgatcagtaaataccgctttctgagcgctcagatcgatgcgtacctgaccgatgacctgtggctgcgtaacgcccgcaaagcaaatgcagctgcgcagcgtctggcccaaggtctggaaggcctgggcggtgttgaagtcctgggcggtaccgaagcaaacattctgttctgtcgcctggattctgccatgatcgacgcactgctgaaagctggctttaaattcgggtacaagcgttggggtccgaacgtggttcgctttgttaccagcttcgctaccacggcggaagatgtggaccacctgctgaatcaggttcgcctggccgcagaccgtacgcaagaacgc

SEQ ID NO: 120 - protein, 376 aa, Artificial sequence
  Engineered sequence
MNGETSRPPALGFSSENIAGASPEVAQALVKHSSGQAGPYGTDELTAQVKHSSGQADPYGTDELTAQVKRKFCEIFERDVEVFLVPTGTAANALCLSAMTPPWGNIYCHHASHINNDECGAPEFFSNGAKLMTVDGPAAKLDIVRLRERTSEKVGDVHTTQPACVSITQATEVGSIYTLDEIEAIGDVCKSSSLGLHMDGSRFANALVSLGCSPAEMTWKAGVDALSFGATKNGVLAAEAIVLFNTSLATEMSYRRKRAGHLISKYRFLSAQIDAYLTDDLWLRNARKANAAAQRLAQGLEGLGGVEVLGGTEANILFCRLDSAMIDALLKAGFKFGYKRWGPNVVRFVTSFATTAEDVDHLLNQVRLAADRTQER

SEQ ID NO: 121 - DNA, 1128 bp, Artificial sequence
  Engineered sequence
atgaacggtgaaacctcgcgtccgccggcgctgggttttagctctgaaaatattgctggtgcaagcccggaagtcgcacaggcactcgttaagcacagttcgggccaggcgggtccctatggcaccgacgagttgacggcacaggtcaagcatagctccggccaagctgacccttatggtaccgatgaactgactgctcaagttaaacgtaaattttgcgaaatcttcgaacgcgacgtcgaagtgttcctggttccgaccggtacggcagcaaacgcactgtgtctgtccgcaatgaccccgccgtggggtaatatttactgccatcacgcgtcccacatcaacaatgatgaatgtggtgcgccggaatttttctcaaacggcgccaaactgatgaccgttgatggtccggcagctaaactggacattgtccgtctgcgcgaacgtacgaacgaaaaagtgggtgatgttcattcgacgcagccggcatgcgtctctattacccaagctacggaagtgggcagtatctataccctggatgaaattgaagccatcggtgacgtgtgcaaatcatcgagcctgggtctgcacatggatggctctcgttttgctaatgcgctggtgtccctgggctgttcaccggcagaaatgacctggaaagccggtgttgacgcactgagttttggtgcgacgaaaaacggcgttctggcggccgaagcaattgtcctgttcaatacctcgctggctacggaaatgagctatcgtcgcaaacgtgccggccacctgatcagtaaataccgctttctgagcgctcagatcgatgcgtacctgaccgatgacctgtggctgcgtaacgcccgcaaagcaaatgcagctgcgcagcgtctggcccaaggtctggaaggcctgggcggtgttgaagtcctgggcggtaccgaagcaaacattctgttctgtcgcctggattctgccatgatcgacgcactgctgaaagctggctttaaattcgggtacaagcgttggggtccgaacgtggttcgctttgttaccagcttcgctaccacggcggaagatgtggaccacctgctgaatcaggttcgcctggccgcagaccgtacgcaagaacgc

SEQ ID NO: 122 - protein, 376 aa, Artificial sequence
  Engineered sequence
MNGETSRPPALGFSSENIAGASPEVAQALVKHSSGQAGPYGTDELTAQVKHSSGQADPYGTDELTAQVKRKFCEIFERDVEVFLVPTGTAANALCLSAMTPPWGNIYCHHASHINNDECGAPEFFSNGAKLMTVDGPAAKLDIVRLRERTNEKVGDVHSTQPACVSITQATEVGSIYTLDEIEAIGDVCKSSSLGLHMDGSRFANALVSLGCSPAEMTWKAGVDALSFGATKNGVLAAEAIVLFNTSLATEMSYRRKRAGHLISKYRFLSAQIDAYLTDDLWLRNARKANAAAQRLAQGLEGLGGVEVLGGTEANILFCRLDSAMIDALLKAGFKFGYKRWGPNVVRFVTSFATTAEDVDHLLNQVRLAADRTQER

SEQ ID NO: 123 - DNA, 1128 bp, Artificial sequence
  Engineered sequence
atgaacggtgaaacctcgcgtccgccggcgctgggttttagctctgaaaatattgctggtgcaagcccggaagtcgcacaggcactcgttaagcacagttcgggccaggcgggtccctatggcaccgacgagttgacggcacaggtcaagcatagctccggccaagctgacccttatggtttcgatgaactgactgctcaagttaaacgtaaattttgcgaaatcttcgaacgcgacgtcgaagtgttcctggttccaaccggtacggcagcaaacgcactgtgtctgtccgcaatgaccccgccgtggggtaatatttactgccatcacgcgtcccacatcaacaatgatgaatgtggtgcgccggaatttttctcaaacggcgccaaactgatgaccgttgatggtccggcagctaaactggacattgtccgtctgcgcgaacgtacgcgcgaaaaagtgggtgatgttcattcgacgcagccggcatgcgtctctattacccaagctacggaagtgggcagtatctataccctggatgaaattgaagccatcggtgacgtgtgcaaatcatcgagcctgggtctgcacatggatggcgcccgttttgctaatgcgctggtgtccctgggctgttcaccggcagaaatgacctggaaagccggtgttgacgcactgagttttggtgcgacgaaaaacggcgttctggcggccgaagcaattgtcctgttcaatacctcgctggctacggaaatgagctatcgtcgcaaacgtgccggccacctgatcagtaaataccgctttctgagcgctcagatcgatgcgtacctgaccgatgacctgtggctgcgtaacgcccgcaaagcaaatgcagctgcgcagcgtctggcccaaggtctggaaggcctgggcggtgttgaagtcctgggcggtaccgaagcaaacattctgttctgtcgcctggattctgccatgatcgacgcactgctgaaagctggctttaaattcgggtacaagcgttggggtccgaacgtggttcgctttgttaccagcttcgctaccacggcggaagatgtggaccacctgctgaatcaggttcgcctggccgcagaccgtacgcaagaacgc

SEQ ID NO: 124 - protein, 376 aa, Artificial sequence
  Engineered sequence
MNGETSRPPALGFSSENIAGASPEVAQALVKHSSGQAGPYGTDELTAQVKHSSGQADPYGFDELTAQVKRKFCEIFERDVEVFLVPTGTAANALCLSAMTPPWGNIYCHHASHINNDECGAPEFFSNGAKLMTVDGPAAKLDIVRLRERTREKVGDVHSTQPACVSITQATEVGSIYTLDEIEAIGDVCKSSSLGLHMDGARFANALVSLGCSPAEMTWKAGVDALSFGATKNGVLAAEAIVLFNTSLATEMSYRRKRAGHLISKYRFLSAQIDAYLTDDLWLRNARKANAAAQRLAQGLEGLGGVEVLGGTEANILFCRLDSAMIDALLKAGFKFGYKRWGPNVVRFVTSFATTAEDVDHLLNQVRLAADRTQER

SEQ ID NO: 125 - DNA, 1128 bp, Artificial sequence
  Engineered sequence
atgaacggtgaaacctcgcgtccgccggcgctgggttttagctctgaaaatattgctggtgcaagcccggaagtcgcacaggcactcgttaagcacagttcgggccaggcgggtccctatggcaccgacgagttgacggcacaggtcaagcatagctccggccaagctgacccttatggtttcgatgaactgactgctcaagttaaacgtaaattttgcgaaatcttcgaacgcgacgtcgaagtgttcctggttggaaccggtacggcagcaaacgcactgtgtctgtccgcaatgaccccgccgtggggtaatatttactgccatcacgcgtcccacatcaacaatgatgaatgtggtgcgccggaatttttctcaaacggcgccaaactgatgaccgttgatggtccggcagctaaactggacattgtccgtctgcgcgaacgtacgcgcgaaaaagtgggtgatgttcatacgacgcagccggcatgcgtctctattacccaagctacggaagtgggcagtatctataccctggatgaaattgaagccatcggtgacgtgtgcaaatcatcgagcctgggtctgcacatggatggcgcccgttttgctaatgcgctggtgtccctgggctgttcaccggcagaaatgacctggaaagccggtgttgacgcactgagttttggtgcgacgaaaaacggcgttctggcggccgaagcaattgtcctgttcaatacctcgctggctacggaaatgagctatcgtcgcaaacgtgccggccacctgatcagtaaataccgctttctgagcgctcagatcgatgcgtacctgaccgatgacctgtggctgcgtaacgcccgcaaagcaaatgcagctgcgcagcgtctggcccaaggtctggaaggcctgggcggtgttgaagtcctgggcggtaccgaagcaaacattctgttctgtcgcctggattctgccatgatcgacgcactgctgaaagctggctttaaattcgggtacaagcgttggggtccgaacgtggttcgctttgttaccagcttcgctaccacggcggaagatgtggaccacctgctgaatcaggttcgcctggccgcagaccgtacgcaagaacgc

SEQ ID NO: 126 - protein, 376 aa, Artificial sequence
  Engineered sequence
MNGETSRPPALGFSSENIAGASPEVAQALVKHSSGQAGPYGTDELTAQVKHSSGQADPYGFDELTAQVKRKFCEIFERDVEVFLVGTGTAANALCLSAMTPPWGNIYCHHASHINNDECGAPEFFSNGAKLMTVDGPAAKLDIVRLRERTREKVGDVHTTQPACVSITQATEVGSIYTLDEIEAIGDVCKSSSLGLHMDGARFANALVSLGCSPAEMTWKAGVDALSFGATKNGVLAAEAIVLFNTSLATEMSYRRKRAGHLISKYRFLSAQIDAYLTDDLWLRNARKANAAAQRLAQGLEGLGGVEVLGGTEANILFCRLDSAMIDALLKAGFKFGYKRWGPNVVRFVTSFATTAEDVDHLLNQVRLAADRTQER

SEQ ID NO: 127 - DNA, 1128 bp, Artificial sequence
  Engineered sequence
atgaacggtgaaacctcgcgtccgccggcgctgggttttagctctgaaaatattgctggtgcaagcccggaagtcgcacaggcactcgttaagcacagttcgggccaggcgggtccctatggcaccgacgagttgacggcacaggtcaagcatagctccggccaagctgacccttatggtttcgatgaactgactgctcaagttaaacgtaaattttgcgaaatcttcgaacgcgacgtcgaagtgttcctggttgccaccggtacggcagcaaacgcactgtgtctgtccgcaatgaccccgccgtggggtaatatttactgccatcacgcgtcccacatcaacaatgatgaatgtggtgcgccggaatttttctcaaacggcgccaaactgatgaccgttgatggtccggcagctaaactggacattgtccgtctgcgcgaacgtacgcgcgaaaaagtgggtgatgttcatacgacgcagccggcatgcgtctctattacccaagctacggaagtgggcagtatctataccctggatgaaattgaagccatcggtgacgtgtgcaaatcatcgagcctgggtctgcacatggatggcgcccgttttgctaatgcgctggtgtccctgggctgttcaccggcagaaatgacctggaaagccggtgttgacgcactgagttttggtgcgacgaaaaacggcgttctggcggccgaagcaattgtcctgttcaatacctcgctggctacggaaatgagctatcgtcgcaaacgtgccggccacctgatcagtaaataccgctttctgagcgctcagatcgatgcgtacctgaccgatgacctgtggctgcgtaacgcccgcaaagcaaatgcagctgcgcagcgtctggcccaaggtctggaaggcctgggcggtgttgaagtcctgggcggtaccgaagcaaacattctgttctgtcgcctggattctgccatgatcgacgcactgctgaaagctggctttaaattcgggtacgagcgttggggtccgaacgtggttcgctttgttaccagcttcgctaccacggcggaagatgtggaccacctgctgaatcaggttcgcctggccgcagaccgtacgcaagaacgc

SEQ ID NO: 128 - protein, 376 aa, Artificial sequence
  Engineered sequence
MNGETSRPPALGFSSENIAGASPEVAQALVKHSSGQAGPYGTDELTAQVKHSSGQADPYGFDELTAQVKRKFCEIFERDVEVFLVATGTAANALCLSAMTPPWGNIYCHHASHINNDECGAPEFFSNGAKLMTVDGPAAKLDIVRLRERTREKVGDVHTTQPACVSITQATEVGSIYTLDEIEAIGDVCKSSSLGLHMDGARFANALVSLGCSPAEMTWKAGVDALSFGATKNGVLAAEAIVLFNTSLATEMSYRRKRAGHLISKYRFLSAQIDAYLTDDLWLRNARKANAAAQRLAQGLEGLGGVEVLGGTEANILFCRLDSAMIDALLKAGFKFGYERWGPNVVRFVTSFATTAEDVDHLLNQVRLAADRTQER

SEQ ID NO: 129 - DNA, 1128 bp, Artificial sequence
  Engineered sequence
atgaacggtgaaacctcgcgtccgccggcgctgggttttagctctgaaaatattgctggtgcaagcccggaagtcgcacaggcactcgttaagcacagttcgggccaggcgggtccctatggcaccgacgagttgacggcacaggtcaagcatagctccggccaagctgacccttatggtaccgatgaactgactgctcaagttaaacgtaaattttgcgaaatcttcgaacgcgacgtcgaagtgttcctggttgccaccggtacggcagcaaacgcactgtgtctgtccgcaatgaccccgccgtggggtaatatttactgccatcacgcgtcccacatcaacaatgatgaatgtggtgcgccggaatttttctcaaacggcgccaaactgatgaccgttgatggtccggcagctaaactggacattgtccgtctgcgcgaacgtacgcgcgaaaaagtgggtgatgttcatacgacgcagccggcatgcgtctctattacccaagctacggaagtgggcagtatctataccctggatgaaattgaagccatcggtgacgtgtgcaaatcatcgagcctgggtctgcacatggatggcgcccgttttgctaatgcgctggtgtccctgggctgttcaccggcagaaatgacctggaaagccggtgttgacgcactgagttttggtgcgacgaaaaacggcgttctggcggccgaagcaattgtcctgttcaatacctcgctggctacggaaatgagctatcgtcgcaaacgtgccggccacctgatcagtaaataccgctttctgagcgctcagatcgatgcgtacctgaccgatgacctgtggctgcgtaacgcccgcaaagcaaatgcagctgcgcagcgtctggcccaaggtctggaaggcctgggcggtgttgaagtcctgggcggtaccgaagcaaacattctgttctgtcgcctggattctgccatgatcgacgcactgctgaaagctggctttaaattcgggtacaagcgttggggtccgaacgtggttcgctttgttaccagcttcgctaccacggcggaagatgtggaccacctgctgaatcaggttcgcctggccgcagaccgtacgcaagaacgc

SEQ ID NO: 130 - protein, 376 aa, Artificial sequence
  Engineered sequence
MNGETSRPPALGFSSENIAGASPEVAQALVKHSSGQAGPYGTDELTAQVKHSSGQADPYGTDELTAQVKRKFCEIFERDVEVFLVATGTAANALCLSAMTPPWGNIYCHHASHINNDECGAPEFFSNGAKLMTVDGPAAKLDIVRLRERTREKVGDVHTTQPACVSITQATEVGSIYTLDEIEAIGDVCKSSSLGLHMDGARFANALVSLGCSPAEMTWKAGVDALSFGATKNGVLAAEAIVLFNTSLATEMSYRRKRAGHLISKYRFLSAQIDAYLTDDLWLRNARKANAAAQRLAQGLEGLGGVEVLGGTEANILFCRLDSAMIDALLKAGFKFGYKRWGPNVVRFVTSFATTAEDVDHLLNQVRLAADRTQER

SEQ ID NO: 131 - DNA, 1128 bp, Artificial sequence
  Engineered sequence
atgaacggtgaaacctcgcgtccgccggcgctgggttttagctctgaaaatattgctggtgcaagcccggaagtcgcacaggcactcgttaagcacagttcgggccaggcgggtccctatggcaccgacgagttgacggcacaggtcaagcatagctccggccaagctgacccttatggtaccgatgaactgactgctcaagttaaacgtaaattttgcgaaatcttcgaacgcgacgtcgaagtgttcctggttgccaccggtacggcagcaaacgcactgtgtctgtccgcaatgaccccgccgtggggtaatatttactgccatcacgcgtcccacatcaacaatgatgaatgtggtgcgccggaatttttctcaaacggcgccaaactgatgaccgttgatggtccggcagctaaactggacattgtccgtctgcgcgaacgtacgcgcgaaaaagtgggtgatgttcatacgacgcagccggcatgcgtctctattacccaagctacggaagtgggcagtatctataccctggatgaaattgaagccatcggtgacgtgtgcaaatcatcgagcctgggtctgcacatggatggcgcccgttttgctaatgcgctggtgtccctgggctgttcaccggcagaaatgacctggaaagccggtgttgacgcactgagttttggtgcgacgaaaaacggcgttctggcggccgaagcaattgtcctgttcaatacctcgctggctacggaaatgagctatcgtcgcaaacgtgccggccacctgatcagtaaataccgctttctgagcgctcagatcgatgcgtacctgaccgatgacctgtggctgcgtaacgcccgcaaagcaaatgcagctgcgcagcgtctggcccaaggtctggaaggcctgggcggtgttgaagtcctgggcggtaccgaagcaaacattctgttctgtcgcctggattctgccatgatcgacgcactgctgaaagctggctttcgcttcgggtacaagcgttggggtccgaacgtggttcgctttgttaccagcttcgctaccacggcggaagatgtggaccacctgctgaatcaggttcgcctggccgcagaccgtacgcaagaacgc

SEQ ID NO: 132 - protein, 376 aa, Artificial sequence
  Engineered sequence
MNGETSRPPALGFSSENIAGASPEVAQALVKHSSGQAGPYGTDELTAQVKHSSGQADPYGTDELTAQVKRKFCEIFERDVEVFLVATGTAANALCLSAMTPPWGNIYCHHASHINNDECGAPEFFSNGAKLMTVDGPAAKLDIVRLRERTREKVGDVHTTQPACVSITQATEVGSIYTLDEIEAIGDVCKSSSLGLHMDGARFANALVSLGCSPAEMTWKAGVDALSFGATKNGVLAAEAIVLFNTSLATEMSYRRKRAGHLISKYRFLSAQIDAYLTDDLWLRNARKANAAAQRLAQGLEGLGGVEVLGGTEANILFCRLDSAMIDALLKAGFRFGYKRWGPNVVRFVTSFATTAEDVDHLLNQVRLAADRTQER

SEQ ID NO: 133 - DNA, 1128 bp, Artificial sequence
  Engineered sequence
atgaacggtgaaacctcgcgtccgccggcgctgggttttagctctgaaaatattgctggtgcaagcccggaagtcgcacaggcactcgttaagcacagttcgggccaggcgggtccctatggcaccgacgagttgacggcacaggtcaagcatagctccggccaagctgacccttatggtaccgatgaactgactgctcaagttaaacgtaaattttgcgaaatcttcgaacgcgacgtcgaagtgttcctggttgccaccggtacggcagcaaacgcactgtgtctgtccgcaatgaccccgccgtggggtaatatttactgccatcacgcgtcccacatcaacaatgatgaatgtggtgcgccggaatttttctcaaacggcgccaaactgatgaccgttgatggtccggcagctaaactggacattgtccgtctgcgcgaacgtacgcgcgaaaaagtgggtgatgttcatacgacgcagccggcatgcgtctctattacccaagctacggaagtgggcagtatctataccctggatgaaattgaagccatcggtgacgtgtgcaaatcatcgagcctgggtctgcacatggatggcgcccgttttgctaatgcgctggtgtccctgggctgttcaccggcagaaatgacctggaaagccggtgttgacgcactgagttttggtgcgacgaaaaacggcgttctggcggccgaagcaattgtcctgttcaatacctcgctggctacggaaatgagctatcgtcacaaacgtgccggccacctgatcagtaaataccgctttctgagcgctcagatcgatgcgtacctgaccgatgacctgtggctgcgtaacgcccgcaaagcaaatgcagctgcgcagcgtctggcccaaggtctggaaggcctgggcggtgttgaagtcctgggcggtaccgaagcaaacattctgttctgtcgcctggattctgccatgatcgacgcactgctgaaagctggctttaaattcgggtacaagcgttggggtccgaacgtggttcgctttgttaccagcttcgctaccacggcggaagatgtggaccacctgctgaatcaggttcgcctggccgcagaccgtacgcaagaacgc

SEQ ID NO: 134 - protein, 376 aa, Artificial sequence
  Engineered sequence
MNGETSRPPALGFSSENIAGASPEVAQALVKHSSGQAGPYGTDELTAQVKHSSGQADPYGTDELTAQVKRKFCEIFERDVEVFLVATGTAANALCLSAMTPPWGNIYCHHASHINNDECGAPEFFSNGAKLMTVDGPAAKLDIVRLRERTREKVGDVHTTQPACVSITQATEVGSIYTLDEIEAIGDVCKSSSLGLHMDGARFANALVSLGCSPAEMTWKAGVDALSFGATKNGVLAAEAIVLFNTSLATEMSYRHKRAGHLISKYRFLSAQIDAYLTDDLWLRNARKANAAAQRLAQGLEGLGGVEVLGGTEANILFCRLDSAMIDALLKAGFKFGYKRWGPNVVRFVTSFATTAEDVDHLLNQVRLAADRTQER

SEQ ID NO: 135 - DNA, 1128 bp, Artificial sequence
  Engineered sequence
atgaacggtgaaacctcgcgtccgccggcgctgggttttagctctgaaaatattgctggtgcaagcccggaagtcgcacaggcactcgttaagcacagttcgggccaggcgggtccctatggcaccgacgagttgacggcacaggtcaagcatagctccggccaagctgacccttatggtaccgatgaactgactgctcaagttaaacgtaaattttgcgaaatcttcgaacgcgacgtcgaagtgttcctggttccaaccggtacggcagcaaacgcactgtgtctgtccgcaatgaccccgccgtggggtaatatttactgccatcacgcgtcccacatcaacaatgatgaatgtggtgcgccggaatttttctcaaacggcgccaaactgatgaccgttgatggtccggcagctaaactggacattgtccgtctgcgcgaacgtacgcgcgaaaaagtgggtgatgttcatacgacgcagccggcatgcgtctctattacccaagctacggaagtgggcagtatctataccctggatgaaattgaagccatcggtgacgtgtgcaaatcatcgagcctgggtctgcacatggatggctcacgttttgctaatgcgctggtgtccctgggctgttcaccggcagaaatgacctggaaagccggtgttgacgcactgagttttggtgcgacgaaaaacggcgttctggcggccgaagcaattgtcctgttcaatacctcgctggctacggaaatgagctatcgtcgcaaacgtgccggccacctgatcagtaaataccgctttctgagcgctcagatcgatgcgtacctgaccgatgacctgtggctgcgtaacgcccgcaaagcaaatgcagctgcgcagcgtctggcccaaggtctggaaggcctgggcggtgttgaagtcctgggcggtaccgaagcaaacattctgttctgtcgcctggattctgccatgatcgacgcactgctgaaagctggctttaaattcgggtacaagcgttggggtccgaacgtggttcgctttgttaccagcttcgctaccacggcggaagatgtggaccacctgctgaatcaggttcgcctggccgcagaccgtacgcaagaacgc

SEQ ID NO: 136 - protein, 376 aa, Artificial sequence
  Engineered sequence
MNGETSRPPALGFSSENIAGASPEVAQALVKHSSGQAGPYGTDELTAQVKHSSGQADPYGTDELTAQVKRKFCEIFERDVEVFLVPTGTAANALCLSAMTPPWGNIYCHHASHINNDECGAPEFFSNGAKLMTVDGPAAKLDIVRLRERTREKVGDVHTTQPACVSITQATEVGSIYTLDEIEAIGDVCKSSSLGLHMDGSRFANALVSLGCSPAEMTWKAGVDALSFGATKNGVLAAEAIVLFNTSLATEMSYRRKRAGHLISKYRFLSAQIDAYLTDDLWLRNARKANAAAQRLAQGLEGLGGVEVLGGTEANILFCRLDSAMIDALLKAGFKFGYKRWGPNVVRFVTSFATTAEDVDHLLNQVRLAADRTQER

SEQ ID NO: 137 - DNA, 1128 bp, Artificial sequence
  Engineered sequence
atgaacggtgaaacctcgcgtccgccggcgctgggttttagctctgaaaatattgctggtgcaagcccggaagtcgcacaggcactcgttaagcacagttcgggccaggcgggtccctatggcaccgacgagttgacggcacaggtcaagcatagctccggccaagctgacccttatggtaccgatgaactgactgctcaagttaaacgtaaattttgcgaaatcttcgaacgcgacgtcgaagtgttcctggttgccaccggtacggcagcaaacgcactgtgtctgtccgcaatgaccccgccgtggggtaatatttactgccatcacgcgtcccacatcaacaatgatgaatgtggtgcgccggaatttttctcaaacggcgccaaactgatgaccgttgatggtccggcagctaaactggacattgtccgtctgcgcgaacgtacgcgcgaaaaagtgggtgatgttcatacgacgcagccggcatgcgtctctattacccaagctacggaagtgggcagtatctataccctggatgaaattgaagccatcggtgacgtgtgcaaatcatcgagcctgggtctgcacatggatggctcacgttttgctaatgcgctggtgtccctgggctgttcaccggcagaaatgacctggaaagccggtgttgacgcactgagttttggtgcgacgaaaaacggcgttctggcggccgaagcaattgtcctgttcaatacctcgctggctacggaaatgagctatcgtcgcaaacgtgccggccacctgatcagtaaataccgctttctgagcgctcagatcgatgcgtacctgaccgatgacctgtggctgcgtaacgcccgcaaagcaaatgcagctgcgcagcgtctggcccaaggtctggaaggcctgggcggtgttgaagtcctgggcggtaccgaagcaaacattctgttctgtcgcctggattctgccatgatcgacgcactgctgaaagctggctttaaattcgggtacaagcgttggggtccgaacgtggttcgctttgttaccagcttcgctaccacggcggaagatgtggaccacctgctgaatcaggttcgcctggccgcagaccgtacgcaagaacgc

SEQ ID NO: 138 - protein, 376 aa, Artificial sequence
  Engineered sequence
MNGETSRPPALGFSSENIAGASPEVAQALVKHSSGQAGPYGTDELTAQVKHSSGQADPYGTDELTAQVKRKFCEIFERDVEVFLVATGTAANALCLSAMTPPWGNIYCHHASHINNDECGAPEFFSNGAKLMTVDGPAAKLDIVRLRERTREKVGDVHTTQPACVSITQATEVGSIYTLDEIEAIGDVCKSSSLGLHMDGSRFANALVSLGCSPAEMTWKAGVDALSFGATKNGVLAAEAIVLFNTSLATEMSYRRKRAGHLISKYRFLSAQIDAYLTDDLWLRNARKANAAAQRLAQGLEGLGGVEVLGGTEANILFCRLDSAMIDALLKAGFKFGYKRWGPNVVRFVTSFATTAEDVDHLLNQVRLAADRTQER

SEQ ID NO: 139 - DNA, 1128 bp, Artificial sequence
  Engineered sequence
atgaacggtgaaacctcgcgtccgccggcgctgggttttagctctgaaaatattgctggtgcaagcccggaagtcgcacaggcactcgttaagcacagttcgggccaggcgggtccctatggcaccgacgagttgacggcacaggtcaagcatagctccggccaagctgacccttatggtaccgatgaactgactgctcaagttaaacgtaaattttgcgaaatcttcgaacgcgacgtcgaagtgttcctggttccgaccggtacggcagcaaacgcactgtgtctgtccgcaatgaccccgccgtggggtaatatttactgccatcacgcgtcccacatcaacaatgatgaatgtggtgcgccggaatttttctcaaacggcgccaaactgatgaccgttgatggtccggcagctaaactggacattgtccgtctgcgcgaacgtacgaaggaaaaagtgggtgatgttcatacgacgcagccggcatgcgtctctattacccaagctacggaagtgggcagtatctataccctggatgaaattgaagccatcggtgacgtgtgcaaatcatcgagcctgggtctgcacatggatggctctcgttttgctaatgcgctggtgtccctgggctgttcaccggcagaaatgacctggaaagccggtgttgacgcactgagttttggtgcgacgaaaaacggcgttctggcggccgaagcaattgtcctgttcaatacctcgctggctacggaaatgagctatcgtcgcaaacgtgccggccacctgatcagtaaataccgctttctgagcgctcagatcgatgcgtacctgaccgatgacctgtggctgcgtaacgcccgcaaagcaaatgcagctgcgcagcgtctggcccaaggtctggaaggcctgggcggtgttgaagtcctgggcggtaccgaagcaaacattctgttctgtcgcctggattctgccatgatcgacgcactgctgaaagctggctttaaattcgggtacaagcgttggggtccgaacgtggttcgctttgttaccagcttcgctaccacggcggaagatgtggaccacctgctgaatcaggttcgcctggccgcagaccgtacgcaagaacgc

SEQ ID NO: 140 - protein, 376 aa, Artificial sequence
  Engineered sequence
MNGETSRPPALGFSSENIAGASPEVAQALVKHSSGQAGPYGTDELTAQVKHSSGQADPYGTDELTAQVKRKFCEIFERDVEVFLVPTGTAANALCLSAMTPPWGNIYCHHASHINNDECGAPEFFSNGAKLMTVDGPAAKLDIVRLRERTKEKVGDVHTTQPACVSITQATEVGSIYTLDEIEAIGDVCKSSSLGLHMDGSRFANALVSLGCSPAEMTWKAGVDALSFGATKNGVLAAEAIVLFNTSLATEMSYRRKRAGHLISKYRFLSAQIDAYLTDDLWLRNARKANAAAQRLAQGLEGLGGVEVLGGTEANILFCRLDSAMIDALLKAGFKFGYKRWGPNVVRFVTSFATTAEDVDHLLNQVRLAADRTQER

SEQ ID NO: 141 - DNA, 1128 bp, Artificial sequence
  Engineered sequence
atgaacggtgaaacctcgcgtccgccggcgctgggttttagctctgaaaatattgttggtgcaagcccggaagtcgcacaggcactcgttaagcacagttcgggccaggcgggtccctatggcaccgacgagttgacggcacaggtcaagcatagctccggccaagctgacccttatggtaccgatgaactgactgctcaagttaaacgtaaattttgcgaaatcttcgaacgcgacgtcgaagtgttcctggttccgaccggtacggcagcaaacgcactgtgtctgtccgcaatgaccccgccgtggggtaatatttactgccatcacgcgtcccacatcaacaatgatgaatgtggtgcgccggaatttttctcaaacggcgccaaactgatgaccgttgatggtccggcagctaaactggacattgtccgtctgcgcgaacgtacgtccgaaaaagtgggtgatgttcatacgacgcagccggcatgcgtctctattacccaagctacggaagtgggcagtatctataccctggatgaaattgaagccatcggtgacgtgtgcaaatcatcgagcctgggtctgcacatggatggctctcgttttgctaatgcgctggtgtccctgggctgttcaccggcagaaatgacctggaaagccggtgttgacgcactgagttttggtgcgacgaaaaacggcgttctggcggccgaagcaattgtcctgttcaatacctcgctggctacggaaatgagctatcgtcgcaaacgtgccggccacctgatcagtaaataccgctttctgagcgctcagatcgatgcgtacctgaccgatgacctgtggctgcgtaacgcccgcaaagcaaatgcagctgcgcagcgtctggcccaaggtctggaaggcctgggcggtgttgaagtcctgggcggtaccgaagcaaacattctgttctgtcgcctggattctgccatgatcgacgcactgctgaaagctggctttcgcttcgggtacaagcgttggggtccgaacgtggttcgctttgttaccagcttcgctaccacggcggaagatgtggaccacctgctgaatcaggttcgcctggccgcagaccgtacgcaagaacgc

SEQ ID NO: 142 - protein, 376 aa, Artificial sequence
  Engineered sequence
MNGETSRPPALGFSSENIVGASPEVAQALVKHSSGQAGPYGTDELTAQVKHSSGQADPYGTDELTAQVKRKFCEIFERDVEVFLVPTGTAANALCLSAMTPPWGNIYCHHASHINNDECGAPEFFSNGAKLMTVDGPAAKLDIVRLRERTSEKVGDVHTTQPACVSITQATEVGSIYTLDEIEAIGDVCKSSSLGLHMDGSRFANALVSLGCSPAEMTWKAGVDALSFGATKNGVLAAEAIVLFNTSLATEMSYRRKRAGHLISKYRFLSAQIDAYLTDDLWLRNARKANAAAQRLAQGLEGLGGVEVLGGTEANILFCRLDSAMIDALLKAGFRFGYKRWGPNVVRFVTSFATTAEDVDHLLNQVRLAADRTQER

SEQ ID NO: 143 - DNA, 1128 bp, Artificial sequence
  Engineered sequence
atgaacggtgaaacctcgcgtccgccggcgctgggttttagctctgaaaatattgctggtgcaagcccggaagtcgcacaggcactcgttaagcacagttcgggccaggcgggtccctatggcaccgacgagttgacggcacaggtcaagcatagctccggccaagctgacccttatggtaccgatgaactgactgctcaagttaaacgtaaattttgcgaaatcttcgaacgcgacgtcgaagtgttcctggttccgaccggtacggcagcaaacgcactgtgtctgtccgcaatgaccccgccgtggggtaatatttactgccatcacgcgtcccacatcaacaatgatgaatgtggtgcgccggaatttttctcaaacggcgccaaactgatgaccgttgatggtccggcagctaaactggacattgtccgtctgcgcgaacgtacgtccgaaaaagtgggtgatgttcattcgacgcagccggcatgcgtctctattacccaagctacggaagtgggcagtatctataccctggatgaaattgaagccatcggtgacgtgtgcaaatcatcgagcctgggtctgcacatggatggctctcgttttgctaatgcgctggtgtccctgggctgttcaccggcagaaatgacctggaaagccggtgttgacgcactgagttttggtgcgacgaaaaacggcgttctggcggccgaagcaattgtcctgttcaatacctcgctggctacggaaatgagctatcgtcgcaaacgtgccggccacctgatcagtaaataccgctttctgagcgctcagatcgatgcgtacctgaccgatgacctgtggctgcgtaacgcccgcaaagcaaatgcagctgcgcagcgtctggcccaaggtctggaaggcctgggcggtgttgaagtcctgggcggtaccgaagcaaacattctgttctgtcgcctggattctgccatgatcgacgcactgctgaaagctggctttaaattcgggtacaagcgttggggtccgaacgtggttcgctttgttaccagcttcgctaccacggcggaagatgtggaccacctgctgaatcaggttcgcctggccgcagaccgtacgcaagaacgc

SEQ ID NO: 144 - protein, 376 aa, Artificial sequence
  Engineered sequence
MNGETSRPPALGFSSENIAGASPEVAQALVKHSSGQAGPYGTDELTAQVKHSSGQADPYGTDELTAQVKRKFCEIFERDVEVFLVPTGTAANALCLSAMTPPWGNIYCHHASHINNDECGAPEFFSNGAKLMTVDGPAAKLDIVRLRERTSEKVGDVHSTQPACVSITQATEVGSIYTLDEIEAIGDVCKSSSLGLHMDGSRFANALVSLGCSPAEMTWKAGVDALSFGATKNGVLAAEAIVLFNTSLATEMSYRRKRAGHLISKYRFLSAQIDAYLTDDLWLRNARKANAAAQRLAQGLEGLGGVEVLGGTEANILFCRLDSAMIDALLKAGFKFGYKRWGPNVVRFVTSFATTAEDVDHLLNQVRLAADRTQER

SEQ ID NO: 145 - DNA, 1128 bp, Artificial sequence
  Engineered sequence
atgaacggtgaaacctcgcgtccgccggcgctgggttttagctctgaaaatattgctggtgcaagcccggaagtcgcacaggcactcgttaagcacagttcgggccaggcgggtccctatggcaccgacgagttgacggcacaggtcaagcatagctccggccaagctgacccttatggtaccgatgaactgactgctcaagttaaacgtaaattttgcgaaatcttcgaacgcgacgtcgaagtgttcctggttccgaccggtacggcagcaaacgcactgtgtctgtccgcaatgaccccgccgtggggtaatatttactgccatcacgcgtcccacatcaacaatgatgaatgtggtgcgccggaatttttctcaaacggcgccaaactgatgaccgttgatggtccggcagctaaactggacattgtccgtctgcgcgaacgtacgaaggaaaaagtgggtgatgttcattcgacgcagccggcatgcgtctctattacccaagctacggaagtgggcagtatctataccctggatgaaattgaagccatcggtgacgtgtgcaaatcatcgagcctgggtctgcacatggatggctctcgttttgctaatgcgctggtgtccctgggctgttcaccggcagaaatgacctggaaagccggtgttgacgcactgagttttggtgcgacgaaaaacggcgttctggcggccgaagcaattgtcctgttcaatacctcgctggctacggaaatgagctatcgtcgcaaacgtgccggccacctgatcagtaaataccgctttctgagcgctcagatcgatgcgtacctgaccgatgacctgtggctgcgtaacgcccgcaaagcaaatgcagctgcgcagcgtctggcccaaggtctggaaggcctgggcggtgttgaagtcctgggcggtaccgaagcaaacattctgttctgtcgcctggattctgccatgatcgacgcactgctgaaagctggctttaaattcgggtacgagcgttggggtccgaacgtggttcgctttgttaccagcttcgctaccacggcggaagatgtggaccacctgctgaatcaggttcgcctggccgcagaccgtacgcaagaacgc

SEQ ID NO: 146 - protein, 376 aa, Artificial sequence
  Engineered sequence
MNGETSRPPALGFSSENIAGASPEVAQALVKHSSGQAGPYGTDELTAQVKHSSGQADPYGTDELTAQVKRKFCEIFERDVEVFLVPTGTAANALCLSAMTPPWGNIYCHHASHINNDECGAPEFFSNGAKLMTVDGPAAKLDIVRLRERTKEKVGDVHSTQPACVSITQATEVGSIYTLDEIEAIGDVCKSSSLGLHMDGSRFANALVSLGCSPAEMTWKAGVDALSFGATKNGVLAAEAIVLFNTSLATEMSYRRKRAGHLISKYRFLSAQIDAYLTDDLWLRNARKANAAAQRLAQGLEGLGGVEVLGGTEANILFCRLDSAMIDALLKAGFKFGYERWGPNVVRFVTSFATTAEDVDHLLNQVRLAADRTQER

SEQ ID NO: 147 - DNA, 1128 bp, Artificial sequence
  Engineered sequence
atgaacggtgaaacctcgcgtccgccggcgctgggttttagctctgaaaatattgctggtgcaagcccggaagtcgcacaggcactcgttaagcacagttcgggccaggcgggtccctatggcaccgacgagttgacggcacaggtcaagcatagctccggccaagctgacccttatggtaccgatgaactgactgctcaagttaaacgtaaattttgcgaaatcttcgaacgcgacgtcgaagtgttcctggttccgaccggtacggcagcaaacgcactgtgtctgtccgcaatgaccccgccgtggggtaatatttactgccatcacgcgtcccacatcaacaatgatgaatgtggtgcgccggaatttttctcaaacggcgccaaactgatgaccgttgatggtccggcagctaaactggacattgtccgtctgcgcgaacgtacgtccgaaaaagtgggtgatgttcattcgacgcagccggcatgcgtctctattacccaagctacggaagtgggcagtatctataccctggatgaaattgaagccatcggtgacgtgtgcaaatcatcgagcctgggtctgcacatggatggctctcgttttgctaatgcgctggtgtccctgggctgttcaccggcagaaatgacctggaaagccggtgttgacgcactgagttttggtgcgacgaaaaacggcgttctggcggccgaagcaattgtcctgttcaatacctcgctggctacggaaatgagctatcgtcgcaaacgtgccggccacctgatcagtaaataccgctttctgagcgctcagatcgatgcgtacctgaccgatgacctgtggctgcgtaacgcccgcaaagcaaatgcagctgcgcagcgtctggcccaaggtctggaaggcctgggcggtgttgaagtcctgggcggtaccgaagcaaacattctgttctgtcgcctggattctgccatgatcgacgcactgctgaaagctggctttactttcgggtacaagcgttggggtccgaacgtggttcgctttgttaccagcttcgctaccacggcggaagatgtggaccacctgctgaatcaggttcgcctggccgcagaccgtacgcaagaacgc

SEQ ID NO: 148 - protein, 376 aa, Artificial sequence
  Engineered sequence
MNGETSRPPALGFSSENIAGASPEVAQALVKHSSGQAGPYGTDELTAQVKHSSGQADPYGTDELTAQVKRKFCEIFERDVEVFLVPTGTAANALCLSAMTPPWGNIYCHHASHINNDECGAPEFFSNGAKLMTVDGPAAKLDIVRLRERTSEKVGDVHSTQPACVSITQATEVGSIYTLDEIEAIGDVCKSSSLGLHMDGSRFANALVSLGCSPAEMTWKAGVDALSFGATKNGVLAAEAIVLFNTSLATEMSYRRKRAGHLISKYRFLSAQIDAYLTDDLWLRNARKANAAAQRLAQGLEGLGGVEVLGGTEANILFCRLDSAMIDALLKAGFTFGYKRWGPNVVRFVTSFATTAEDVDHLLNQVRLAADRTQER

SEQ ID NO: 149 - DNA, 1128 bp, Artificial sequence
  Engineered sequence
atgaacggtgaaacctcgcgtccgccggcgctgggttttagctctgaaaatattgctggtgcaagcccggaagtcgcacaggcactcgttaagcacagttcgggccaggcgggtccctatggcaccgacgagttgacggcacaggtcaagcatagctccggccaagctgacccttatggtaccgatgaactgactgctcaagttaaacgtaaattttgcgaaatcttcgaacgcgacgtcgaagtgttcctggttccgaccggtacggcagcaaacgcactgtgtctgtccgcaatgaccccgccgtggggtaatatttactgccatcacgcgtcccacatcaacaatgatgaatgtggtgcgccggaatttttctcaaacggcgccaaactgatgaccgttgatggtccggcagctaaactggacattgtccgtctgcgcgaacgtacgagagaaaaagtgggtgatgttcattcgacgcagccggcatgcgtctctattacccaagctacggaagtgggcagtatctataccctggatgaaattgaagccatcggtgacgtgtgcaaatcatcgagcctgggtctgcacatggatggctctcgttttgctaatgcgctggtgtccctgggctgttcaccggcagaaatgacctggaaagccggtgttgacgcactgagttttggtgcgacgaaaaacggcgttctggcggccgaagcaattgtcctgttcaatacctcgctggctacggaaatgagctatcgtcgcaaacgtgccggccacctgatcagtaaataccgctttctgagcgctcagatcgatgcgtacctgaccgatgacctgtggctgcgtaacgcccgcaaagcaaatgcagctgcgcagcgtctggcccaaggtctggaaggcctgggcggtgttgaagtcctgggcggtaccgaagcaaacattctgttctgtcgcctggattctgccatgatcgacgcactgctgaaagctggctttaaattcgggtacaagcgttggggtccgaacgtggttcgctttgttaccagcttcgctaccacggcggaagatgtggaccacctgctgaatcaggttcgcctggccgcagaccgtacgcaagaacgc

SEQ ID NO: 150 - protein, 376 aa, Artificial sequence
  Engineered sequence
MNGETSRPPALGFSSENIAGASPEVAQALVKHSSGQAGPYGTDELTAQVKHSSGQADPYGTDELTAQVKRKFCEIFERDVEVFLVPTGTAANALCLSAMTPPWGNIYCHHASHINNDECGAPEFFSNGAKLMTVDGPAAKLDIVRLRERTREKVGDVHSTQPACVSITQATEVGSIYTLDEIEAIGDVCKSSSLGLHMDGSRFANALVSLGCSPAEMTWKAGVDALSFGATKNGVLAAEAIVLFNTSLATEMSYRRKRAGHLISKYRFLSAQIDAYLTDDLWLRNARKANAAAQRLAQGLEGLGGVEVLGGTEANILFCRLDSAMIDALLKAGFKFGYKRWGPNVVRFVTSFATTAEDVDHLLNQVRLAADRTQER

SEQ ID NO: 151 - DNA, 1128 bp, Artificial sequence
  Engineered sequence
atgaacggtgaaacctcgcgtccgccggcgctgggttttagctctgaaaatattgctggtgcaagcccggaagtcgcacaggcactcgttaagcacagttcgggccaggcgggtccctatggcaccgacgagttgacggcacaggtcaagcatagctccggccaagctgacccttatggtaccgatgaactgactgctcaagttaaacgtaaattttgcgaaatcttcgaacgcgacgtcgaagtgttcctggttccgaccggtacggcagcaaacgcactgtgtctgtccgcaatgaccccgccgtggggtaatatttactgccatcacgcgtcccacatcaacaatgatgaatgtggtgcgccggaatttttctcaaacggcgccaaactgatgaccgttgatggtccggcagctaaactggacattgtccgtctgcgcgaacgtacgagagaaaaagtgggtgatgttcattcgacgcagccggcatgcgtctctattacccaagctacggaagtgggcagtatctataccctggatgaaattgaagccatcggtgacgtgtgcaaatcatcgagcctgggtctgcacatggatggctctcgttttgctaatgcgctggtgtccctgggctgttcaccggcagaaatgacctggaaagccggtgttgacgcactgagttttggtgcgacgaaaaacggcgttctggcggccgaagcaattgtcctgttcaatacctcgctggctacggaaatgagctatcgtcgcaaacgtgccggccacctgatcagtaaataccgctttctgagcgctcagatcgatgcgtacctgaccgatgacctgtggctgcgtaacgcccgcaaagcaaatgcagctgcgcagcgtctggcccaaggtctggaaggcctgggcggtgttgaagtcctgggcggtaccgaagcaaacattctgttctgtcgcctggattctgccatgatcgacgcactgctgaaagctggctttaaattcgggtacgagcgttggggtccgaacgtggttcgctttgttaccagcttcgctaccacggcggaagatgtggaccacctgctgaatcaggttcgcctggccgcagaccgtacgcaagaacgc

SEQ ID NO: 152 - protein, 376 aa, Artificial sequence
  Engineered sequence
MNGETSRPPALGFSSENIAGASPEVAQALVKHSSGQAGPYGTDELTAQVKHSSGQADPYGTDELTAQVKRKFCEIFERDVEVFLVPTGTAANALCLSAMTPPWGNIYCHHASHINNDECGAPEFFSNGAKLMTVDGPAAKLDIVRLRERTREKVGDVHSTQPACVSITQATEVGSIYTLDEIEAIGDVCKSSSLGLHMDGSRFANALVSLGCSPAEMTWKAGVDALSFGATKNGVLAAEAIVLFNTSLATEMSYRRKRAGHLISKYRFLSAQIDAYLTDDLWLRNARKANAAAQRLAQGLEGLGGVEVLGGTEANILFCRLDSAMIDALLKAGFKFGYERWGPNVVRFVTSFATTAEDVDHLLNQVRLAADRTQER

SEQ ID NO: 153 - DNA, 1128 bp, Artificial sequence
  Engineered sequence
atgaacggtgaaacctcgcgtccgccggcgctgggttttagctctgaaaatattgctggtgcaagcccggaagtcgcacaggcactcgttaagcacagttcgggccaggcgggtccctatggcaccgacgagttgacggcacaggtcaagcatagctccggccaagctgacccttatggtaccgatgaactgactgctcaagttaaacgtaaattttgcgaaatcttcgaacgcgacgtcgaagtgttcctggttccgaccggtacggcagcaaacgcactgtgtctgtccgcaatgaccccgccgtggggtaatatttactgccatcacgcgtcccacatcaacaatgatgaatgtggtgcgccggaatttttctcaaacggcgccaaactgatgaccgttgatggtccggcagctaaactggacattgtccgtctgcgcgaacgtacgaaggaaaaagtgggtgatgttcattcgacgcagccggcatgcgtctctattacccaagctacggaagtgggcagtatctataccctggatgaaattgaagccatcggtgacgtgtgcaaatcatcgagcctgggtctgcacatggatggctctcgttttgctaatgcgctggtgtccctgggctgttcaccggcagaaatgacctggaaagccggtgttgacgcactgagttttggtgcgacgaaaaacggcgttctggcggccgaagcaattgtcctgttcaatacctcgctggctacggaaatgagctatcgtcgcaaacgtgccggccacctgatcagtaaataccgctttctgagcgctcagatcgatgcgtacctgaccgatgacctgtggctgcgtaacgcccgcaaagcaaatgcagctgcgcagcgtctggcccaaggtctggaaggcctgggcggtgttgaagtcctgggcggtaccgaagcaaacattctgttctgtcgcctggattctgccatgatcgacgcactgctgaaagctggctttaaattcgggtacaagcgttggggtccgaacgtggttcgctttgttaccagcttcgctaccacggcggaagatgtggaccacctgctgaatcaggttcgcctggccgcagaccgtacgcaagaacgc

SEQ ID NO: 154 - protein, 376 aa, Artificial sequence
  Engineered sequence
MNGETSRPPALGFSSENIAGASPEVAQALVKHSSGQAGPYGTDELTAQVKHSSGQADPYGTDELTAQVKRKFCEIFERDVEVFLVPTGTAANALCLSAMTPPWGNIYCHHASHINNDECGAPEFFSNGAKLMTVDGPAAKLDIVRLRERTKEKVGDVHSTQPACVSITQATEVGSIYTLDEIEAIGDVCKSSSLGLHMDGSRFANALVSLGCSPAEMTWKAGVDALSFGATKNGVLAAEAIVLFNTSLATEMSYRRKRAGHLISKYRFLSAQIDAYLTDDLWLRNARKANAAAQRLAQGLEGLGGVEVLGGTEANILFCRLDSAMIDALLKAGFKFGYKRWGPNVVRFVTSFATTAEDVDHLLNQVRLAADRTQER

SEQ ID NO: 155 - DNA, 1128 bp, Artificial sequence
  Engineered sequence
atgaacggtgaaacctcgcgtccgccggcgctgggttttagctctgaaaatattgctggtgcaagcccggaagtcgcacaggcactcgttaagcacagttcgggccaggcgggtccctatggcaccgacgagttgacggcacaggtcaagcatagctccggccaagctgacccttatggtaccgatgaactgactgctcaagttaaacgtaaattttgcgaaatcttcgaacgcgacgtcgaagtgttcctggttccaaccggtacggcagcaaacgcactgtgtctgtccgcaatgaccccgccgtggggtaatatttactgccatcacgcgtcccacatcaacaatgatgaatgtggtgcgccggaatttttctcaaacggcgccaaactgatgaccgttgatggtccggcagctaaactggacattgtccgtctgcgcgaacgtacgcgcgaaaaagtgggtgatgttcatacgacgcagccggcatgcgtctctattacccaagctacggaagtgggcagtatctataccctggatgaaattgaagccatcggtgacgtgtgcaaatcatcgagcctgggtctgcacatggatggcgcccgttttgctaatgcgctggtgtccctgggctgttcaccggcagaaatgacctggaaagccggtgttgacgcactgagttttggtgcgacgaaaaacggcgttctggcggccgaagcaattgtcctgttcaatacctcgctggctacggaaatgagctatcgtcgcaaacgtgccggccacctgatcagtaaataccgctttctgagcgctcagatcgatgcgtacctgaccgatgacctgtggctgcgtaacgcccgcaaagcaaatgcagctgcgcagcgtctggcccaaggtctggaaggcctgggcggtgttgaagtcctgggcggtaccgaagcaaacattctgttctgtcgcctggattctgccatgatcgacgcactgctgaaagctggctttaaattcgggtacaagcgttggggtccgaacgtggttcgctttgttaccagcttcgctaccacggcggaagatgtggaccacctgctgaatcaggttcgcctggccgcagaccgtacgcaagaacgc

SEQ ID NO: 156 - protein, 376 aa, Artificial sequence
  Engineered sequence
MNGETSRPPALGFSSENIAGASPEVAQALVKHSSGQAGPYGTDELTAQVKHSSGQADPYGTDELTAQVKRKFCEIFERDVEVFLVPTGTAANALCLSAMTPPWGNIYCHHASHINNDECGAPEFFSNGAKLMTVDGPAAKLDIVRLRERTREKVGDVHTTQPACVSITQATEVGSIYTLDEIEAIGDVCKSSSLGLHMDGARFANALVSLGCSPAEMTWKAGVDALSFGATKNGVLAAEAIVLFNTSLATEMSYRRKRAGHLISKYRFLSAQIDAYLTDDLWLRNARKANAAAQRLAQGLEGLGGVEVLGGTEANILFCRLDSAMIDALLKAGFKFGYKRWGPNVVRFVTSFATTAEDVDHLLNQVRLAADRTQER

SEQ ID NO: 157 - DNA, 1128 bp, Artificial sequence
  Engineered sequence
atgaacggtgaaacctcgcgtccgccggcgctgggttttagctctgaaaatattgctggtgcaagcccggaagtcgcacaggcactcgttaagcacagttcgggccaggcgggtccctatggcaccgacgagttgacggcacaggtcaagcatagctccggccaagctgacccttatggtaccgatgaactgactgctcaagttaaacgtaaattttgcgaaatcttcgaacgcgacgtcgaagtgttcctggttccaaccggtacggcagcaaacgcactgtgtctgtccgcaatgaccccgccgtggggtaatatttactgccatcacgcgtcccacatcaacaatgatgaatgtggtgcgccggaatttttctcaaacggcgccaaactgatgaccgttgatggtccggcagctaaactggacattgtccgtctgcgcgaacgtacgcgcgaaaaagtgggtgatgttcatacgacgcagccggcatgcgtctctattacccaagctacggaagtgggcagtatctataccctggatgaaattgaagccatcggtgacgtgtgcaaatcatcgagcctgggtctgcacatggatggcgcccgttttgctaatgcgctggtgtccctgggctgttcaccggcagaaatgacctggaaagccggtgttgacgcactgagttttggtgcgacgaaaaacggcgttctggcggccgaagcaattgtcctgttcaatacctcgctggctacggaaatgagctatcgtcgcaaacgtgccggccacctgatcagtaaataccgctttctgagcgctcagatcgatgcgtacctgaccgatgacctgtggctgcgtaacgcccgcaaagcaaatgcagctgcgcagcgtctggcccaaggtctggaaggcctgggcggtgttgaagtcctgggcggtaccgaagcaaacattctgttctgtcgcctggattctgccatgatcgacgcactgctgaaagctggctttaaattcgggtacgagcgttggggtccgaacgtggttcgctttgttaccagcttcgctaccacggcggaagatgtggaccacctgctgaatcaggttcgcctggccgcagaccgtacgcaagaacgc

SEQ ID NO: 158 - protein, 376 aa, Artificial sequence
  Engineered sequence
MNGETSRPPALGFSSENIAGASPEVAQALVKHSSGQAGPYGTDELTAQVKHSSGQADPYGTDELTAQVKRKFCEIFERDVEVFLVPTGTAANALCLSAMTPPWGNIYCHHASHINNDECGAPEFFSNGAKLMTVDGPAAKLDIVRLRERTREKVGDVHTTQPACVSITQATEVGSIYTLDEIEAIGDVCKSSSLGLHMDGARFANALVSLGCSPAEMTWKAGVDALSFGATKNGVLAAEAIVLFNTSLATEMSYRRKRAGHLISKYRFLSAQIDAYLTDDLWLRNARKANAAAQRLAQGLEGLGGVEVLGGTEANILFCRLDSAMIDALLKAGFKFGYERWGPNVVRFVTSFATTAEDVDHLLNQVRLAADRTQER

SEQ ID NO: 159 - DNA, 1128 bp, Artificial sequence
  Engineered sequence
atgaacggtgaaacctcgcgtccgccggcgctgggttttagctctgaaaatattgctggtgcaagcccggaagtcgcacaggcactcgttaagcacagttcgggccaggcgggtccctatggcaccgacgagttgacggcacaggtcaagcatagctccggccaagctgacccttatggtttcgatgaactgactgctcaagttaaacgtaaattttgcgaaatcttcgaacgcgacgtcgaagtgttcctggttgccaccggtacggcagcaaacgcactgtgtctgtccgcaatgaccccgccgtggggtaatatttactgccatcacgcgtcccacatcaacaatgatgaatgtggtgcgccggaatttttctcaaacggcgccaaactgatgaccgttgatggtccggcagctaaactggacattgtccgtctgcgcgaacgtacgcgcgaaaaagtgggtgatgttcatacgacgcagccggcatgcgtctctattacccaagctacggaagtgggcagtatctataccctggatgaaattgaagccatcggtgacgtgtgcaaatcatcgagcctgggtctgcacatggatggcgcccgttttgctaatgcgctggtgtccctgggctgttcaccggcagaaatgacctggaaagccggtgttgacgcactgagttttggtgcgacgaaaaacggcgttctggcggccgaagcaattgtcctgttcaatacctcgctggctacggaaatgagctatcgtcgcaaacgtgccggccacctgatcagtaaataccgctttctgagcgctcagatcgatgcgtacctgaccgatgacctgtggctgcgtaacgcccgcaaagcaaatgcagctgcgcagcgtctggcccaaggtctggaaggcctgggcggtgttgaagtcctgggcggtaccgaagcaaacattctgttctgtcgcctggattctgccatgatcgacgcactgctgaaagctggctttggcttcgggtacaagcgttggggtccgaacgtggttcgctttgttaccagcttcgctaccacggcggaagatgtggaccacctgctgaatcaggttcgcctggccgcagaccgtacgcaagaacgc

SEQ ID NO: 160 - protein, 376 aa, Artificial sequence
  Engineered sequence
MNGETSRPPALGFSSENIAGASPEVAQALVKHSSGQAGPYGTDELTAQVKHSSGQADPYGFDELTAQVKRKFCEIFERDVEVFLVATGTAANALCLSAMTPPWGNIYCHHASHINNDECGAPEFFSNGAKLMTVDGPAAKLDIVRLRERTREKVGDVHTTQPACVSITQATEVGSIYTLDEIEAIGDVCKSSSLGLHMDGARFANALVSLGCSPAEMTWKAGVDALSFGATKNGVLAAEAIVLFNTSLATEMSYRRKRAGHLISKYRFLSAQIDAYLTDDLWLRNARKANAAAQRLAQGLEGLGGVEVLGGTEANILFCRLDSAMIDALLKAGFGFGYKRWGPNVVRFVTSFATTAEDVDHLLNQVRLAADRTQER

SEQ ID NO: 161 - DNA, 1128 bp, Artificial sequence
  Engineered sequence
atgaacggtgaaacctcgcgtccgccggcgctgggttttagctctgaaaatattgctggtgcaagcccggaagtcgcacaggcactcgttaagcacagttcgggccaggcgggtccctatggcaccgacgagttgacggcacaggtcaagcatagctccggccaagctgacccttatggtaccgatgaactgactgctcaagttaaacgtaaattttgcgaaatcttcgaacgcgacgtcgaagtgttcctggttccaaccggtacggcagcaaacgcactgtgtctgtccgcaatgaccccgccgtggggtaatatttactgccatcacgcgtcccacatcaacaatgatgaatgtggtgcgccggaatttttctcaaacggcgccaaactgatgaccgttgatggtccggcagctaaactggacattgtccgtctgcgcgaacgtacgcgcgaaaaagtgggtgatgttcatacgacgcagccggcatgcgtctctattacccaagctacggaagtgggcagtatctataccctggatgaaattgaagccatcggtgacgtgtgcaaatcatcgagcctgggtctgcacatggatggcgcccgttttgctaatgcgctggtgtccctgggctgttcaccggcagaaatgacctggaaagccggtgttgacgcactgagttttggtgcgacgaaaaacggcgttctggcggccgaagcaattgtcctgttcaatacctcgctggctacggaaatgagctatcgtcgcaaacgtgccggccacctgatcagtaaataccgctttctgagcgctcagatcgatgcgtacctgaccgatgacctgtggctgcgtaacgcccgcaaagcaaatgcagctgcgcagcgtctggcccaaggtctggaaggcctgggcggtgttgaagtcctgggcggtaccgaagcaaacattctgttctgtcgcctggattctgccatgatcgacgcactgctgaaagctggctttggcttcgggtacaagcgttggggtccgaacgtggttcgctttgttaccagcttcgctaccacggcggaagatgtggaccacctgctgaatcaggttcgcctggccgcagaccgtacgcaagaacgc

SEQ ID NO: 162 - protein, 376 aa, Artificial sequence
  Engineered sequence
MNGETSRPPALGFSSENIAGASPEVAQALVKHSSGQAGPYGTDELTAQVKHSSGQADPYGTDELTAQVKRKFCEIFERDVEVFLVPTGTAANALCLSAMTPPWGNIYCHHASHINNDECGAPEFFSNGAKLMTVDGPAAKLDIVRLRERTREKVGDVHTTQPACVSITQATEVGSIYTLDEIEAIGDVCKSSSLGLHMDGARFANALVSLGCSPAEMTWKAGVDALSFGATKNGVLAAEAIVLFNTSLATEMSYRRKRAGHLISKYRFLSAQIDAYLTDDLWLRNARKANAAAQRLAQGLEGLGGVEVLGGTEANILFCRLDSAMIDALLKAGFGFGYKRWGPNVVRFVTSFATTAEDVDHLLNQVRLAADRTQER

SEQ ID NO: 163 - DNA, 1128 bp, Artificial sequence
  Engineered sequence
atgaacggtgaaacctcgcgtccgccggcgctgggttttagctctgaaaatattgctggtgcaagcccggaagtcgcacaggcactcgttaagcacagttcgggccaggcgggtccctatggcaccgacgagttgacggcacaggtcaagcatagctccggccaagctgacccttatggtaccgatgaactgactgctcaagttaaacgtaaattttgcgaaatcttcgaacgcgacgtcgaagtgttcctggttccaaccggtacggcagcaaacgcactgtgtctgtccgcaatgaccccgccgtggggtaatatttactgccatcacgcgtcccacatcaacaatgatgaatgtggtgcgccggaatttttctcaaacggcgccaaactgatgaccgttgatggtccggcagctaaactggacattgtccgtctgcgcgaacgtacgcgcgaaaaagtgggtgatgttcattcgacgcagccggcatgcgtctctattacccaagctacggaagtgggcagtatctataccctggatgaaattgaagccatcggtgacgtgtgcaaatcatcgagcctgggtctgcacatggatggcgcccgttttgctaatgcgctggtgtccctgggctgttcaccggcagaaatgacctggaaagccggtgttgacgcactgagttttggtgcgacgaaaaacggcgttctggcggccgaagcaattgtcctgttcaatacctcgctggctacggaaatgagctatcgtcgcaaacgtgccggccacctgatcagtaaataccgctttctgagcgctcagatcgatgcgtacctgaccgatgacctgtggctgcgtaacgcccgcaaagcaaatgcagctgcgcagcgtctggcccaaggtctggaaggcctgggcggtgttgaagtcctgggcggtaccgaagcaaacattctgttctgtcgcctggattctgccatgatcgacgcactgctgaaagctggctttaaattcgggtacaagcgttggggtccgaacgtggttcgctttgttaccagcttcgctaccacggcggaagatgtggaccacctgctgaatcaggttcgcctggccgcagaccgtacgcaagaacgc

SEQ ID NO: 164 - protein, 376 aa, Artificial sequence
  Engineered sequence
MNGETSRPPALGFSSENIAGASPEVAQALVKHSSGQAGPYGTDELTAQVKHSSGQADPYGTDELTAQVKRKFCEIFERDVEVFLVPTGTAANALCLSAMTPPWGNIYCHHASHINNDECGAPEFFSNGAKLMTVDGPAAKLDIVRLRERTREKVGDVHSTQPACVSITQATEVGSIYTLDEIEAIGDVCKSSSLGLHMDGARFANALVSLGCSPAEMTWKAGVDALSFGATKNGVLAAEAIVLFNTSLATEMSYRRKRAGHLISKYRFLSAQIDAYLTDDLWLRNARKANAAAQRLAQGLEGLGGVEVLGGTEANILFCRLDSAMIDALLKAGFKFGYKRWGPNVVRFVTSFATTAEDVDHLLNQVRLAADRTQER

SEQ ID NO: 165 - DNA, 1128 bp, Artificial sequence
  Engineered sequence
atgaacggtgaaacctcgcgtccgccggcgctgggttttagctctgaaaatattgctggtgcaagcccggaagtcgcacaggcactcgttaagcacagttcgggccaggcgggtccctatggcaccgacgagttgacggcacaggtcaagcatagctccggccaagctgacccttatggtaccgatgaactgactgctcaagttaaacgtaaattttgcgaaatcttcgaacgcgacgtcgaagtgttcctggttgccaccggtacggcagcaaacgcactgtgtctgtccgcaatgaccccgccgtggggtaatatttactgccatcacgcgtcccacatcaacaatgatgaatgtggtgcgccggaatttttctcaaacggcgccaaactgatgaccgttgatggtccggcagctaaactggacattgtccgtctgcgcgaacgtacgcgcgaaaaagtgggtgatgttcatacgacgcagccggcatgcgtctctattacccaagctacggaagtgggcagtatctataccctggatgaaattgaagccatcggtgacgtgtgcaaatcatcgagcctgggtctgcacatggatggcgcccgttttgctaatgcgctggtgtccctgggctgttcaccggcagaaatgacctggaaagccggtgttgacgcactgagttttggtgcgacgaaaaacggcgttctggcggccgaagcaattgtcctgttcaatacctcgctggctacggaaatgagctatcgtcgcaaacgtgccggccacctgatcagtaaataccgctttctgagcgctcagatcgatgcgtacctgaccgatgacctgtggctgcgtaacgcccgcaaagcaaatgcagctgcgcagcgtctggcccaaggtctggaaggcctgggcggtgttgaagtcctgggcggtaccgaagcaaacattctgttctgtcgcctggattctgccatgatcgacgcactgctgaaagctggctttaaattcgggtacgagcgttggggtccgaacgtggttcgctttgttaccagcttcgctaccacggcggaagatgtggaccacctgctgaatcaggttcgcctggccgcagaccgtacgcaagaacgc

SEQ ID NO: 166 - protein, 376 aa, Artificial sequence
  Engineered sequence
MNGETSRPPALGFSSENIAGASPEVAQALVKHSSGQAGPYGTDELTAQVKHSSGQADPYGTDELTAQVKRKFCEIFERDVEVFLVATGTAANALCLSAMTPPWGNIYCHHASHINNDECGAPEFFSNGAKLMTVDGPAAKLDIVRLRERTREKVGDVHTTQPACVSITQATEVGSIYTLDEIEAIGDVCKSSSLGLHMDGARFANALVSLGCSPAEMTWKAGVDALSFGATKNGVLAAEAIVLFNTSLATEMSYRRKRAGHLISKYRFLSAQIDAYLTDDLWLRNARKANAAAQRLAQGLEGLGGVEVLGGTEANILFCRLDSAMIDALLKAGFKFGYERWGPNVVRFVTSFATTAEDVDHLLNQVRLAADRTQER

SEQ ID NO: 167 - DNA, 1128 bp, Artificial sequence
  Engineered sequence
atgaacggtgaaacctcgcgtccgccggcgctgggttttagctctgaaaatattgctggtgcaagcccggaagtcgcacaggcactcgttaagcacagttcgggccaggcgggtccctatggcaccgacgagttgacggcacaggtcaagcatagctccggccaagctgacccttatggtaccgatgaactgactgctcaagttaaacgtaaattttgcgaaatcttcgaacgcgacgtcgaagtgttcctggttgccaccggtacggcagcaaacgcactgtgtctgtccgcaatgaccccgccgtggggtaatatttactgccatcacgcgtcccacatcaacaatgatgaatgtggtgcgccggaatttttctcaaacggcgccaaactgatgaccgttgatggtccggcagctaaactggacattgtccgtctgcgcgaacgtacgcgcgaaaaagtgggtgatgttcattcgacgcagccggcatgcgtctctattacccaagctacggaagtgggcagtatctataccctggatgaaattgaagccatcggtgacgtgtgcaaatcatcgagcctgggtctgcacatggatggcgcccgttttgctaatgcgctggtgtccctgggctgttcaccggcagaaatgacctggaaagccggtgttgacgcactgagttttggtgcgacgaaaaacggcgttctggcggccgaagcaattgtcctgttcaatacctcgctggctacggaaatgagctatcgtcgcaaacgtgccggccacctgatcagtaaataccgctttctgagcgctcagatcgatgcgtacctgaccgatgacctgtggctgcgtaacgcccgcaaagcaaatgcagctgcgcagcgtctggcccaaggtctggaaggcctgggcggtgttgaagtcctgggcggtaccgaagcaaacattctgttctgtcgcctggattctgccatgatcgacgcactgctgaaagctggctttaaattcgggtacaagcgttggggtccgaacgtggttcgctttgttaccagcttcgctaccacggcggaagatgtggaccacctgctgaatcaggttcgcctggccgcagaccgtacgcaagaacgc

SEQ ID NO: 168 - protein, 376 aa, Artificial sequence
  Engineered sequence
MNGETSRPPALGFSSENIAGASPEVAQALVKHSSGQAGPYGTDELTAQVKHSSGQADPYGTDELTAQVKRKFCEIFERDVEVFLVATGTAANALCLSAMTPPWGNIYCHHASHINNDECGAPEFFSNGAKLMTVDGPAAKLDIVRLRERTREKVGDVHSTQPACVSITQATEVGSIYTLDEIEAIGDVCKSSSLGLHMDGARFANALVSLGCSPAEMTWKAGVDALSFGATKNGVLAAEAIVLFNTSLATEMSYRRKRAGHLISKYRFLSAQIDAYLTDDLWLRNARKANAAAQRLAQGLEGLGGVEVLGGTEANILFCRLDSAMIDALLKAGFKFGYKRWGPNVVRFVTSFATTAEDVDHLLNQVRLAADRTQER

SEQ ID NO: 169 - DNA, 1128 bp, Artificial sequence
  Engineered sequence
atgaacggtgaaacctcgcgtccgccggcgctgggttttagctctgaaaatattgctggtgcaagcccggaagtcgcacaggcactcgttaagcacagttcgggccaggcgggtccctatggcaccgacgagttgacggcacaggtcaagcatagctccggccaagctgacccttatggtaccgatgaactgactgctcaagttaaacgtaaattttgcgaaatcttcgaacgcgacgtcgaagtgttcctggttgccaccggtacggcagcaaacgcactgtgtctgtccgcaatgaccccgccgtggggtaatatttactgccatcacgcgtcccacatcaacaatgatgaatgtggtgcgccggaatttttctcaaacggcgccaaactgatgaccgttgatggtccggcagctaaactggacattgtccgtctgcgcgaacgtacgcgcgaaaaagtgggtgatgttcatacgacgcagccggcatgcgtctctattacccaagctacggaagtgggcagtatctataccctggatgaaattgaagccatcggtgacgtgtgcaaatcatcgagcctgggtctgcacatggatggctcacgttttgctaatgcgctggtgtccctgggctgttcaccggcagaaatgacctggaaagccggtgttgacgcactgagttttggtgcgacgaaaaacggcgttctggcggccgaagcaattgtcctgttcaatacctcgctggctacggaaatgagctatcgtcgcaaacgtgccggccacctgatcagtaaataccgctttctgagcgctcagatcgatgcgtacctgaccgatgacctgtggctgcgtaacgcccgcaaagcaaatgcagctgcgcagcgtctggcccaaggtctggaaggcctgggcggtgttgaagtcctgggcggtaccgaagcaaacattctgttctgtcgcctggattctgccatgatcgacgcactgctgaaagctggctttaaattcgggtacgagcgttggggtccgaacgtggttcgctttgttaccagcttcgctaccacggcggaagatgtggaccacctgctgaatcaggttcgcctggccgcagaccgtacgcaagaacgc

SEQ ID NO: 170 - protein, 376 aa, Artificial sequence
  Engineered sequence
MNGETSRPPALGFSSENIAGASPEVAQALVKHSSGQAGPYGTDELTAQVKHSSGQADPYGTDELTAQVKRKFCEIFERDVEVFLVATGTAANALCLSAMTPPWGNIYCHHASHINNDECGAPEFFSNGAKLMTVDGPAAKLDIVRLRERTREKVGDVHTTQPACVSITQATEVGSIYTLDEIEAIGDVCKSSSLGLHMDGSRFANALVSLGCSPAEMTWKAGVDALSFGATKNGVLAAEAIVLFNTSLATEMSYRRKRAGHLISKYRFLSAQIDAYLTDDLWLRNARKANAAAQRLAQGLEGLGGVEVLGGTEANILFCRLDSAMIDALLKAGFKFGYERWGPNVVRFVTSFATTAEDVDHLLNQVRLAADRTQER

SEQ ID NO: 171 - DNA, 1128 bp, Artificial sequence
  Engineered sequence
atgaacggtgaaacctcgcgtccgccggcgctgggttttagctctgaaaatattgctggtgcaagcccggaagtcgcacaggcactcgttaagcacagttcgggccaggcgggtccctatggcaccgacgagttgacggcacaggtcaagcatagctccggccaagctgacccttatggtaccgatgaactgactgctcaagttaaacgtaaattttgcgaaatcttcgaacgcgacgtcgaagtgttcctggttccaaccggtacggcagcaaacgcactgtgtctgtccgcaatgaccccgccgtggggtaatatttactgccatcacgcgtcccacatcaacaatgatgaatgtggtgcgccggaatttttctcaaacggcgccaaactgatgaccgttgatggtccggcagctaaactggacattgtccgtctgcgcgaacgtacgcgcgaaaaagtgggtgatgttcatacgacgcagccggcatgcgtctctattacccaagctacggaagtgggcagtatctataccctggatgaaattgaagccatcggtgacgtgtgcaaatcatcgagcctgggtctgcacatggatggcgcccgttttgctaatgcgctggtgtccctgggctgttcaccggcagaaatgacctggaaagccggtgttgacgcactgagttttggtgcgacgaaaaacggcgttctggcggccgaagcaattgtcctgttcaatacctcgctggctacggaaatgagctatcgtcgcaaacgtgccggccacctgatcagtaaataccgctttctgagcgctcagatcgatgcgtacctgaccgatgacctgtggctgcgtaacgcccgcaaagcaaatgcagctgcgcagcgtctggcccaaggtctggaaggcctgggcggtgttgaagtcctgggcggtaccgaagcaaacattctgttctgtcgcctggattctgccatgatcgacgcactgctgaaagctggctttcgcttcgggtacaagcgttggggtccgaacgtggttcgctttgttaccagcttcgctaccacggcggaagatgtggaccacctgctgaatcaggttcgcctggccgcagaccgtacgcaagaacgc

SEQ ID NO: 172 - protein, 376 aa, Artificial sequence
  Engineered sequence
MNGETSRPPALGFSSENIAGASPEVAQALVKHSSGQAGPYGTDELTAQVKHSSGQADPYGTDELTAQVKRKFCEIFERDVEVFLVPTGTAANALCLSAMTPPWGNIYCHHASHINNDECGAPEFFSNGAKLMTVDGPAAKLDIVRLRERTREKVGDVHTTQPACVSITQATEVGSIYTLDEIEAIGDVCKSSSLGLHMDGARFANALVSLGCSPAEMTWKAGVDALSFGATKNGVLAAEAIVLFNTSLATEMSYRRKRAGHLISKYRFLSAQIDAYLTDDLWLRNARKANAAAQRLAQGLEGLGGVEVLGGTEANILFCRLDSAMIDALLKAGFRFGYKRWGPNVVRFVTSFATTAEDVDHLLNQVRLAADRTQER

SEQ ID NO: 173 - DNA, 1128 bp, Artificial sequence
  Engineered sequence
atgaacggtgaaacctcgcgtccgccggcgctgggttttagctctgaaaatattgctggtgcaagcccggaagtcgcacaggcactcgttaagcacagttcgggccaggcgggtccctatggcaccgacgagttgacggcacaggtcaagcatagctccggccaagctgacccttatggtaccgatgaactgactgctcaagttaaacgtaaattttgcgaaatcttcgaacgcgacgtcgaagtgttcctggttggaaccggtacggcagcaaacgcactgtgtctgtccgcaatgaccccgccgtggggtaatatttactgccatcacgcgtcccacatcaacaatgatgaatgtggtgcgccggaatttttctcaaacggcgccaaactgatgaccgttgatggtccggcagctaaactggacattgtccgtctgcgcgaacgtacgcgcgaaaaagtgggtgatgttcattcgacgcagccggcatgcgtctctattacccaagctacggaagtgggcagtatctataccctggatgaaattgaagccatcggtgacgtgtgcaaatcatcgagcctgggtctgcacatggatggctcacgttttgctaatgcgctggtgtccctgggctgttcaccggcagaaatgacctggaaagccggtgttgacgcactgagttttggtgcgacgaaaaacggcgttctggcggccgaagcaattgtcctgttcaatacctcgctggctacggaaatgagctatcgtcgcaaacgtgccggccacctgatcagtaaataccgctttctgagcgctcagatcgatgcgtacctgaccgatgacctgtggctgcgtaacgcccgcaaagcaaatgcagctgcgcagcgtctggcccaaggtctggaaggcctgggcggtgttgaagtcctgggcggtaccgaagcaaacattctgttctgtcgcctggattctgccatgatcgacgcactgctgaaagctggctttcgcttcgggtacaagcgttggggtccgaacgtggttcgctttgttaccagcttcgctaccacggcggaagatgtggaccacctgctgaatcaggttcgcctggccgcagaccgtacgcaagaacgc

SEQ ID NO: 174 - protein, 376 aa, Artificial sequence
  Engineered sequence
MNGETSRPPALGFSSENIAGASPEVAQALVKHSSGQAGPYGTDELTAQVKHSSGQADPYGTDELTAQVKRKFCEIFERDVEVFLVGTGTAANALCLSAMTPPWGNIYCHHASHINNDECGAPEFFSNGAKLMTVDGPAAKLDIVRLRERTREKVGDVHSTQPACVSITQATEVGSIYTLDEIEAIGDVCKSSSLGLHMDGSRFANALVSLGCSPAEMTWKAGVDALSFGATKNGVLAAEAIVLFNTSLATEMSYRRKRAGHLISKYRFLSAQIDAYLTDDLWLRNARKANAAAQRLAQGLEGLGGVEVLGGTEANILFCRLDSAMIDALLKAGFRFGYKRWGPNVVRFVTSFATTAEDVDHLLNQVRLAADRTQER

SEQ ID NO: 175 - DNA, 1128 bp, Artificial sequence
  Engineered sequence
atgaacggtgaaacctcgcgtccgccggcgctgggttttagctctgaaaatattgctggtgcaagcccggaagtcgcacaggcactcgttaagcacagttcgggccaggcgggtccctatggcaccgacgagttgacggcacaggtcaagcatagctccggccaagctgacccttatggtaccgatgaactgactgctcaagttaaacgtaaattttgcgaaatcttcgaacgcgacgtcgaagtgttcctggttgcaaccggtacggcagcaaacgcactgtgtctgtccgcaatgaccccgccgtggggtaatatttactgccatcacgcgtcccacatcaacaatgatgaatgtggtgcgccggaatttttctcaaacggcgccaaactgatgaccgttgatggtccggcagctaaactggacattgtccgtctgcgcgaacgtacgtccgaaaaagtgggtgatgttcattccacgcagccggcatgcgtctctattacccaagctacggaagtgggcagtatctataccctggatgaaattgaagccatcggtgacgtgtgcaaatcatcgagcctgggtctgcacatggatggcagccgttttgctaatgcgctggtgtccctgggctgttcaccggcagaaatgacctggaaagccggtgttgacgcactgagttttggtgcgacgaaaaacggcgttctggcggccgaagcaattgtcctgttcaatacctcgctggctacggaaatgagctatcgtcacaaacgtgccggccacctgatcagtaaataccgctttctgagcgctcagatcgatgcgtacctgaccgatgacctgtggctgcgtaacgcccgcaaagcaaatgcagctgcgcagcgtctggcccaaggtctggaaggcctgggcggtgttgaagtcctgggcggtaccgaagcaaacattctgttctgtcgcctggattctgccatgatcgacgcactgctgaaagctggctttaaattcgggtacaaacgttggggtccgaacgtggttcgctttgttaccagcttcgctaccacggcggaagatgtggaccacctgctgaatcaggttcgcctggccgcagaccgtacgcaagaacgc

SEQ ID NO: 176 - protein, 376 aa, Artificial sequence
  Engineered sequence
MNGETSRPPALGFSSENIAGASPEVAQALVKHSSGQAGPYGTDELTAQVKHSSGQADPYGTDELTAQVKRKFCEIFERDVEVFLVATGTAANALCLSAMTPPWGNIYCHHASHINNDECGAPEFFSNGAKLMTVDGPAAKLDIVRLRERTSEKVGDVHSTQPACVSITQATEVGSIYTLDEIEAIGDVCKSSSLGLHMDGSRFANALVSLGCSPAEMTWKAGVDALSFGATKNGVLAAEAIVLFNTSLATEMSYRHKRAGHLISKYRFLSAQIDAYLTDDLWLRNARKANAAAQRLAQGLEGLGGVEVLGGTEANILFCRLDSAMIDALLKAGFKFGYKRWGPNVVRFVTSFATTAEDVDHLLNQVRLAADRTQER

SEQ ID NO: 177 - DNA, 1128 bp, Artificial sequence
  Engineered sequence
atgaacggtgaaacctcgcgtccgccggcgctgggttttagctctgaaaatattgctggtgcaagcccggaagtcgcacaggcactcgttaagcacagttcgggccaggcgggtccctatggcaccgacgagttgacggcacaggtcaagcatagctccggccaagctgacccttatggtaccgatgaactgactgctcaagttaaacgtaaattttgcgaaatcttcgaacgcgacgtcgaagtgttcctggttgcaaccggtacggcagcaaacgcactgtgtctgtccgcaatgaccccgccgtggggtaatatttactgccatcacgcgtcccacatcaacaatgatgaatgtggtgcgccggaatttttctcaaacggcgccaaactgatgaccgttgatggtccggcagctaaactggacattgtccgtctgcgcgaacgtacgtccgaaaaagtgggtgatgttcataccacgcagccggcatgcgtctctattacccaagctacggaagtgggcagtatctataccctggatgaaattgaagccatcggtgacgtgtgcaaatcatcgagcctgggtctgcacatggatggcgcgcgttttgctaatgcgctggtgtccctgggctgttcaccggcagaaatgacctggaaagccggtgttgacgcactgagttttggtgcgacgaaaaacggcgttctggcggccgaagcaattgtcctgttcaatacctcgctggctacggaaatgagctatcgtcgtaaacgtgccggccacctgatcagtaaataccgctttctgagcgctcagatcgatgcgtacctgaccgatgacctgtggctgcgtaacgcccgcaaagcaaatgcagctgcgcagcgtctggcccaaggtctggaaggcctgggcggtgttgaagtcctgggcggtaccgaagcaaacattctgttctgtcgcctggattctgccatgatcgacgcactgctgaaagctggctttaaattcgggtacaaacgttggggtccgaacgtggttcgctttgttaccagcttcgctaccacggcggaagatgtggaccacctgctgaatcaggttcgcctggccgcagaccgtacgcaagaacgc

SEQ ID NO: 178 - protein, 376 aa, Artificial sequence
  Engineered sequence
MNGETSRPPALGFSSENIAGASPEVAQALVKHSSGQAGPYGTDELTAQVKHSSGQADPYGTDELTAQVKRKFCEIFERDVEVFLVATGTAANALCLSAMTPPWGNIYCHHASHINNDECGAPEFFSNGAKLMTVDGPAAKLDIVRLRERTSEKVGDVHTTQPACVSITQATEVGSIYTLDEIEAIGDVCKSSSLGLHMDGARFANALVSLGCSPAEMTWKAGVDALSFGATKNGVLAAEAIVLFNTSLATEMSYRRKRAGHLISKYRFLSAQIDAYLTDDLWLRNARKANAAAQRLAQGLEGLGGVEVLGGTEANILFCRLDSAMIDALLKAGFKFGYKRWGPNVVRFVTSFATTAEDVDHLLNQVRLAADRTQER

SEQ ID NO: 179 - DNA, 1128 bp, Artificial sequence
  Engineered sequence
atgaacggtgaaacctcgcgtccgccggcgctgggttttagctctgaaaatattgctggtgcaagcccggaagtcgcacaggcactcgttaagcacagttcgggccaggcgggtccctatggcaccgacgagttgacggcacaggtcaagcatagctccggccaagctgacccttatggtaccgatgaactgactgctcaagttaaacgtaaattttgcgaaatcttcgaacgcgacgtcgaagtgttcctggttcctaccggtacggcagcaaacgcactgtgtctgtccgcaatgaccccgccgtggggtaatatttactgccatcacgcgtcccacatcaacaatgatgaatgtggtgcgccggaatttttctcaaacggcgccaaactgatgaccgttgatggtccggcagctaaactggacattgtccgtctgcgcgaacgtacgtccgaaaaagtgggtgatgttcataccacgcagccggcatgcgtctctattacccaagctacggaagtgggcagtatctataccctggatgaaattgaagccatcggtgacgtgtgcaaatcatcgagcctgggtctgcacatggatggcgcgcgttttgctaatgcgctggtgtccctgggctgttcaccggcagaaatgacctggaaagccggtgttgacgcactgagttttggtgcgacgaaaaacggcgttctggcggccgaagcaattgtcctgttcaatacctcgctggctacggaaatgagctatcgtcacaaacgtgccggccacctgatcagtaaataccgctttctgagcgctcagatcgatgcgtacctgaccgatgacctgtggctgcgtaacgcccgcaaagcaaatgcagctgcgcagcgtctggcccaaggtctggaaggcctgggcggtgttgaagtcctgggcggtaccgaagcaaacattctgttctgtcgcctggattctgccatgatcgacgcactgctgaaagctggctttaaattcgggtacaaacgttggggtccgaacgtggttcgctttgttaccagcttcgctaccacggcggaagatgtggaccacctgctgaatcaggttcgcctggccgcagaccgtacgcaagaacgc

SEQ ID NO: 180 - protein, 376 aa, Artificial sequence
  Engineered sequence
MNGETSRPPALGFSSENIAGASPEVAQALVKHSSGQAGPYGTDELTAQVKHSSGQADPYGTDELTAQVKRKFCEIFERDVEVFLVPTGTAANALCLSAMTPPWGNIYCHHASHINNDECGAPEFFSNGAKLMTVDGPAAKLDIVRLRERTSEKVGDVHTTQPACVSITQATEVGSIYTLDEIEAIGDVCKSSSLGLHMDGARFANALVSLGCSPAEMTWKAGVDALSFGATKNGVLAAEAIVLFNTSLATEMSYRHKRAGHLISKYRFLSAQIDAYLTDDLWLRNARKANAAAQRLAQGLEGLGGVEVLGGTEANILFCRLDSAMIDALLKAGFKFGYKRWGPNVVRFVTSFATTAEDVDHLLNQVRLAADRTQER

SEQ ID NO: 181 - DNA, 1128 bp, Artificial sequence
  Engineered sequence
atgaacggtgaaacctcgcgtccgccggcgctgggttttagctctgaaaatattgctggtgcaagcccggaagtcgcacaggcactcgttaagcacagttcgggccaggcgggtccctatggcaccgacgagttgacggcacaggtcaagcatagctccggccaagctgacccttatggtaccgatgaactgactgctcaagttaaacgtaaattttgcgaaatcttcgaacgcgacgtcgaagtgttcctggttgcaaccggtacggcagcaaacgcactgtgtctgtccgcaatgaccccgccgtggggtaatatttactgccatcacgcgtcccacatcaacaatgatgaatgtggtgcgccggaatttttctcaaacggcgccaaactgatgaccgttgatggtccggcagctaaactggacattgtccgtctgcgcgaacgtacgtccgaaaaagtgggtgatgttcattccacgcagccggcatgcgtctctattacccaagctacggaagtgggcagtatctataccctggatgaaattgaagccatcggtgacgtgtgcaaatcatcgagcctgggtctgcacatggatggcgcgcgttttgctaatgcgctggtgtccctgggctgttcaccggcagaaatgacctggaaagccggtgttgacgcactgagttttggtgcgacgaaaaacggcgttctggcggccgaagcaattgtcctgttcaatacctcgctggctacggaaatgagctatcgtcacaaacgtgccggccacctgatcagtaaataccgctttctgagcgctcagatcgatgcgtacctgaccgatgacctgtggctgcgtaacgcccgcaaagcaaatgcagctgcgcagcgtctggcccaaggtctggaaggcctgggcggtgttgaagtcctgggcggtaccgaagcaaacattctgttctgtcgcctggattctgccatgatcgacgcactgctgaaagctggctttaaattcgggtacaaacgttggggtccgaacgtggttcgctttgttaccagcttcgctaccacggcggaagatgtggaccacctgctgaatcaggttcgcctggccgcagaccgtacgcaagaacgc

SEQ ID NO: 182 - protein, 376 aa, Artificial sequence
  Engineered sequence
MNGETSRPPALGFSSENIAGASPEVAQALVKHSSGQAGPYGTDELTAQVKHSSGQADPYGTDELTAQVKRKFCEIFERDVEVFLVATGTAANALCLSAMTPPWGNIYCHHASHINNDECGAPEFFSNGAKLMTVDGPAAKLDIVRLRERTSEKVGDVHSTQPACVSITQATEVGSIYTLDEIEAIGDVCKSSSLGLHMDGARFANALVSLGCSPAEMTWKAGVDALSFGATKNGVLAAEAIVLFNTSLATEMSYRHKRAGHLISKYRFLSAQIDAYLTDDLWLRNARKANAAAQRLAQGLEGLGGVEVLGGTEANILFCRLDSAMIDALLKAGFKFGYKRWGPNVVRFVTSFATTAEDVDHLLNQVRLAADRTQER

SEQ ID NO: 183 - DNA, 1128 bp, Artificial sequence
  Engineered sequence
atgaacggtgaaacctcgcgtccgccggcgctgggttttagctctgaaaatattgctggtgcaagcccggaagtcgcacaggcactcgttaagcacagttcgggccaggcgggtccctatggcaccgacgagttgacggcacaggtcaagcatagctccggccaagctgacccttatggtaccgatgaactgactgctcaagttaaacgtaaattttgcgaaatcttcgaacgcgacgtcgaagtgttcctggttcctaccggtacggcagcaaacgcactgtgtctgtccgcaatgaccccgccgtggggtaatatttactgccatcacgcgtcccacatcaacaatgatgaatgtggtgcgccggaatttttctcaaacggcgccaaactgatgaccgttgatggtccggcagctaaactggacattgtccgtctgcgcgaacgtacgtccgaaaaagtgggtgatgttcataccacgcagccggcatgcgtctctattacccaagctacggaagtgggcagtatctataccctggatgaaattgaagccatcggtgacgtgtgcaaatcatcgagcctgggtctgcacatggatggcgcgcgttttgctaatgcgctggtgtccctgggctgttcaccggcagaaatgacctggaaagccggtgttgacgcactgagttttggtgcgacgaaaaacggcgttctggcggccgaagcaattgtcctgttcaatacctcgctggctacggaaatgagctatcgtcgtaaacgtgccggccacctgatcagtaaataccgctttctgagcgctcagatcgatgcgtacctgaccgatgacctgtggctgcgtaacgcccgcaaagcaaatgcagctgcgcagcgtctggcccaaggtctggaaggcctgggcggtgttgaagtcctgggcggtaccgaagcaaacattctgttctgtcgcctggattctgccatgatcgacgcactgctgaaagctggctttaaattcgggtacaaacgttggggtccgaacgtggttcgctttgttaccagcttcgctaccacggcggaagatgtggaccacctgctgaatcaggttcgcctggccgcagaccgtacgcaagaacgc

SEQ ID NO: 184 - protein, 376 aa, Artificial sequence
  Engineered sequence
MNGETSRPPALGFSSENIAGASPEVAQALVKHSSGQAGPYGTDELTAQVKHSSGQADPYGTDELTAQVKRKFCEIFERDVEVFLVPTGTAANALCLSAMTPPWGNIYCHHASHINNDECGAPEFFSNGAKLMTVDGPAAKLDIVRLRERTSEKVGDVHTTQPACVSITQATEVGSIYTLDEIEAIGDVCKSSSLGLHMDGARFANALVSLGCSPAEMTWKAGVDALSFGATKNGVLAAEAIVLFNTSLATEMSYRRKRAGHLISKYRFLSAQIDAYLTDDLWLRNARKANAAAQRLAQGLEGLGGVEVLGGTEANILFCRLDSAMIDALLKAGFKFGYKRWGPNVVRFVTSFATTAEDVDHLLNQVRLAADRTQER

SEQ ID NO: 185 - DNA, 1071 bp, Artificial sequence
  Engineered sequence
atgaacggtgaaacctcgcgtccgccggcgctgggttttagctctgataatattgctggtgcaagcccggaagtcgcacaggcactcgttaagcacagttcgggccaggcgggtccctattttaccgacgagttgacggcacaggtcaagcgtaaattttgcgaaatcttcgaacgcgacgtcgaagtgttcctggttccgaccggtacggcagcaaacgcactgtgtctgtccgcaatgaccccgccgtggggtaatatttactgccatccggcgtcccacatcaacaatgatgaatgtggtgcgccggaatttttctcaaacggcgccaaactgatgaccgttgatggtccggcagctaaactggacattgtccgtctgcgcgaacgtacgcgcgaaaaagtgggtgatgttcataccacgcagccggcatgcgtctctattacccaagctacggaagtgggcagtatctataccctggatgaaattgaagccatcggtgacgtgtgcaaatcatcgagcctgggtctgcacatggatggctctcgttttgctaatgcgctggtgtccctgggctgttcaccggcagaaatgacctggaaagccggtgttgacgcactgagttttggtgcgacgaaaaacggcgttctggcggccgaagcaattgtcctgttcaatacctcgctggctacggaaatgagctatcgtcgcaaacgtgccggccacctgtctagtaaaatgcgctttctgagcgctcagatcgatgcgtacctgaccgatgacctgtggctgcgtaacgcccgcaaagcaaatgcagctgcgcagcgtctggcccaaggtctggaaggcctgggcggtgttgaagtcctgggcggtaccgaagcaaacattctgttctgtcgcctggattctgccatgatcgacgcactgctgaaagctggctttggtttctatcatgatcgttggggtccgaacgtggttcgctttgttaccagcttcgctaccacggcggaagatgtggaccacctgctgaatcaggttcgcctggccgcagaccgtacgcaagaacgc

SEQ ID NO: 186 - protein, 357 aa, Artificial sequence
  Engineered sequence
MNGETSRPPALGFSSDNIAGASPEVAQALVKHSSGQAGPYFTDELTAQVKRKFCEIFERDVEVFLVPTGTAANALCLSAMTPPWGNIYCHPASHINNDECGAPEFFSNGAKLMTVDGPAAKLDIVRLRERTREKVGDVHTTQPACVSITQATEVGSIYTLDEIEAIGDVCKSSSLGLHMDGSRFANALVSLGCSPAEMTWKAGVDALSFGATKNGVLAAEAIVLFNTSLATEMSYRRKRAGHLSSKMRFLSAQIDAYLTDDLWLRNARKANAAAQRLAQGLEGLGGVEVLGGTEANILFCRLDSAMIDALLKAGFGFYHDRWGPNVVRFVTSFATTAEDVDHLLNQVRLAADRTQER

SEQ ID NO: 187 - DNA, 1071 bp, Artificial sequence
  Engineered sequence
atgaacggtgaaacctcgcgtccgccggcgctgggttttagctctgataatattgctggtgcaagcccggaagtcgcacaggcactcgttaagcacagttcgggccaggcgggtccctatcagaccgacgagttgacggcacaggtcaagcgtaaattttgcgaaatcttcgaacgcgacgtcgaagtgttcctggttccgaccggtacggcagcaaacgcactgtgtctgtccgcaatgaccccgccgtggggtaatatttactgccatccggcgtcccacatcaacaatgatgaatgtggtgcgccggaatttttctcaaacggcgccaaactgatgaccgttgatggtccggcagctaaactggacattgtccgtctgcgcgaacgtacgcgcgaaaaagtgggtgatgttcataccacgcagccggcatgcgtctctattacccaagctacggaagtgggcagtatctataccctggatgaaattgaagccatcggtgacgtgtgcaaatcatcgagcctgggtctgcacatggatggctctcgttttgctaatgcgctggtgtccctgggctgttcaccggcagaaatgacctggaaagccggtgttgacgcactgagttttggtgcgacgaaaaacggcgttctggcggccgaagcaattgtcctgttcaatacctcgctggctacggaaatgagctatcgtcgcaaacgtgccggccacctgtctagtaaaatgcgctttctgagcgctcagatcgatgcgtacctgaccgatgacctgtggctgcgtaacgcccgcaaagcaaatgcagctgcgcagcgtctggcccaaggtctggaaggcctgggcggtgttgaagtcctgggcggtaccgaagcaaacattctgttctgtcgcctggattctgccatgatcgacgcactgctgaaagctggctttggtttctatcatgatcgttggggtccgaacgtggttcgctttgttaccagcttcgctaccacggcggaagatgtggaccacctgctgaatcaggttcgcctggccgcagaccgtacgcaagaacgc

SEQ ID NO: 188 - protein, 357 aa, Artificial sequence
  Engineered sequence
MNGETSRPPALGFSSDNIAGASPEVAQALVKHSSGQAGPYQTDELTAQVKRKFCEIFERDVEVFLVPTGTAANALCLSAMTPPWGNIYCHPASHINNDECGAPEFFSNGAKLMTVDGPAAKLDIVRLRERTREKVGDVHTTQPACVSITQATEVGSIYTLDEIEAIGDVCKSSSLGLHMDGSRFANALVSLGCSPAEMTWKAGVDALSFGATKNGVLAAEAIVLFNTSLATEMSYRRKRAGHLSSKMRFLSAQIDAYLTDDLWLRNARKANAAAQRLAQGLEGLGGVEVLGGTEANILFCRLDSAMIDALLKAGFGFYHDRWGPNVVRFVTSFATTAEDVDHLLNQVRLAADRTQER

SEQ ID NO: 189 - DNA, 1071 bp, Artificial sequence
  Engineered sequence
atgaacggtgaaacctcgcgtccgccggcgctgggttttagctctgataatattgctggtgcaagcccggaagtcgcacaggcactcgttaagcacagttcgggccaggcgggtccctatcataccgacgagttgacggcacaggtcaagcgtaaattttgcgaaatcttcgaacgcgacgtcgaagtgttcctggttccgaccggtacggcagcaaacgcactgtgtctgtccgcaatgaccccgccgtggggtaatatttactgccatccggcgtcccacatcaacaatgatgaatgtggtgcgccggaatttttctcaaacggcgccaaactgatgaccgttgatggtccggcagctaaactggacattgtccgtctgcgcgaacgtacgcgcgaaaaagtgggtgatgttcataccacgcagccggcatgcgtctctattacccaagctacggaagtgggcagtatctataccctggatgaaattgaagccatcggtgacgtgtgcaaatcatcgagcctgggtctgcacatggatggctctcgttttgctaatgcgctggtgtccctgggctgttcaccggcagaaatgacctggaaagccggtgttgacgcactgagttttggtgcgacgaaaaacggcgttctggcggccgaagcaattgtcctgttcaatacctcgctggctacggaaatgagctatcgtcgcaaacgtgccggccacctgtctagtaaaatgcgctttctgagcgctcagatcgatgcgtacctgaccgatgacctgtggctgcgtaacgcccgcaaagcaaatgcagctgcgcagcgtctggcccaaggtctggaaggcctgggcggtgttgaagtcctgggcggtaccgaagcaaacattctgttctgtcgcctggattctgccatgatcgacgcactgctgaaagctggctttggtttctatcatgatcgttggggtccgaacgtggttcgctttgttaccagcttcgctaccacggcggaagatgtggaccacctgctgaatcaggttcgcctggccgcagaccgtacgcaagaacgc

SEQ ID NO: 190 - protein, 357 aa, Artificial sequence
  Engineered sequence
MNGETSRPPALGFSSDNIAGASPEVAQALVKHSSGQAGPYHTDELTAQVKRKFCEIFERDVEVFLVPTGTAANALCLSAMTPPWGNIYCHPASHINNDECGAPEFFSNGAKLMTVDGPAAKLDIVRLRERTREKVGDVHTTQPACVSITQATEVGSIYTLDEIEAIGDVCKSSSLGLHMDGSRFANALVSLGCSPAEMTWKAGVDALSFGATKNGVLAAEAIVLFNTSLATEMSYRRKRAGHLSSKMRFLSAQIDAYLTDDLWLRNARKANAAAQRLAQGLEGLGGVEVLGGTEANILFCRLDSAMIDALLKAGFGFYHDRWGPNVVRFVTSFATTAEDVDHLLNQVRLAADRTQER

SEQ ID NO: 191 - DNA, 1071 bp, Artificial sequence
  Engineered sequence
atgaacggtgaaacctcgcgtccgccggcgctgggttttagctctgataatattgctggtgcaagcccggaagtcgcacaggcactcgttaagcacagttcgggccaggcgggtccttatggtaccgatgacctgactgctcaagttaaacgtaaattttgcgaaatcttcgaacgcgacgtcgaagtgttcctggttccgaccggtacggcagcaaacgcactgtgtctgtccgcaatgaccccgccgtggggtaatatttactgccatccggcgtcccacatcaacaatgatgaatgtggtgcgccggaatttttctcaaacggcgccaaactgatgaccgttgatggtccggcagctaaactggacattgtccgtctgcgcgaacgtacgcgcgaaaaagtgggtgatgttcataccacgcagccggcatgcgtctctattacccaagctacggaagtgggcagtatctataccctggatgaaattgaagccatcggtgacgtgtgcaaatcatcgagcctgggtctgcacatggatggctctcgttttgctaatgcgctggtgtccctgggctgttcaccggcagaaatgacctggaaagccggtgttgacgcactgagttttggtgcgacgaaaaacggcgttctggcggccgaagcaattgtcctgttcaatacctcgctggctacggaaatgagctatcgtcgcaaacgtgccggccacctgacgagtaaataccgctttctgagcgctcagatcgatgcgtacctgaccgatgacctgtggctgcgtaacgcccgcaaagcaaatgcagctgcgcagcgtctggcccaaggtctggaaggcctgggcggtgttgaagtcctgggcggtaccgaagcaaacattctgttctgtcgcctggattctgccatgatcgacgcactgctgaaagctggctttggtttcgggacgaagcgttggggtccgaacgtggttcgctttgttaccagcttcgctaccacggcggaagatgtggaccacctgctgaatcaggttcgcctggccgcagaccgtacgcaagaacgc

SEQ ID NO: 192 - protein, 357 aa, Artificial sequence
  Engineered sequence
MNGETSRPPALGFSSDNIAGASPEVAQALVKHSSGQAGPYGTDDLTAQVKRKFCEIFERDVEVFLVPTGTAANALCLSAMTPPWGNIYCHPASHINNDECGAPEFFSNGAKLMTVDGPAAKLDIVRLRERTREKVGDVHTTQPACVSITQATEVGSIYTLDEIEAIGDVCKSSSLGLHMDGSRFANALVSLGCSPAEMTWKAGVDALSFGATKNGVLAAEAIVLFNTSLATEMSYRRKRAGHLTSKYRFLSAQIDAYLTDDLWLRNARKANAAAQRLAQGLEGLGGVEVLGGTEANILFCRLDSAMIDALLKAGFGFGTKRWGPNVVRFVTSFATTAEDVDHLLNQVRLAADRTQER

SEQ ID NO: 193 - DNA, 1071 bp, Artificial sequence
  Engineered sequence
atgaacggtgaaacctcgcgtccgccggcgctgggttttagctctgataatattgctggtgcaagcccggaagtcgcacaggcactcgttaagcacagttcgggccaggcgggtccctatggtaccgatgaattcactgctcaagttaaacgtaaattttgcgaaatcttcgaacgcgacgtcgaagtgttcctggttccgaccggtacggcagcaaacgcactgtgtctgtccgcaatgaccccgccgtggggtaatatttactgccatccggcgtcccacatcaacaatgatgaatgtggtgcgccggaatttttctcaaacggcgccaaactgatgaccgttgatggtccggcagctaaactggacattgtccgtctgcgcgaacgtacgcgcgaaaaagtgggtgatgttcataccacgcagccggcatgcgtctctattacccaagctacggaagtgggcagtatctataccctggatgaaattgaagccatcggtgacgtgtgcaaatcatcgagcctgggtctgcacatggatggctctcgttttgctaatgcgctggtgtccctgggctgttcaccggcagaaatgacctggaaagccggtgttgacgcactgagttttggtgcgacgaaaaacggcgttctggcggccgaagcaattgtcctgttcaatacctcgctggctacggaaatgagctatcgtcgcaaacgtgccggccacctgacgagtaaataccgctttctgagcgctcagatcgatgcgtacctgaccgatgacctgtggctgcgtaacgcccgcaaagcaaatgcagctgcgcagcgtctggcccaaggtctggaaggcctgggcggtgttgaagtcctgggcggtaccgaagcaaacattctgttctgtcgcctggattctgccatgatcgacgcactgctgaaagctggctttggtttcgggacgaagcgttggggtccgaacgtggttcgctttgttaccagcttcgctaccacggcggaagatgtggaccacctgctgaatcaggttcgcctggccgcagaccgtacgcaagaacgc

SEQ ID NO: 194 - protein, 357 aa, Artificial sequence
  Engineered sequence
MNGETSRPPALGFSSDNIAGASPEVAQALVKHSSGQAGPYGTDEFTAQVKRKFCEIFERDVEVFLVPTGTAANALCLSAMTPPWGNIYCHPASHINNDECGAPEFFSNGAKLMTVDGPAAKLDIVRLRERTREKVGDVHTTQPACVSITQATEVGSIYTLDEIEAIGDVCKSSSLGLHMDGSRFANALVSLGCSPAEMTWKAGVDALSFGATKNGVLAAEAIVLFNTSLATEMSYRRKRAGHLTSKYRFLSAQIDAYLTDDLWLRNARKANAAAQRLAQGLEGLGGVEVLGGTEANILFCRLDSAMIDALLKAGFGFGTKRWGPNVVRFVTSFATTAEDVDHLLNQVRLAADRTQER

SEQ ID NO: 195 - DNA, 1095 bp, Artificial sequence
  Engineered sequence
atgaatggtgaaaccagtcgtccgccggcactgggttttagcagcgaaaacattgcaggcgcaagtccggaagttgcgcaagcactggttaaacatagctctggtcaagcagatccgcatagcagcggtcaagctggtccgtatggtatggatgaaattaccgcgcaggttaaacgtaaattctgcgagatcttcgagcgcgacgttgaagtttttctggttccgaccggtaccgctgctaacgcactgtgtctgtctgcaatgaccccgccgtggggtaatatttattgccaccatgcaagccatattaataacgacgagtgcggcgcaccggaatttttcagcaacggcgccaaactgatgaccgttgacggtccggcagcaaaactggatattgtacgtctgcgcgaacgtaccagcgaaaaagttggcgacgttcataccacccaaccggcttgcgttagtattacccaggcaaccgaagttggtagcatctataccctggacgaaatcgaagcgattggcgacgtctgcaaaagtagtagtctgggcctgcatatggacggtagtcgttttgcgaacgcactggttagtctgggttgttctccggcagaaatgacctggaaagcaggtgttgacgcactgagttttggcgcaaccaaaaacggcgttctggctgcagaagcaattgttctgtttaacaccagcctggccaccgaaatgagctatcgtcgtaaacgcgcaggtcatctgattagcaaacatcgtttcctgagcgcacagattgacgcatatctgaccgacgatctgtggctgcgtaacgcacgtaaagcaaacgcagcagcacaacgtctggcacaaggtctggaaggtctgggcggcgttgaagttctgggcggtaccgaagcaaacattctgttctgccgtatggactctccgatgattgacgcactgctgaaagcgggctttaaatttggctatgaacgctggggtccgaacgttgttcgttttgtcaccagctttgcaaccaccgcagaagacgttgatcatctgctgaaccaagttcgtctggcagcagatcgtacccaagaacgt

SEQ ID NO: 196 - protein, 365 aa, Artificial sequence
  Engineered sequence
MNGETSRPPALGFSSENIAGASPEVAQALVKHSSGQADPHSSGQAGPYGMDEITAQVKRKFCEIFERDVEVFLVPTGTAANALCLSAMTPPWGNIYCHHASHINNDECGAPEFFSNGAKLMTVDGPAAKLDIVRLRERTSEKVGDVHTTQPACVSITQATEVGSIYTLDEIEAIGDVCKSSSLGLHMDGSRFANALVSLGCSPAEMTWKAGVDALSFGATKNGVLAAEAIVLFNTSLATEMSYRRKRAGHLISKHRFLSAQIDAYLTDDLWLRNARKANAAAQRLAQGLEGLGGVEVLGGTEANILFCRMDSPMIDALLKAGFKFGYERWGPNVVRFVTSFATTAEDVDHLLNQVRLAADRTQER

SEQ ID NO: 197 - DNA, 1101 bp, Artificial sequence
  Engineered sequence
atgaatggtgaaaccagtcgtccgccggcactgggttttagcagcgaaaacattgcaggcgcaagtccggaagttgcgcaagcactggttaaacatagctctggtcaagcagatccgtatggtcatagcagcggtcaagctggtccgtatggtatggatgaaattaccgcgcaggttaaacgtaaattctgcgagatcttcgagcgcgacgttgaagtttttctggttccgaccggtaccgctgctaacgcactgtgtctgtctgcaatgaccccgccgtggggtaatatttattgccaccatgcaagccatattaataacgacgagtgcggcgcaccggaatttttcagcaacggcgccaaactgatgaccgttgacggtccggcagcaaaactggatattgtacgtctgcgcgaacgtaccagcgaaaaagttggcgacgttcataccacccaaccggcttgcgttagtattacccaggcaaccgaagttggtagcatctataccctggacgaaatcgaagcgattggcgacgtctgcaaaagtagtagtctgggcctgcatatggacggtagtcgttttgcgaacgcactggttagtctgggttgttctccggcagaaatgacctggaaagcaggtgttgacgcactgagttttggcgcaaccaaaaacggcgttctggctgcagaagcaattgttctgtttaacaccagcctggccaccgaaatgagctatcgtcgtaaacgcgcaggtcatctgattagcaaacatcgtttcctgagcgcacagattgacgcatatctgaccgacgatctgtggctgcgtaacgcacgtaaagcaaacgcagcagcacaacgtctggcacaaggtctggaaggtctgggcggcgttgaagttctgggcggtaccgaagcaaacattctgttctgccgtatggactctccgatgattgacgcactgctgaaagcgggctttaaatttggctatgaacgctggggtccgaacgttgttcgttttgtcaccagctttgcaaccaccgcagaagacgttgatcatctgctgaaccaagttcgtctggcagcagatcgtacccaagaacgt

SEQ ID NO: 198 - protein, 367 aa, Artificial sequence
  Engineered sequence
MNGETSRPPALGFSSENIAGASPEVAQALVKHSSGQADPYGHSSGQAGPYGMDEITAQVKRKFCEIFERDVEVFLVPTGTAANALCLSAMTPPWGNIYCHHASHINNDECGAPEFFSNGAKLMTVDGPAAKLDIVRLRERTSEKVGDVHTTQPACVSITQATEVGSIYTLDEIEAIGDVCKSSSLGLHMDGSRFANALVSLGCSPAEMTWKAGVDALSFGATKNGVLAAEAIVLFNTSLATEMSYRRKRAGHLISKHRFLSAQIDAYLTDDLWLRNARKANAAAQRLAQGLEGLGGVEVLGGTEANILFCRMDSPMIDALLKAGFKFGYERWGPNVVRFVTSFATTAEDVDHLLNQVRLAADRTQER

SEQ ID NO: 199 - DNA, 1107 bp, Artificial sequence
  Engineered sequence
atgaatggtgaaaccagtcgtccgccggcactgggttttagcagcgaaaacattgcaggcgcaagtccggaagttgcgcaagcactggttaaacatagctctggtcaagcagatccgtatggtaccgaccatagcagcggtcaagctggtccgtatggtatggatgaaattaccgcgcaggttaaacgtaaattctgcgagatcttcgagcgcgacgttgaagtttttctggttccgaccggtaccgctgctaacgcactgtgtctgtctgcaatgaccccgccgtggggtaatatttattgccaccatgcaagccatattaataacgacgagtgcggcgcaccggaatttttcagcaacggcgccaaactgatgaccgttgacggtccggcagcaaaactggatattgtacgtctgcgcgaacgtaccagcgaaaaagttggcgacgttcataccacccaaccggcttgcgttagtattacccaggcaaccgaagttggtagcatctataccctggacgaaatcgaagcgattggcgacgtctgcaaaagtagtagtctgggcctgcatatggacggtagtcgttttgcgaacgcactggttagtctgggttgttctccggcagaaatgacctggaaagcaggtgttgacgcactgagttttggcgcaaccaaaaacggcgttctggctgcagaagcaattgttctgtttaacaccagcctggccaccgaaatgagctatcgtcgtaaacgcgcaggtcatctgattagcaaacatcgtttcctgagcgcacagattgacgcatatctgaccgacgatctgtggctgcgtaacgcacgtaaagcaaacgcagcagcacaacgtctggcacaaggtctggaaggtctgggcggcgttgaagttctgggcggtaccgaagcaaacattctgttctgccgtatggactctccgatgattgacgcactgctgaaagcgggctttaaatttggctatgaacgctggggtccgaacgttgttcgttttgtcaccagctttgcaaccaccgcagaagacgttgatcatctgctgaaccaagttcgtctggcagcagatcgtacccaagaacgt

SEQ ID NO: 200 - protein, 369 aa, Artificial sequence
  Engineered sequence
MNGETSRPPALGFSSENIAGASPEVAQALVKHSSGQADPYGTDHSSGQAGPYGMDEITAQVKRKFCEIFERDVEVFLVPTGTAANALCLSAMTPPWGNIYCHHASHINNDECGAPEFFSNGAKLMTVDGPAAKLDIVRLRERTSEKVGDVHTTQPACVSITQATEVGSIYTLDEIEAIGDVCKSSSLGLHMDGSRFANALVSLGCSPAEMTWKAGVDALSFGATKNGVLAAEAIVLFNTSLATEMSYRRKRAGHLISKHRFLSAQIDAYLTDDLWLRNARKANAAAQRLAQGLEGLGGVEVLGGTEANILFCRMDSPMIDALLKAGFKFGYERWGPNVVRFVTSFATTAEDVDHLLNQVRLAADRTQER

SEQ ID NO: 201 - DNA, 1083 bp, Artificial sequence
  Engineered sequence
atgagtcgtccgccggcactgggttttagcagcgaaaacattgcaggcgcaagtccggaagttgcgcaagcactggttaaacatagctctggtcaagcagatccgcatagcagcggtcaagctggtccgtatggtatggatgaaattaccgcgcaggttaaacgtaaattctgcgagatcttcgagcgcgacgttgaagtttttctggttccgaccggtaccgctgctaacgcactgtgtctgtctgcaatgaccccgccgtggggtaatatttattgccaccatgcaagccatattaataacgacgagtgcggcgcaccggaatttttcagcaacggcgccaaactgatgaccgttgacggtccggcagcaaaactggatattgtacgtctgcgcgaacgtaccagcgaaaaagttggcgacgttcataccacccaaccggcttgcgttagtattacccaggcaaccgaagttggtagcatctataccctggacgaaatcgaagcgattggcgacgtctgcaaaagtagtagtctgggcctgcatatggacggtagtcgttttgcgaacgcactggttagtctgggttgttctccggcagaaatgacctggaaagcaggtgttgacgcactgagttttggcgcaaccaaaaacggcgttctggctgcagaagcaattgttctgtttaacaccagcctggccaccgaaatgagctatcgtcgtaaacgcgcaggtcatctgattagcaaacatcgtttcctgagcgcacagattgacgcatatctgaccgacgatctgtggctgcgtaacgcacgtaaagcaaacgcagcagcacaacgtctggcacaaggtctggaaggtctgggcggcgttgaagttctgggcggtaccgaagcaaacattctgttctgccgtatggactctccgatgattgacgcactgctgaaagcgggctttaaatttggctatgaacgctggggtccgaacgttgttcgttttgtcaccagctttgcaaccaccgcagaagacgttgatcatctgctgaaccaagttcgtctggcagcagatcgtacccaagaacgt

SEQ ID NO: 202 - protein, 361 aa, Artificial sequence
  Engineered sequence
MSRPPALGFSSENIAGASPEVAQALVKHSSGQADPHSSGQAGPYGMDEITAQVKRKFCEIFERDVEVFLVPTGTAANALCLSAMTPPWGNIYCHHASHINNDECGAPEFFSNGAKLMTVDGPAAKLDIVRLRERTSEKVGDVHTTQPACVSITQATEVGSIYTLDEIEAIGDVCKSSSLGLHMDGSRFANALVSLGCSPAEMTWKAGVDALSFGATKNGVLAAEAIVLFNTSLATEMSYRRKRAGHLISKHRFLSAQIDAYLTDDLWLRNARKANAAAQRLAQGLEGLGGVEVLGGTEANILFCRMDSPMIDALLKAGFKFGYERWGPNVVRFVTSFATTAEDVDHLLNQVRLAADRTQER

SEQ ID NO: 203 - DNA, 1080 bp, Artificial sequence
  Engineered sequence
atgcgtccgccggcactgggttttagcagcgaaaacattgcaggcgcaagtccggaagttgcgcaagcactggttaaacatagctctggtcaagcagatccgcatagcagcggtcaagctggtccgtatggtatggatgaaattaccgcgcaggttaaacgtaaattctgcgagatcttcgagcgcgacgttgaagtttttctggttccgaccggtaccgctgctaacgcactgtgtctgtctgcaatgaccccgccgtggggtaatatttattgccaccatgcaagccatattaataacgacgagtgcggcgcaccggaatttttcagcaacggcgccaaactgatgaccgttgacggtccggcagcaaaactggatattgtacgtctgcgcgaacgtaccagcgaaaaagttggcgacgttcataccacccaaccggcttgcgttagtattacccaggcaaccgaagttggtagcatctataccctggacgaaatcgaagcgattggcgacgtctgcaaaagtagtagtctgggcctgcatatggacggtagtcgttttgcgaacgcactggttagtctgggttgttctccggcagaaatgacctggaaagcaggtgttgacgcactgagttttggcgcaaccaaaaacggcgttctggctgcagaagcaattgttctgtttaacaccagcctggccaccgaaatgagctatcgtcgtaaacgcgcaggtcatctgattagcaaacatcgtttcctgagcgcacagattgacgcatatctgaccgacgatctgtggctgcgtaacgcacgtaaagcaaacgcagcagcacaacgtctggcacaaggtctggaaggtctgggcggcgttgaagttctgggcggtaccgaagcaaacattctgttctgccgtatggactctccgatgattgacgcactgctgaaagcgggctttaaatttggctatgaacgctggggtccgaacgttgttcgttttgtcaccagctttgcaaccaccgcagaagacgttgatcatctgctgaaccaagttcgtctggcagcagatcgtacccaagaacgt

SEQ ID NO: 204 - protein, 360 aa, Artificial sequence
  Engineered sequence
MRPPALGFSSENIAGASPEVAQALVKHSSGQADPHSSGQAGPYGMDEITAQVKRKFCEIFERDVEVFLVPTGTAANALCLSAMTPPWGNIYCHHASHINNDECGAPEFFSNGAKLMTVDGPAAKLDIVRLRERTSEKVGDVHTTQPACVSITQATEVGSIYTLDEIEAIGDVCKSSSLGLHMDGSRFANALVSLGCSPAEMTWKAGVDALSFGATKNGVLAAEAIVLFNTSLATEMSYRRKRAGHLISKHRFLSAQIDAYLTDDLWLRNARKANAAAQRLAQGLEGLGGVEVLGGTEANILFCRMDSPMIDALLKAGFKFGYERWGPNVVRFVTSFATTAEDVDHLLNQVRLAADRTQER

SEQ ID NO: 205 - DNA, 1074 bp, Artificial sequence
  Engineered sequence
atgccggcactgggttttagcagcgaaaacattgcaggcgcaagtccggaagttgcgcaagcactggttaaacatagctctggtcaagcagatccgcatagcagcggtcaagctggtccgtatggtatggatgaaattaccgcgcaggttaaacgtaaattctgcgagatcttcgagcgcgacgttgaagtttttctggttccgaccggtaccgctgctaacgcactgtgtctgtctgcaatgaccccgccgtggggtaatatttattgccaccatgcaagccatattaataacgacgagtgcggcgcaccggaatttttcagcaacggcgccaaactgatgaccgttgacggtccggcagcaaaactggatattgtacgtctgcgcgaacgtaccagcgaaaaagttggcgacgttcataccacccaaccggcttgcgttagtattacccaggcaaccgaagttggtagcatctataccctggacgaaatcgaagcgattggcgacgtctgcaaaagtagtagtctgggcctgcatatggacggtagtcgttttgcgaacgcactggttagtctgggttgttctccggcagaaatgacctggaaagcaggtgttgacgcactgagttttggcgcaaccaaaaacggcgttctggctgcagaagcaattgttctgtttaacaccagcctggccaccgaaatgagctatcgtcgtaaacgcgcaggtcatctgattagcaaacatcgtttcctgagcgcacagattgacgcatatctgaccgacgatctgtggctgcgtaacgcacgtaaagcaaacgcagcagcacaacgtctggcacaaggtctggaaggtctgggcggcgttgaagttctgggcggtaccgaagcaaacattctgttctgccgtatggactctccgatgattgacgcactgctgaaagcgggctttaaatttggctatgaacgctggggtccgaacgttgttcgttttgtcaccagctttgcaaccaccgcagaagacgttgatcatctgctgaaccaagttcgtctggcagcagatcgtacccaagaacgt

SEQ ID NO: 206 - protein, 358 aa, Artificial sequence
  Engineered sequence
MPALGFSSENIAGASPEVAQALVKHSSGQADPHSSGQAGPYGMDEITAQVKRKFCEIFERDVEVFLVPTGTAANALCLSAMTPPWGNIYCHHASHINNDECGAPEFFSNGAKLMTVDGPAAKLDIVRLRERTSEKVGDVHTTQPACVSITQATEVGSIYTLDEIEAIGDVCKSSSLGLHMDGSRFANALVSLGCSPAEMTWKAGVDALSFGATKNGVLAAEAIVLFNTSLATEMSYRRKRAGHLISKHRFLSAQIDAYLTDDLWLRNARKANAAAQRLAQGLEGLGGVEVLGGTEANILFCRMDSPMIDALLKAGFKFGYERWGPNVVRFVTSFATTAEDVDHLLNQVRLAADRTQER

SEQ ID NO: 207 - DNA, 1077 bp, Artificial sequence
  Engineered sequence
atgaatggtgaaaccagtcgtccgccggcactgggttttagcagcgaaaacattgcaggcgcaagtccggaagttgcgcaagcactggttaaacatagcagcggtcaagctggtccgtatggtatggatgaaattaccgcgcaggttaaacatagccgtaaattctgcgagatcttcgagcgcgacgttgaagtttttctggttccgaccggtaccgctgctaacgcactgtgtctgtctgcaatgaccccgccgtggggtaatatttattgccaccatgcaagccatattaataacgacgagtgcggcgcaccggaatttttcagcaacggcgccaaactgatgaccgttgacggtccggcagcaaaactggatattgtacgtctgcgcgaacgtaccagcgaaaaagttggcgacgttcataccacccaaccggcttgcgttagtattacccaggcaaccgaagttggtagcatctataccctggacgaaatcgaagcgattggcgacgtctgcaaaagtagtagtctgggcctgcatatggacggtagtcgttttgcgaacgcactggttagtctgggttgttctccggcagaaatgacctggaaagcaggtgttgacgcactgagttttggcgcaaccaaaaacggcgttctggctgcagaagcaattgttctgtttaacaccagcctggccaccgaaatgagctatcgtcgtaaacgcgcaggtcatctgattagcaaacatcgtttcctgagcgcacagattgacgcatatctgaccgacgatctgtggctgcgtaacgcacgtaaagcaaacgcagcagcacaacgtctggcacaaggtctggaaggtctgggcggcgttgaagttctgggcggtaccgaagcaaacattctgttctgccgtatggactctccgatgattgacgcactgctgaaagcgggctttaaatttggctatgaacgctggggtccgaacgttgttcgttttgtcaccagctttgcaaccaccgcagaagacgttgatcatctgctgaaccaagttcgtctggcagcagatcgtacccaagaacgt

SEQ ID NO: 208 - protein, 359 aa, Artificial sequence
  Engineered sequence
MNGETSRPPALGFSSENIAGASPEVAQALVKHSSGQAGPYGMDEITAQVKHSRKFCEIFERDVEVFLVPTGTAANALCLSAMTPPWGNIYCHHASHINNDECGAPEFFSNGAKLMTVDGPAAKLDIVRLRERTSEKVGDVHTTQPACVSITQATEVGSIYTLDEIEAIGDVCKSSSLGLHMDGSRFANALVSLGCSPAEMTWKAGVDALSFGATKNGVLAAEAIVLFNTSLATEMSYRRKRAGHLISKHRFLSAQIDAYLTDDLWLRNARKANAAAQRLAQGLEGLGGVEVLGGTEANILFCRMDSPMIDALLKAGFKFGYERWGPNVVRFVTSFATTAEDVDHLLNQVRLAADRTQER

SEQ ID NO: 209 - DNA, 1077 bp, Artificial sequence
  Engineered sequence
atgaatggtgaaaccagtcgtccgccggcactgggttttagcagcgaaaacattgcaggcgcaagtccggaagttgcgcaagcactggttaaacatagccatagcagcggtcaagctggtccgtatggtatggatgaaattaccgcgcaggttaaacgtaaattctgcgagatcttcgagcgcgacgttgaagtttttctggttccgaccggtaccgctgctaacgcactgtgtctgtctgcaatgaccccgccgtggggtaatatttattgccaccatgcaagccatattaataacgacgagtgcggcgcaccggaatttttcagcaacggcgccaaactgatgaccgttgacggtccggcagcaaaactggatattgtacgtctgcgcgaacgtaccagcgaaaaagttggcgacgttcataccacccaaccggcttgcgttagtattacccaggcaaccgaagttggtagcatctataccctggacgaaatcgaagcgattggcgacgtctgcaaaagtagtagtctgggcctgcatatggacggtagtcgttttgcgaacgcactggttagtctgggttgttctccggcagaaatgacctggaaagcaggtgttgacgcactgagttttggcgcaaccaaaaacggcgttctggctgcagaagcaattgttctgtttaacaccagcctggccaccgaaatgagctatcgtcgtaaacgcgcaggtcatctgattagcaaacatcgtttcctgagcgcacagattgacgcatatctgaccgacgatctgtggctgcgtaacgcacgtaaagcaaacgcagcagcacaacgtctggcacaaggtctggaaggtctgggcggcgttgaagttctgggcggtaccgaagcaaacattctgttctgccgtatggactctccgatgattgacgcactgctgaaagcgggctttaaatttggctatgaacgctggggtccgaacgttgttcgttttgtcaccagctttgcaaccaccgcagaagacgttgatcatctgctgaaccaagttcgtctggcagcagatcgtacccaagaacgt

SEQ ID NO: 210 - protein, 359 aa, Artificial sequence
  Engineered sequence
MNGETSRPPALGFSSENIAGASPEVAQALVKHSHSSGQAGPYGMDEITAQVKRKFCEIFERDVEVFLVPTGTAANALCLSAMTPPWGNIYCHHASHINNDECGAPEFFSNGAKLMTVDGPAAKLDIVRLRERTSEKVGDVHTTQPACVSITQATEVGSIYTLDEIEAIGDVCKSSSLGLHMDGSRFANALVSLGCSPAEMTWKAGVDALSFGATKNGVLAAEAIVLFNTSLATEMSYRRKRAGHLISKHRFLSAQIDAYLTDDLWLRNARKANAAAQRLAQGLEGLGGVEVLGGTEANILFCRMDSPMIDALLKAGFKFGYERWGPNVVRFVTSFATTAEDVDHLLNQVRLAADRTQER

SEQ ID NO: 211 - DNA, 1083 bp, Artificial sequence
  Engineered sequence
atgaatggtgaaaccagtcgtccgccggcactgggttttagcagcgaaaacattgcaggcgcaagtccggaagttgcgcaagcactggttaaacatagctctggtcatagcagcggtcaagctggtccgtatggtatggatgaaattaccgcgcaggttaaacgtaaattctgcgagatcttcgagcgcgacgttgaagtttttctggttccgaccggtaccgctgctaacgcactgtgtctgtctgcaatgaccccgccgtggggtaatatttattgccaccatgcaagccatattaataacgacgagtgcggcgcaccggaatttttcagcaacggcgccaaactgatgaccgttgacggtccggcagcaaaactggatattgtacgtctgcgcgaacgtaccagcgaaaaagttggcgacgttcataccacccaaccggcttgcgttagtattacccaggcaaccgaagttggtagcatctataccctggacgaaatcgaagcgattggcgacgtctgcaaaagtagtagtctgggcctgcatatggacggtagtcgttttgcgaacgcactggttagtctgggttgttctccggcagaaatgacctggaaagcaggtgttgacgcactgagttttggcgcaaccaaaaacggcgttctggctgcagaagcaattgttctgtttaacaccagcctggccaccgaaatgagctatcgtcgtaaacgcgcaggtcatctgattagcaaacatcgtttcctgagcgcacagattgacgcatatctgaccgacgatctgtggctgcgtaacgcacgtaaagcaaacgcagcagcacaacgtctggcacaaggtctggaaggtctgggcggcgttgaagttctgggcggtaccgaagcaaacattctgttctgccgtatggactctccgatgattgacgcactgctgaaagcgggctttaaatttggctatgaacgctggggtccgaacgttgttcgttttgtcaccagctttgcaaccaccgcagaagacgttgatcatctgctgaaccaagttcgtctggcagcagatcgtacccaagaacgt

SEQ ID NO: 212 - protein, 361 aa, Artificial sequence
  Engineered sequence
MNGETSRPPALGFSSENIAGASPEVAQALVKHSSGHSSGQAGPYGMDEITAQVKRKFCEIFERDVEVFLVPTGTAANALCLSAMTPPWGNIYCHHASHINNDECGAPEFFSNGAKLMTVDGPAAKLDIVRLRERTSEKVGDVHTTQPACVSITQATEVGSIYTLDEIEAIGDVCKSSSLGLHMDGSRFANALVSLGCSPAEMTWKAGVDALSFGATKNGVLAAEAIVLFNTSLATEMSYRRKRAGHLISKHRFLSAQIDAYLTDDLWLRNARKANAAAQRLAQGLEGLGGVEVLGGTEANILFCRMDSPMIDALLKAGFKFGYERWGPNVVRFVTSFATTAEDVDHLLNQVRLAADRTQER

SEQ ID NO: 213 - DNA, 1026 bp, Artificial sequence
  Engineered sequence
atgaatggtgaaaccagtcgtccgccggcactgggttttagcagcgaaaacattgcaggcgcaagtccggaagttgcgcaagcactggttaaacatagctctggtcgtaaattctgcgagatcttcgagcgcgacgttgaagtttttctggttccgaccggtaccgctgctaacgcactgtgtctgtctgcaatgaccccgccgtggggtaatatttattgccaccatgcaagccatattaataacgacgagtgcggcgcaccggaatttttcagcaacggcgccaaactgatgaccgttgacggtccggcagcaaaactggatattgtacgtctgcgcgaacgtaccagcgaaaaagttggcgacgttcataccacccaaccggcttgcgttagtattacccaggcaaccgaagttggtagcatctataccctggacgaaatcgaagcgattggcgacgtctgcaaaagtagtagtctgggcctgcatatggacggtagtcgttttgcgaacgcactggttagtctgggttgttctccggcagaaatgacctggaaagcaggtgttgacgcactgagttttggcgcaaccaaaaacggcgttctggctgcagaagcaattgttctgtttaacaccagcctggccaccgaaatgagctatcgtcgtaaacgcgcaggtcatctgattagcaaacatcgtttcctgagcgcacagattgacgcatatctgaccgacgatctgtggctgcgtaacgcacgtaaagcaaacgcagcagcacaacgtctggcacaaggtctggaaggtctgggcggcgttgaagttctgggcggtaccgaagcaaacattctgttctgccgtatggactctccgatgattgacgcactgctgaaagcgggctttaaatttggctatgaacgctggggtccgaacgttgttcgttttgtcaccagctttgcaaccaccgcagaagacgttgatcatctgctgaaccaagttcgtctggcagcagatcgtacccaagaacgt

SEQ ID NO: 214 - protein, 342 aa, Artificial sequence
  Engineered sequence
MNGETSRPPALGFSSENIAGASPEVAQALVKHSSGRKFCEIFERDVEVFLVPTGTAANALCLSAMTPPWGNIYCHHASHINNDECGAPEFFSNGAKLMTVDGPAAKLDIVRLRERTSEKVGDVHTTQPACVSITQATEVGSIYTLDEIEAIGDVCKSSSLGLHMDGSRFANALVSLGCSPAEMTWKAGVDALSFGATKNGVLAAEAIVLFNTSLATEMSYRRKRAGHLISKHRFLSAQIDAYLTDDLWLRNARKANAAAQRLAQGLEGLGGVEVLGGTEANILFCRMDSPMIDALLKAGFKFGYERWGPNVVRFVTSFATTAEDVDHLLNQVRLAADRTQER

SEQ ID NO: 215 - DNA, 1038 bp, Artificial sequence
  Engineered sequence
atgaatggtgaaaccagtcgtccgccggcactgggttttagcagcgaaaacattgcaggcgcaagtccggaagttgcgcaagcactggttaaacatagctctggtcaagcagatccgcgtaaattctgcgagatcttcgagcgcgacgttgaagtttttctggttccgaccggtaccgctgctaacgcactgtgtctgtctgcaatgaccccgccgtggggtaatatttattgccaccatgcaagccatattaataacgacgagtgcggcgcaccggaatttttcagcaacggcgccaaactgatgaccgttgacggtccggcagcaaaactggatattgtacgtctgcgcgaacgtaccagcgaaaaagttggcgacgttcataccacccaaccggcttgcgttagtattacccaggcaaccgaagttggtagcatctataccctggacgaaatcgaagcgattggcgacgtctgcaaaagtagtagtctgggcctgcatatggacggtagtcgttttgcgaacgcactggttagtctgggttgttctccggcagaaatgacctggaaagcaggtgttgacgcactgagttttggcgcaaccaaaaacggcgttctggctgcagaagcaattgttctgtttaacaccagcctggccaccgaaatgagctatcgtcgtaaacgcgcaggtcatctgattagcaaacatcgtttcctgagcgcacagattgacgcatatctgaccgacgatctgtggctgcgtaacgcacgtaaagcaaacgcagcagcacaacgtctggcacaaggtctggaaggtctgggcggcgttgaagttctgggcggtaccgaagcaaacattctgttctgccgtatggactctccgatgattgacgcactgctgaaagcgggctttaaatttggctatgaacgctggggtccgaacgttgttcgttttgtcaccagctttgcaaccaccgcagaagacgttgatcatctgctgaaccaagttcgtctggcagcagatcgtacccaagaacgt

SEQ ID NO: 216 - protein, 346 aa, Artificial sequence
  Engineered sequence
MNGETSRPPALGFSSENIAGASPEVAQALVKHSSGQADPRKFCEIFERDVEVFLVPTGTAANALCLSAMTPPWGNIYCHHASHINNDECGAPEFFSNGAKLMTVDGPAAKLDIVRLRERTSEKVGDVHTTQPACVSITQATEVGSIYTLDEIEAIGDVCKSSSLGLHMDGSRFANALVSLGCSPAEMTWKAGVDALSFGATKNGVLAAEAIVLFNTSLATEMSYRRKRAGHLISKHRFLSAQIDAYLTDDLWLRNARKANAAAQRLAQGLEGLGGVEVLGGTEANILFCRMDSPMIDALLKAGFKFGYERWGPNVVRFVTSFATTAEDVDHLLNQVRLAADRTQER